European Patent Application EP 4 159 853 A1, published April 5, 2023. Title: GENOME EDITING SYSTEM AND METHOD. Applicant: ShanghaiTech University. Application EP20938166.4. The sequence listing filed with the application follows.

SEQUENCE LISTING (130 sequences)

SEQ ID NO: 1 - protein, 497 aa, Artificial Sequence
  SpCas12f1
MGESVKAIKLKILDMFLDPECTKQDDNWRKDLSTMSRFCAEAGNMCLRDLYNYFSMPKEDRISSKDLYNAMYHKTKLLHPELPGKVANQIVNHAKDVWKRNAKLIYRNQISMPTYKITTAPIRLQNNIYKLIKNKNKYIIDVQLYSKEYSKDSGKGTHRYFLVAVRDSSTRMIFDRIMSKDHIDSSKSYTQGQLQIKKDHQGKWYCIIPYTFPTHETVLDPDKVMGVDLGVAKAVYWAFNSSYKRGCIDGGEIEHFRKMIRARRVSIQNQIKHSGDARKGHGRKRALKPIETLSEKEKNFRDTINHRYANRIVEAAIKQGCGTIQIENLEGIADTTGSKFLKNWPYYDLQTKIVNKAKEHGITVVAINPQYTSQRCSMCGYIEKTNRSSQAVFECKQCGYGSRTICINCRHVQVSGDVCEECGGIVKKENVNADYNAAKNISTPYIDQIIMEKCLELGIPYRSITCKECGHIQASGNTCEVCGSTNILKPKKIRKAK

SEQ ID NO: 2 - DNA, 1491 bp, Artificial Sequence
  SpCas12f1
atgggtgaaagcgttaaagcgatcaaactgaaaatcctggacatgttcctggacccggaatgcaccaaacaggatgataactggcgtaaagatctgtctaccatgagccgcttctgcgctgaagcgggcaacatgtgcctgcgtgatctgtacaactacttcagcatgccgaaagaagatcgtatcagcagcaaagatctgtacaacgcgatgtaccacaaaaccaaactgctgcacccggaactgccgggcaaagtggcaaaccagatcgtgaaccacgcgaaagatgtttggaaacgtaacgcgaaactgatctaccgtaaccagatctccatgccgacctataaaattaccaccgcgccgatccgcctgcagaacaacatctacaaactgatcaaaaacaaaaacaaatacatcatcgacgttcagctgtacagcaaagaatacagcaaagacagcggtaaaggcacccaccgctacttcctggttgcagtgcgtgacagctctacccgtatgatcttcgatcgtatcatgagcaaagatcacatcgattcctccaaaagctacacgcagggtcagctgcagatcaaaaaagaccaccagggtaaatggtactgtatcatcccgtacaccttcccgacccacgaaaccgtgctggacccggacaaagttatgggtgttgatctgggcgttgcgaaagcggtgtactgggcgttcaactcttcttacaaacgcggctgcatcgatggcggtgaaatcgaacactttcgtaaaatgatccgtgcgcgccgtgtttccattcagaaccagatcaaacacagcggtgatgcgcgtaaaggtcacggtcgtaaacgcgctctgaaaccgatcgaaaccctgtctgaaaaagagaaaaacttccgcgataccatcaaccaccgctatgctaaccgtatcgttgaagcggcgatcaaacagggctgcggcaccatccagatcgaaaacctggaaggcatcgctgacaccaccggcagcaaattcctgaaaaactggccgtactatgatctgcagaccaaaatcgttaacaaagcgaaagaacacggcatcaccgttgtggcgatcaacccgcagtacaccagccagcgttgcagcatgtgtggctacatcgaaaaaaccaaccgcagctcccaggcagttttcgaatgcaaacagtgtggttacggcagccgtaccatctgcatcaactgccgtcacgttcaggtttccggtgatgtttgcgaagaatgcggcggcattgttaaaaaagaaaacgtgaacgcggactacaacgcggcgaaaaacattagcaccccgtacatcgatcagatcatcatggaaaaatgcctggaactgggtatcccgtaccgtagcatcacctgcaaagaatgcggtcacatccaggcgtccggtaacacctgcgaagtttgcggctctaccaacatcctgaaaccgaaaaagatccgtaaagctaaa

SEQ ID NO: 3 - RNA, 230 nt, Artificial Sequence
  SpCas12f1RNA
aagccugacauaauuuacucuguuucgcgcgccagggcaguuaggugcccuaaaagagcgaaguggccgaaaggaaaggcuaacgcuucucuaacgcuacggcgaccuuggcgaaaugccaucaauaccacgcggcccgaaaggguucgcgcgaaacugaguaauaaaacauugcggaugcggcaauacagaaccgcugucgcaucuugcguaagcgcguggauugaaac

SEQ ID NO: 4 - DNA, 7992 bp, Artificial Sequence
  pCas12f
tggctggttggcgtactgttgtggtaaatacccatatggacagttttccctttgatatgtaacggtgaacagttgttctacttttgtttgttagtcttgatgcttcactgatagatacaagagcgtcgggtgatgctgccaacttactgatttagtgtatgatggtgtttttgaggtgctccagtggcttctgtttctatcagctgtccctcctgttcagctactgacggggtggtgcgtaacggcaaaagcaccgccggacatcagcgctagcggagtgtatactggcttactatgttggcactgatgagggtgtcagtgaagtgcttcatgtggcaggagaaaaaaggctgcaccggtgcgtcagcagaatatgtgatacaggatatattccgcttcctcgctcactgactcgctacgctcggtcgttcgactgcggcgagcggaaatggcttacgaacggggcggagatttcctggaagatgccaggaagatacttaacagggaagtgagagggccgcggcaaagccgtttttccataggctccgcccccctgacaagcatcacgaaatctgacgctcaaatcagtggtggcgaaacccgacaggactataaagataccaggcgtttccccctggcggctccctcgtgcgctctcctgttcctgcctttcggtttaccggtgtcattccgctgttatggccgcgtttgtctcattccacgcctgacactcagttccgggtaggcagttcgctccaagctggactgtatgcacgaaccccccgttcagtccgaccgctgcgccttatccggtaactatcgtcttgagtccaacccggaaagacatgcaaaagcaccactggcagcagccactggtaattgatttagaggagttagtcttgaagtcatgcgccggttaaggctaaactgaaaggacaagttttggtgactgcgctcctccaagccagttacctcggttcaaagagttggtagctcagagaaccttcgaaaaaccgccctgcaaggcggttttttcgttttcagagcaagagattacgcgcagaccaaaacgatctcaagaagatcatcttattaatcagataaaatatttctagatttcagtgcaatttatctcttcaaatgtagcacctgaagtcagccccatacgatataagttgtgacgtaaaatgagacgttgatcggcacgtaagaggttccaactttcaccataatgaaataagatcactaccgggcgtattttttgagttatcgagattttcaggagctaaggaagctaaaatggagaaaaaaatcactggatataccaccgttgatatatcccaatggcatcgtaaagaacattttgaggcatttcagtcagttgctcaatgtacctataaccagaccgttcagctgggtcatccaccggatcaattcccctgctcgcgcaggctgggtgccaagctctcgggtaacatcaaggcccgatccttggagcccttgccctcccgcacgatgatcgtgccgtgatcgaaatccagatccttgacccgcagttgcaaaccctcactgatccggctcacggtaactgatgccgtatttgcagtaccagcgtacggcccacagaatgatgtcacgctgaaaatgccggcctttgaatgggttcatgtgcagctccatcagcaaaaggggatgataagtttatcaccaccgactatttgcaacagtgccgttgatcgtgctatgatcgactgatgtcatcagcggtggagtgcaatgtcgtgcaatacgaatggcgaaaagccgagctcatcggtcagcttctcaaccttggggttacccccggcggtgtgctgctggtccacagctccttccgtagcgtccggcccctcgaagatgggccacttggactgatcgaggccctgcgtgctgcgctgggtccgggagggacgctcgtcatgccctcgtggtcaggtctggacgacgagccgttcgatcctgccacgtcgcccgttacaccggaccttggagttgtctctgacacattctggcgcctgccaaatgtaaagcgcagcgcccatccatttgcctttgcggcagcggggccacaggcagagcagatcatctctgatccattgcccctgccacctcactcgcctgcaagcccggtcgcccgtgtccatgaactcgatgggcaggtacttctcctcggcgtgggacacgatgccaacacgacgctgcatcttgccgagttgatggcaaaggttccctatggggtgccgagacactgcaccattcttcaggatggcaagttggtacgcgtcgattatctcgagaatgaccactgctgtgagcgctttgccttggcggacaggtggctcaaggagaagagccttcagaaggaaggtccagtcggtcatgcctttgctcggttgatccgctcccgcgacattgtggcgacagccctgggtcaactgggccgagatccgttgatcttcctgcatccgccagaggcgggatgcgaagaatgcgatgccgctcgccagtcgattggctgagctcatgagcggagaacgagatgacgttggaggggcaaggtcgcgctgattgctggggcaacacgtgaaaggcgagatcaccaaggtagtcggcaaataatgtctaacggtacccggggatcctctagagtcgacctgcataatgtgcctgtcaaatggacgaagcagggattctgcaaaccctatgctactccgtcaagccgtcaattgtctgattcgttaccaattatgacaacttgacggctacatcattcactttttcttcacaaccggcacggaactcgctcgggctggccccggtgcattttttaaatacccgcgagaaatagagttgatcgtcaaaaccaacattgcgaccgacggtggcgataggcatccgggtggtgctcaaaagcagcttcgcctggctgatacgttggtcctcgcgccagcttaagacgctaatccctaactgctggcggaaaagatgtgacagacgcgacggcgacaagcaaacatgctgtgcgacgctggcgatatcaaaattgctgtctgccaggtgatcgctgatgtactgacaagcctcgcgtacccgattatccatcggtggatggagcgactcgttaatcgcttccatgcgccgcagtaacaattgctcaagcagatttatcgccagcagctccgaatagcgcccttccccttgcccggcgttaatgatttgcccaaacaggtcgctgaaatgcggctggtgcgcttcatccgggcgaaagaaccccgtattggcaaatattgacggccagttaagccattcatgccagtaggcgcgcggacgaaagtaaacccactggtgataccattcgcgagcctccggatgacgaccgtagtgatgaatctctcctggcgggaacagcaaaatatcacccggtcggcaaacaaattctcgtccctgatttttcaccaccccctgaccgcgaatggtgagattgagaatataacctttcattcccagcggtcggtcgataaaaaaatcgagataaccgttggcctcaatcggcgttaaacccgccaccagatgggcattaaacgagtatcccggcagcaggggatcattttgcgcttcagccatacttttcatactcccgccattcagagaagaaaccaattgtccatattgcatcagacattgccgtcactgcgtcttttactggctcttctcgctaaccaaaccggtaaccccgcttattaaaagcattctgtaacaaagcgggaccaaagccatgacaaaaacgcgtaacaaaagtgtctataatcacggcagaaaagtccacattgattatttgcacggcgtcacactttgctatgccatagcatttttatccataagattagcggatcctacctgacgctttttatcgcaactctctactgtttctccatacccgtttttttgggctagcgaaaagatgtttcgtgaagccgtcgacgcttataaaaaatggatattaatactgaaactgagatcaagcaaaagcattcactaaccccctttcctgttttcctaatcagcccggcatttcgcgggcgatattttcacagctatttcaggagttcagccatgaacgcttattacattcaggatcgtcttgaggctcagagctgggcgcgtcactaccagcagctcgcccgtgaagagaaagaggcagaactggcagacgacatggaaaaaggcctgccccagcacctgtttgaatcgctatgcatcgatcatttgcaacgccacggggccagcaaaaaatccattacccgtgcgtttgatgacgatgttgagtttcaggagcgcatggcagaacacatccggtacatggttgaaaccattgctcaccaccaggttgatattgattcagaggtataaaacgaatgagtactgcactcgcaacgctggctgggaagctggctgaacgtgtcggcatggattctgtcgacccacaggaactgatcaccactcttcgccagacggcatttaaaggtgatgccagcgatgcgcagttcatcgcattactgatcgttgccaaccagtacggccttaatccgtggacgaaagaaatttacgcctttcctgataagcagaatggcatcgttccggtggtgggcgttgatggctggtcccgcatcatcaatgaaaaccagcagtttgatggcatggactttgagcaggacaatgaatcctgtacatgccggatttaccgcaaggaccgtaatcatccgatctgcgttaccgaatggatggatgaatgccgccgcgaaccattcaaaactcgcgaaggcagagaaatcacggggccgtggcagtcgcatcccaaacggatgttacgtcataaagccatgattcagtgtgcccgtctggccttcggatttgctggtatctatgacaaggatgaagccgagcgcattgtcgaaaatactgcatacactgcagaacgtcagccggaacgcgacatcactccggttaacgatgaaaccatgcaggagattaacactctgctgatcgccctggataaaacatgggatgacgacttattgccgctctgttcccagatatttcgccgcgacattcgtgcatcgtcagaactgacacaggccgaagcagtaaaagctcttggattcctgaaacagaaagccgcagagcagaaggtggcagcatgacaccggacattatcctgcagcgtaccgggatcgatgtgagagctgtcgaacagggggatgatgcgtggcacaaattacggctcggcgtcatcaccgcttcagaagttcacaacgtgatagcaaaaccccgctccggaaagaagtggcctgacatgaaaatgtcctacttccacaccctgcttgctgaggtttgcaccggtgtggctccggaagttaacgctaaagcactggcctggggaaaacagtacgagaacgacgccagaaccctgtttgaattcacttccggcgtgaatgttactgaatccccgatcatctatcgcgacgaaagtatgcgtaccgcctgctctcccgatggtttatgcagtgacggcaacggccttgaactgaaatgcccgtttacctcccgggatttcatgaagttccggctcggtggtttcgaggccataaagtcagcttacatggcccaggtgcagtacagcatgtgggtgacgcgaaaaaatgcctggtactttgccaactatgacccgcgtatgaagcgtgaaggcctgcattatgtcgtgattgagcgggatgaaaagtacatggcgagttttgacgagatcgtgccggagttcatcgaaaaaatggacgaggcactggctgaaattggttttgtatttggggagcaatggcgatgacgcatcctcacgataataagcttcctgctgaacatcaaaggcaagaaaacatctgttgtcaaagacagcatccttgaacaaggacaattaacagttaacaaataaaaacgcaaaagaaaatgccgatattgactaccggaagcagtgtgaccgtgtgcttctcaaatgcctgattcaggctgtctatgtgtgactgttgagctgtaacaagttgtctcaggtgttcaatttcatgttctagttgctttgttttactggtttcacctgttctattaggtgttacatgctgttcatctgttacattgtcgatctgttcatggtgaacagctttaaatgcaccaaaaactcgtaaaagctctgatgtatctatcttttttacaccgttttcatctgtgcatatagctatactgatttcgtcagactcacagtcaaacatgccggtcagttggcctggtgatggcgggatcgttgtatatttcttgacaccttttcggcaccgccctaaaattctgcgtcctcataatatatgaggcgatttattacgtgtttacgaagcaaaagctaaaaccaggagctatttaatgggtgaaagcgttaaagcgatcaaactgaaaatcctggacatgttcctggacccggaatgcaccaaacaggatgataactggcgtaaagatctgtctaccatgagccgcttctgcgctgaagcgggcaacatgtgcctgcgtgatctgtacaactacttcagcatgccgaaagaagatcgtatcagcagcaaagatctgtacaacgcgatgtaccacaaaaccaaactgctgcacccggaactgccgggcaaagtggcaaaccagatcgtgaaccacgcgaaagatgtttggaaacgtaacgcgaaactgatctaccgtaaccagatctccatgccgacctataaaattaccaccgcgccgatccgcctgcagaacaacatctacaaactgatcaaaaacaaaaacaaatacatcatcgacgttcagctgtacagcaaagaatacagcaaagacagcggtaaaggcacccaccgctacttcctggttgcagtgcgtgacagctctacccgtatgatcttcgatcgtatcatgagcaaagatcacatcgattcctccaaaagctacacgcagggtcagctgcagatcaaaaaagaccaccagggtaaatggtactgtatcatcccgtacaccttcccgacccacgaaaccgtgctggacccggacaaagttatgggtgttgatctgggcgttgcgaaagcggtgtactgggcgttcaactcttcttacaaacgcggctgcatcgatggcggtgaaatcgaacactttcgtaaaatgatccgtgcgcgccgtgtttccattcagaaccagatcaaacacagcggtgatgcgcgtaaaggtcacggtcgtaaacgcgctctgaaaccgatcgaaaccctgtctgaaaaagagaaaaacttccgcgataccatcaaccaccgctatgctaaccgtatcgttgaagcggcgatcaaacagggctgcggcaccatccagatcgaaaacctggaaggcatcgctgacaccaccggcagcaaattcctgaaaaactggccgtactatgatctgcagaccaaaatcgttaacaaagcgaaagaacacggcatcaccgttgtggcgatcaacccgcagtacaccagccagcgttgcagcatgtgtggctacatcgaaaaaaccaaccgcagctcccaggcagttttcgaatgcaaacagtgtggttacggcagccgtaccatctgcatcaactgccgtcacgttcaggtttccggtgatgtttgcgaagaatgcggcggcattgttaaaaaagaaaacgtgaacgcggactacaacgcggcgaaaaacattagcaccccgtacatcgatcagatcatcatggaaaaatgcctggaactgggtatcccgtaccgtagcatcacctgcaaagaatgcggtcacatccaggcgtccggtaacacctgcgaagtttgcggctctaccaacatcctgaaaccgaaaaagatccgtaaagctaaataa

SEQ ID NO: 5 - DNA, 1061 bp, Artificial Sequence
  p15a
cgtcgggtgatgctgccaacttactgatttagtgtatgatggtgtttttgaggtgctccagtggcttctgtttctatcagctgtccctcctgttcagctactgacggggtggtgcgtaacggcaaaagcaccgccggacatcagcgctagcggagtgtatactggcttactatgttggcactgatgagggtgtcagtgaagtgcttcatgtggcaggagaaaaaaggctgcaccggtgcgtcagcagaatatgtgatacaggatatattccgcttcctcgctcactgactcgctacgctcggtcgttcgactgcggcgagcggaaatggcttacgaacggggcggagatttcctggaagatgccaggaagatacttaacagggaagtgagagggccgcggcaaagccgtttttccataggctccgcccccctgacaagcatcacgaaatctgacgctcaaatcagtggtggcgaaacccgacaggactataaagataccaggcgtttccccctggcggctccctcgtgcgctctcctgttcctgcctttcggtttaccggtgtcattccgctgttatggccgcgtttgtctcattccacgcctgacactcagttccgggtaggcagttcgctccaagctggactgtatgcacgaaccccccgttcagtccgaccgctgcgccttatccggtaactatcgtcttgagtccaacccggaaagacatgcaaaagcaccactggcagcagccactggtaattgatttagaggagttagtcttgaagtcatgcgccggttaaggctaaactgaaaggacaagttttggtgactgcgctcctccaagccagttacctcggttcaaagagttggtagctcagagaaccttcgaaaaaccgccctgcaaggcggttttttcgttttcagagcaagagattacgcgcagaccaaaacgatctcaagaagatcatcttattaatcagataaaatatttctagatttcagtgcaatttatctcttcaaatgtagcacctgaagtcagccccatacgatataagttgtgacgt

SEQ ID NO: 6 - DNA, 40 bp, Artificial Sequence
  -Red5'
tacgatataagttgtgacgtaaaatgagacgttgatcggc

SEQ ID NO: 7 - DNA, 26 bp, Artificial Sequence
  -Red3'
taaatagctcctggttttagcttttg

SEQ ID NO: 8 - DNA, 40 bp, Artificial Sequence
  p15a5'
ttcactgatagatacaagagcgtcgggtgatgctgccaac

SEQ ID NO: 9 - DNA, 45 bp, Artificial Sequence
  p15a3'
gccgatcaacgtctcattttacgtcacaacttatatcgtatgggg

SEQ ID NO: 10 - DNA, 48 bp, Artificial Sequence
  Cas12f5'
aaagctaaaaccaggagctatttaatgggtgaaagcgttaaagcgatc

SEQ ID NO: 11 - DNA, 160 bp, Artificial Sequence
  Cas12f3'
ccgacgctcttgtatctatcagtgaagcatcaagactaacaaacaaaagtagaacaactgttcaccgttacatatcaaagggaaaactgtccatatgggtatttaccacaacagtacgccaaccagccattatttagctttacggatctttttcggtttc

SEQ ID NO: 12 - DNA, 5051 bp, Artificial Sequence
  pgRNA
gatatcgaattcctgcagcccgggggatccactagttctagagcggccgccaccgcggtggagctcatcccaatggcgcgccgagcttggctcgagcatggtcatagctgtttcctgtgtgaaattgttatccgctcacaattccacacaacatacgagccggaagcataaagtgtaaagcctggggtgcctaatgagtgagctaactcacattaattgcgttgcgctcactgcccgctttccagtcgggaaacctgtcgtgccagctgcattaatgaatcggccaacgcgcggggagaggcggtttgcgtattgggcgctcttccgcttcctcgctcactgactcgctgcgctcggtcgttcggctgcggcgagcggtatcagctcactcaaaggcggtaatacggttatccacagaatcaggggataacgcaggaaagaacatgtgagcaaaaggccagcaaaaggccaggaaccgtaaaaaggccgcgttgctggcgtttttccataggctccgcccccctgacgagcatcacaaaaatcgacgctcaagtcagaggtggcgaaacccgacaggactataaagataccaggcgtttccccctggaagctccctcgtgcgctctcctgttccgaccctgccgcttaccggatacctgtccgcctttctcccttcgggaagcgtggcgctttctcatagctcacgctgtaggtatctcagttcggtgtaggtcgttcgctccaagctgggctgtgtgcacgaaccccccgttcagcccgaccgctgcgccttatccggtaactatcgtcttgagtccaacccggtaagacacgacttatcgccactggcagcagccactggtaacaggattagcagagcgaggtatgtaggcggtgctacagagttcttgaagtggtggcctaactacggctacactagaagaacagtatttggtatctgcgctctgctgaagccagttaccttcggaaaaagagttggtagctcttgatccggcaaacaaaccaccgctggtagcggtggtttttttgtttgcaagcagcagattacgcgcagaaaaaaaggatctcaagaagatcctttgatcttttctacggggtctgacgctcagtggaacgaaaactcacgttaagggattttggtcatgagattatcaaaaaggatcttcacctagatccttttaaattaaaaatgaagttttaaatcaatctaaagtatatatgagtaaacttggtctgacagttagaaaaactcatcgagcatcaaatgaaactgcaatttattcatatcaggattatcaataccatatttttgaaaaagccgtttctgtaatgaaggagaaaactcaccgaggcagttccataggatggcaagatcctggtatcggtctgcgattccgactcgtccaacatcaatacaacctattaatttcccctcgtcaaaaataaggttatcaagtgagaaatcaccatgagtgacgactgaatccggtgagaatggcaaaagtttatgcatttctttccagacttgttcaacaggccagccattacgctcgtcatcaaaatcactcgcatcaaccaaaccgttattcattcgtgattgcgcctgagcgagacgaaatacgcgatcgctgttaaaaggacaattacaaacaggaatcgaatgcaaccggcgcaggaacactgccagcgcatcaacaatattttcacctgaatcaggatattcttctaatacctggaatgctgttttcccagggatcgcagtggtgagtaaccatgcatcatcaggagtacggataaaatgcttgatggtcggaagaggcataaattccgtcagccagtttagtctgaccatctcatctgtaacatcattggcaacgctacctttgccatgtttcagaaacaactctggcgcatcgggcttcccatacaatcgatagattgtcgcacctgattgcccgacattatcgcgagcccatttatacccatataaatcagcatccatgttggaatttaatcgcggcctagagcaagacgtttcccgttgaatatggctcatactcttcctttttcaatattattgaagcatttatcagggttattgtctcatgagcggatacatatttgaatgtatttagaaaaataaacaaataggggttccgcgcacatttccccgaaaagtgccacctgacgtctaagaaaccattattatcatgacattaacctataaaaataggcgtatcacgaggccctttcgtctcgcgcgtttcggtgatgacggtgaaaacctctgacacatgcagctcccggagacggtcacagcttgtctgtaagcggatgccgggagcagacaagcccgtcagggcgcgtcagcgggtgttggcgggtgtcggggctggcttaactatgcggcatcagagcagattgtactgagagtgcaccatatgcggtgtgaaataccgcacagatgcgtaaggagaaaataccgcatcaggcgccattcgccattcaggctgcgcaactgttgggaagggcgatcggtgcgggcctcttcgctattacgccagctggcgaaagggggatgtgctgcaaggcgattaagttgggtaacgccagggttttcccagtcacgacgttgtaaaacgacggccagtgaattgacgcgtattgggatggtaccgggccccccctcgaggtcgacggtatcgatacggcatcagagcagattgtactgagagtgcaccataatcggcattttcttttgcgtttttatttgttaactgttaattgtccttgttcaaggatgctgtctttgacaacagatgttttcttgcctttgatgttcagcaggaagctaggcgcaaacgttgattgtttgtctgcgtagaatcctctgtttgtcatatagcttgtaatcacgacattgtttcctttcgcttgaggtacagcgaagtgtgagtaagtaaaggttacatcgttaggatcaagatccatttttaacacaaggccagttttgttcagcggcttgtatgggccagttaaagaattagaaacataaccaagcatgtaaatatcgttagacgtaatgccgtcaatcgtcatttttgatccgcgggagtcagtgaacagataccatttgccgttcattttaaagacgttcgcgcgttcaatttcatctgttactgtgttagatgcaatcagcggtttcatcacttttttcagtgtgtaatcatcgtttagctcaatcataccgagagcgccgtttgctaactcagccgtgcgttttttatcgctttgcagaagtttttgactttcttgacggaagaatgatgtgcttttgccatagtatgctttgttaaataaagattcttcgccttggtagccatcttcagttccagtgtttgcttcaaatactaagtatttgtggcctttatcttctacgtagtgaggatctctcagcgtatggttgtcgcctgagctgtagttgccttcatcgatgaactgctgtacattttgatacgtttttccgtcaccgtcaaagattgatttataatcctctacaccgttgatgttcaaagagctgtctgatgctgatacgttaacttgtgcagttgtcagtgtttgtttgccgtaatgtttaccggagaaatcagtgtagaataaacggatttttccgtcagatgtaaatgtggctgaacctgaccattcttgtgtttggtcttttaggatagaatcatttgcatcgaatttgtcgctgtctttaaagacgcggccagcgtttttccagctgtcaatagaagtttcgccgactttttgatagaacatgtaaatcgatgtgtcatccgcatttttaggatctccggctaatgcaaagacgatgtggtagccgtgatagtttgcgacagtgccgtcagcgttttgtaatggccagctgtcccaaacgtccaggccttttgcagaagagatatttttaattgtggacgaatcgaactcaggaacttgatatttttcatttttttgctgttcagggatttgcagcatatcatggcgtgtaatatgggaaatgccgtatgtttccttatatggcttttggttcgtttctttcgcaaacgcttgagttgcgcctcctgccagcagtgcggtagtaaaggttaatactgttgcttgttttgcaaactttttgatgttcatcgttcatgtctccttttttatgtactgtgttagcggtctgcttcttccagccctcctgtttgaagatggcaagttagttacgcacaataaaaaaagacctaaaatatgtaaggggtgacgccaaagtatacactttgccctttacacattttaggtcttgcctgctttatcagtaacaaacccgcgcgatttacttttcgacctcattctattagactctcgtttggattgcaactggtctattttcctcttttgtttgatagaaaatcataaaaggatttgcagactacgggcctaaagaactaaaaaatctatctgtttcttttcattctctgtattttttatagtttctgttgcatgggcataaagttgcaagcttgatatcttgacagctagctcagtcctaggtataatactagttcgcgaaccccaagttataaaaaaggtctttgacaacaaaacaagtcatatcgctttaaagcctgacataatttactctgtttcgcgcgccagggcagttaggtgccctaaaagagcgaagtggccgaaaggaaaggctaacgcttctctaacgctacggcgaccttggcgaaatgccatcaataccacgcggcccgaaagggttcgcgcgaaactgagtaataaaacattgcggatgcggcaatacagaaccgctgtcgcatcttgcgtaagcgcgtggattgaaaccgagaccattggtctcagtcgcatcttgcgtaagcgcgtggattgaaacttaattaacctaggctgctgccaccgctgagcaataactagcataaccccttggggcctctaaacgggtcttgaggggttttttg

SEQ ID NO: 13 - DNA, 480 bp, Artificial Sequence
  RNADNA
ttgacagctagctcagtcctaggtataatactagttcgcgaaccccaagttataaaaaaggtctttgacaacaaaacaagtcatatcgctttaaagcctgacataatttactctgtttcgcgcgccagggcagttaggtgccctaaaagagcgaagtggccgaaaggaaaggctaacgcttctctaacgctacggcgaccttggcgaaatgccatcaataccacgcggcccgaaagggttcgcgcgaaactgagtaataaaacattgcggatgcggcaatacagaaccgctgtcgcatcttgcgtaagcgcgtggattgaaaccgagaccattggtctcagtcgcatcttgcgtaagcgcgtggattgaaacttaattaacctaggctgctgccaccgctgagcaataactagcataaccccttggggcctctaaacgggtcttgaggggttttttggatatcgaattcctgcagcccgg

SEQ ID NO: 14 - DNA, 23 bp, Artificial Sequence
  pSGKP5'
gatatcgaattcctgcagcccgg

SEQ ID NO: 15 - DNA, 30 bp, Artificial Sequence
  pSGKP3'
actagtattatacctaggactgagctagct

SEQ ID NO: 16 - DNA, 23 bp, Artificial Sequence
  RNADNA5'
ttgacagctagctcagtcctagg

SEQ ID NO: 17 - DNA, 23 bp, Artificial Sequence
  RNADNA3'
ccgggctgcaggaattcgatatc

SEQ ID NO: 18 - DNA, 20 bp, Artificial Sequence
  lacZspacerDNA
atggcggttaacgccgcgga

SEQ ID NO: 19 - DNA, 24 bp, Artificial Sequence
  lacZ
aaacatggcggttaacgccgcgga

SEQ ID NO: 20 - DNA, 24 bp, Artificial Sequence
  lacZ
cgactccgcggcgttaaccgccat

SEQ ID NO: 21 - DNA, 24 bp, Artificial Sequence
  dhaK
aaacaggcggtgaccggcgaggcg

SEQ ID NO: 22 - DNA, 24 bp, Artificial Sequence
  dhaK
cgaccgcctcgccggtcaccgcct

SEQ ID NO: 23 - DNA, 24 bp, Artificial Sequence
  rpiR5
aaacgcggtgacgacccgctgcgt

SEQ ID NO: 24 - DNA, 24 bp, Artificial Sequence
  rpiR5
cgacacgcagcgggtcgtcaccgc

SEQ ID NO: 25 - DNA, 90 bp, Artificial Sequence
  lacZ
tgtcgttgcccaccgtcagccgttaggcaccccgacggtggatgatgtaccactggctgaagcgtaacgacccgacccgtccggtgcagt

SEQ ID NO: 26 - DNA, 90 bp, Artificial Sequence
  dhaK
gagcgacccggcgatccgggtggtggtccgtcgcgacctgaataagcgcgccgtctcggctacaacgtggaaatgctgatcgtcggcgac

SEQ ID NO: 27 - DNA, 90 bp, Artificial Sequence
  rpiR5
cgtattcgtcagcgctatcccaccctggcggcgagcgacaaaaaggatctggagcgggcgccggagcgcattcgccatagcgaagcgctg

SEQ ID NO: 28 - DNA, 20 bp, Artificial Sequence
  lacZPCR5'
atgtggcggatgagcggtat

SEQ ID NO: 29 - DNA, 20 bp, Artificial Sequence
  lacZPCR3'
ccagtaatcggcgaagttgc

SEQ ID NO: 30 - DNA, 20 bp, Artificial Sequence
  dhaKPCR5'
ctttgtccgttaccgctccg

SEQ ID NO: 31 - DNA, 20 bp, Artificial Sequence
  dhaKPCR3'
ggttgacgatgtccgcactg

SEQ ID NO: 32 - DNA, 22 bp, Artificial Sequence
  rpiR5PCR5'
ctgttgatgcaaggttccgtcc

SEQ ID NO: 33 - DNA, 20 bp, Artificial Sequence
  rpiR5PCR3'
ttctcgacgtgtgccggatc

SEQ ID NO: 34 - DNA, 271 bp, Artificial Sequence
  Synthetic DNA
ttaatacgactcactatagggaagcctgacataatttactctgtttcgcgcgccagggcagttaggtgccctaaaagagcgaagtggccgaaaggaaaggctaacgcttctctaacgctacggcgaccttggcgaaatgccatcaataccacgcggcccgaaagggttcgcgcgaaactgagtaataaaacattgcggatgcggcaatacagaaccgctgtcgcatcttgcgtaagcgcgtggattgaaacatggcggttaacgccgcgga

SEQ ID NO: 35 - protein, 422 aa, Artificial Sequence
  The amino acid sequence of the AsCas12f1 nuclease
MIKVYRYEIVKPLDLDWKEFGTILRQLQQETRFALNKATQLAWEWMGFSSDYKDNHGEYPKSKDILGYTNVHGYAYHTIKTKAYRLNSGNLSQTIKRATDRFKAYQKEILRGDMSIPSYKRDIPLDLIKENISVNRMNHGDYIASLSLLSNPAKQEMNVKRKISVIIIVRGAGKTIMDRILSGEYQVSASQIIHDDRKNKWYLNISYDFEPQTRVLDLNKIMGIDLGVAVAVYMAFQHTPARYKLEGGEIENFRRQVESRRISMLRQGKYAGGARGGHGRDKRIKPIEQLRDKIANFRDTTNHRYSRYIVDMAIKEGCGTIQMEDLTNIRDIGSRFLQNWTYYDLQQKIIYKAEEAGIKVIKIDPQYTSQRCSECGNIDSGNRIGQAIFKCRACGYEANADYNAARNIAIPNIDKIIAESIK

SEQ ID NO: 36 - DNA, 1266 bp, Artificial Sequence
  The coding gene sequence of AsCas12f1after condon optimization according to E. coli
atgatcaaagtttaccgttatgaaatcgttaaaccgctggacctggattggaaagaattcggcaccatcctgcgtcagctgcagcaggaaacccgcttcgcgctgaacaaagcaacccagctggcgtgggaatggatgggtttcagctctgattacaaagacaaccatggcgaatacccgaaaagcaaagacatcctgggctacaccaacgttcacggttacgcataccacaccatcaaaaccaaagcttatcgtctgaacagcggcaacctgagccagaccatcaaacgtgcgaccgatcgcttcaaagcgtaccagaaagaaatcctgcgtggtgacatgtccatcccgtcttacaaacgtgatatcccgctggatctgatcaaagaaaacatcagcgttaaccgtatgaaccacggtgattatatcgcttccctgtccctgctgtctaacccggcgaaacaggaaatgaacgttaaacgtaaaatctccgtgattatcatcgttcgtggcgcgggtaaaaccatcatggatcgcatcctgagcggcgaataccaggtgagcgcgagccagatcatccacgacgaccgtaaaaacaaatggtacctgaacatctcttatgatttcgaaccgcagacccgtgttctggatctgaacaaaatcatgggcatcgatctgggtgttgcggtggcggtgtacatggcgttccagcacaccccggcgcgctacaaactggaaggcggtgaaatcgaaaacttccgtcgtcaggtggagtctcgtcgcatctccatgctgcgccagggtaaatacgcgggtggtgctcgtggcggtcacggccgtgataaacgtatcaaaccgatcgaacagctgcgtgacaaaatcgctaacttccgcgataccactaaccaccgttactctcgttacatcgttgatatggctatcaaagaaggttgcggtaccattcagatggaagatctgaccaacatccgtgatatcggctctcgtttcctgcagaactggacctactacgatctgcagcagaaaatcatctacaaagcggaagaagcgggcatcaaagttatcaaaattgatccgcagtacaccagccagcgttgcagcgaatgcggcaacatcgattccggtaaccgtatcggtcaggcgatcttcaaatgccgtgcttgcggctacgaagcgaacgcggactacaacgcagctcgtaacatcgcgatcccgaacatcgataaaatcatcgcggaaagcatcaaa

SEQ ID NO: 37 - RNA, 171 nt, Artificial Sequence
  The backbone sequence of the guide RNA corresponding to the AsCas12f1 nuclease
auucgucgguucagcgacgauaagccgagaagugccaauaaaacuguuaagugguuugguaacgcucgguaagguagccaaaaggcugaaacuccgugcacaaagaccgcacggacgcuucacauauagcucauaaacaaggguuugcgagcuagcuuguggagugugaac

SEQ ID NO: 38 - DNA, 5010 bp, Artificial Sequence
  p15a-PAMdepletion
tggctggttggcgtactgttgtggtaaatacccatatggacagttttccctttgatatgtaacggtgaacagttgttctacttttgtttgttagtcttgatgcttcactgatagatacaagagcgtcgggtgatgctgccaacttactgatttagtgtatgatggtgtttttgaggtgctccagtggcttctgtttctatcagctgtccctcctgttcagctactgacggggtggtgcgtaacggcaaaagcaccgccggacatcagcgctagcggagtgtatactggcttactatgttggcactgatgagggtgtcagtgaagtgcttcatgtggcaggagaaaaaaggctgcaccggtgcgtcagcagaatatgtgatacaggatatattccgcttcctcgctcactgactcgctacgctcggtcgttcgactgcggcgagcggaaatggcttacgaacggggcggagatttcctggaagatgccaggaagatacttaacagggaagtgagagggccgcggcaaagccgtttttccataggctccgcccccctgacaagcatcacgaaatctgacgctcaaatcagtggtggcgaaacccgacaggactataaagataccaggcgtttccccctggcggctccctcgtgcgctctcctgttcctgcctttcggtttaccggtgtcattccgctgttatggccgcgtttgtctcattccacgcctgacactcagttccgggtaggcagttcgctccaagctggactgtatgcacgaaccccccgttcagtccgaccgctgcgccttatccggtaactatcgtcttgagtccaacccggaaagacatgcaaaagcaccactggcagcagccactggtaattgatttagaggagttagtcttgaagtcatgcgccggttaaggctaaactgaaaggacaagttttggtgactgcgctcctccaagccagttacctcggttcaaagagttggtagctcagagaaccttcgaaaaaccgccctgcaaggcggttttttcgttttcagagcaagagattacgcgcagaccaaaacgatctcaagaagatcatcttattaatcagataaaatatttctagatttcagtgcaatttatctcttcaaatgtagcacctgaagtcagccccatacgatataagttgtgacgtaaaatgagacgttgatcggcacgtaagaggttccaactttcaccataatgaaataagatcactaccgggcgtattttttgagttatcgagattttcaggagctaaggaagctaaaatggagaaaaaaatcactggatataccaccgttgatatatcccaatggcatcgtaaagaacattttgaggcatttcagtcagttgctcaatgtacctataaccagaccgttcagctgggtcatccaccggatcaattcccctgctcgcgcaggctgggtgccaagctctcgggtaacatcaaggcccgatccttggagcccttgccctcccgcacgatgatcgtgccgtgatcgaaatccagatccttgacccgcagttgcaaaccctcactgatccggctcacggtaactgatgccgtatttgcagtaccagcgtacggcccacagaatgatgtcacgctgaaaatgccggcctttgaatgggttcatgtgcagctccatcagcaaaaggggatgataagtttatcaccaccgactatttgcaacagtgccgttgatcgtgctatgatcgactgatgtcatcagcggtggagtgcaatgtcgtgcaatacgaatggcgaaaagccgagctcatcggtcagcttctcaaccttggggttacccccggcggtgtgctgctggtccacagctccttccgtagcgtccggcccctcgaagatgggccacttggactgatcgaggccctgcgtgctgcgctgggtccgggagggacgctcgtcatgccctcgtggtcaggtctggacgacgagccgttcgatcctgccacgtcgcccgttacaccggaccttggagttgtctctgacacattctggcgcctgccaaatgtaaagcgcagcgcccatccatttgcctttgcggcagcggggccacaggcagagcagatcatctctgatccattgcccctgccacctcactcgcctgcaagcccggtcgcccgtgtccatgaactcgatgggcaggtacttctcctcggcgtgggacacgatgccaacacgacgctgcatcttgccgagttgatggcaaaggttccctatggggtgccgagacactgcaccattcttcaggatggcaagttggtacgcgtcgattatctcgagaatgaccactgctgtgagcgctttgccttggcggacaggtggctcaaggagaagagccttcagaaggaaggtccagtcggtcatgcctttgctcggttgatccgctcccgcgacattgtggcgacagccctgggtcaactgggccgagatccgttgatcttcctgcatccgccagaggcgggatgcgaagaatgcgatgccgctcgccagtcgattggctgagctcatgagcggagaacgagatgacgttggaggggcaaggtcgcgctgattgctggggcaacacgtgaaaggcgagatcaccaaggtagtcggcaaataatgtctaacggtacccggggatcctctagagtcgacctgcataatgtgcctgtcaaatggacgaagcagggattctgcaaaccctatgctactccgtcaagccgtcaattgtctgattcgttaccaaaagcttgatatcttgacagctagctcagtcctaggtataatactagtattcgtcggttcagcgacgataagccgagaagtgccaataaaactgttaagtggtttggtaacgctcggtaaggtagccaaaaggctgaaactccgtgcacaaagaccgcacggacgcttcacatatagctcataaacaagggtttgcgagctagcttgtggagtgtgaactgtcctcttcctctttagcgggccggcatggtcccagcctcctcgctggcgccggctgggcaacatgcttcggcatggcgaatgggacgatctgacagctagcataaccccttggggcctctaaacgggtcttgaggggttttttggatatcgaattccgcatcctcacgataataagcttcctgctgaacatcaaaggcaagaaaacatctgttgtcaaagacagcatccttgaacaaggacaattaacagttaacaaataaaaacgcaaaagaaaatgccgatattgactaccggaagcagtgtgaccgtgtgcttctcaaatgcctgattcaggctgtctatgtgtgactgttgagctgtaacaagttgtctcaggtgttcaatttcatgttctagttgctttgttttactggtttcacctgttctattaggtgttacatgctgttcatctgttacattgtcgatctgttcatggtgaacagctttaaatgcaccaaaaactcgtaaaagctctgatgtatctatcttttttacaccgttttcatctgtgcatatagctatactgatttcgtcagactcacagtcaaacatgccggtcagttggcctggtgatggcgggatcgttgtatatttcttgacaccttttcggcaccgccctaaaattctgcgtcctcataatatatgaggcgatttattacgtgtttacgaagcaaaagctaaaaccaggagctatttaatgatcaaagtttaccgttatgaaatcgttaaaccgctggacctggattggaaagaattcggcaccatcctgcgtcagctgcagcaggaaacccgcttcgcgctgaacaaagcaacccagctggcgtgggaatggatgggtttcagctctgattacaaagacaaccatggcgaatacccgaaaagcaaagacatcctgggctacaccaacgttcacggttacgcataccacaccatcaaaaccaaagcttatcgtctgaacagcggcaacctgagccagaccatcaaacgtgcgaccgatcgcttcaaagcgtaccagaaagaaatcctgcgtggtgacatgtccatcccgtcttacaaacgtgatatcccgctggatctgatcaaagaaaacatcagcgttaaccgtatgaaccacggtgattatatcgcttccctgtccctgctgtctaacccggcgaaacaggaaatgaacgttaaacgtaaaatctccgtgattatcatcgttcgtggcgcgggtaaaaccatcatggatcgcatcctgagcggcgaataccaggtgagcgcgagccagatcatccacgacgaccgtaaaaacaaatggtacctgaacatctcttatgatttcgaaccgcagacccgtgttctggatctgaacaaaatcatgggcatcgatctgggtgttgcggtggcggtgtacatggcgttccagcacaccccggcgcgctacaaactggaaggcggtgaaatcgaaaacttccgtcgtcaggtggagtctcgtcgcatctccatgctgcgccagggtaaatacgcgggtggtgctcgtggcggtcacggccgtgataaacgtatcaaaccgatcgaacagctgcgtgacaaaatcgctaacttccgcgataccactaaccaccgttactctcgttacatcgttgatatggctatcaaagaaggttgcggtaccattcagatggaagatctgaccaacatccgtgatatcggctctcgtttcctgcagaactggacctactacgatctgcagcagaaaatcatctacaaagcggaagaagcgggcatcaaagttatcaaaattgatccgcagtacaccagccagcgttgcagcgaatgcggcaacatcgattccggtaaccgtatcggtcaggcgatcttcaaatgccgtgcttgcggctacgaagcgaacgcggactacaacgcagctcgtaacatcgcgatcccgaacatcgataaaatcatcgcggaaagcatcaaataa

SEQ ID NO: 39 - DNA, 2796 bp, Artificial Sequence
  p15a-backbone
tggctggttggcgtactgttgtggtaaatacccatatggacagttttccctttgatatgtaacggtgaacagttgttctacttttgtttgttagtcttgatgcttcactgatagatacaagagcgtcgggtgatgctgccaacttactgatttagtgtatgatggtgtttttgaggtgctccagtggcttctgtttctatcagctgtccctcctgttcagctactgacggggtggtgcgtaacggcaaaagcaccgccggacatcagcgctagcggagtgtatactggcttactatgttggcactgatgagggtgtcagtgaagtgcttcatgtggcaggagaaaaaaggctgcaccggtgcgtcagcagaatatgtgatacaggatatattccgcttcctcgctcactgactcgctacgctcggtcgttcgactgcggcgagcggaaatggcttacgaacggggcggagatttcctggaagatgccaggaagatacttaacagggaagtgagagggccgcggcaaagccgtttttccataggctccgcccccctgacaagcatcacgaaatctgacgctcaaatcagtggtggcgaaacccgacaggactataaagataccaggcgtttccccctggcggctccctcgtgcgctctcctgttcctgcctttcggtttaccggtgtcattccgctgttatggccgcgtttgtctcattccacgcctgacactcagttccgggtaggcagttcgctccaagctggactgtatgcacgaaccccccgttcagtccgaccgctgcgccttatccggtaactatcgtcttgagtccaacccggaaagacatgcaaaagcaccactggcagcagccactggtaattgatttagaggagttagtcttgaagtcatgcgccggttaaggctaaactgaaaggacaagttttggtgactgcgctcctccaagccagttacctcggttcaaagagttggtagctcagagaaccttcgaaaaaccgccctgcaaggcggttttttcgttttcagagcaagagattacgcgcagaccaaaacgatctcaagaagatcatcttattaatcagataaaatatttctagatttcagtgcaatttatctcttcaaatgtagcacctgaagtcagccccatacgatataagttgtgacgtaaaatgagacgttgatcggcacgtaagaggttccaactttcaccataatgaaataagatcactaccgggcgtattttttgagttatcgagattttcaggagctaaggaagctaaaatggagaaaaaaatcactggatataccaccgttgatatatcccaatggcatcgtaaagaacattttgaggcatttcagtcagttgctcaatgtacctataaccagaccgttcagctgggtcatccaccggatcaattcccctgctcgcgcaggctgggtgccaagctctcgggtaacatcaaggcccgatccttggagcccttgccctcccgcacgatgatcgtgccgtgatcgaaatccagatccttgacccgcagttgcaaaccctcactgatccggctcacggtaactgatgccgtatttgcagtaccagcgtacggcccacagaatgatgtcacgctgaaaatgccggcctttgaatgggttcatgtgcagctccatcagcaaaaggggatgataagtttatcaccaccgactatttgcaacagtgccgttgatcgtgctatgatcgactgatgtcatcagcggtggagtgcaatgtcgtgcaatacgaatggcgaaaagccgagctcatcggtcagcttctcaaccttggggttacccccggcggtgtgctgctggtccacagctccttccgtagcgtccggcccctcgaagatgggccacttggactgatcgaggccctgcgtgctgcgctgggtccgggagggacgctcgtcatgccctcgtggtcaggtctggacgacgagccgttcgatcctgccacgtcgcccgttacaccggaccttggagttgtctctgacacattctggcgcctgccaaatgtaaagcgcagcgcccatccatttgcctttgcggcagcggggccacaggcagagcagatcatctctgatccattgcccctgccacctcactcgcctgcaagcccggtcgcccgtgtccatgaactcgatgggcaggtacttctcctcggcgtgggacacgatgccaacacgacgctgcatcttgccgagttgatggcaaaggttccctatggggtgccgagacactgcaccattcttcaggatggcaagttggtacgcgtcgattatctcgagaatgaccactgctgtgagcgctttgccttggcggacaggtggctcaaggagaagagccttcagaaggaaggtccagtcggtcatgcctttgctcggttgatccgctcccgcgacattgtggcgacagccctgggtcaactgggccgagatccgttgatcttcctgcatccgccagaggcgggatgcgaagaatgcgatgccgctcgccagtcgattggctgagctcatgagcggagaacgagatgacgttggaggggcaaggtcgcgctgattgctggggcaacacgtgaaaggcgagatcaccaaggtagtcggcaaataatgtctaacggtacccggggatcctctagagtcgacctgcataatgtgcctgtcaaatggacgaagcagggattctgcaaaccctatgctactccgtcaagccgtcaattgtctgattcgttaccaaaagcttgatatc

SEQ ID NO: 40 - DNA, 1491 bp, Artificial Sequence
  rpsL-AsCas12fEc
accgttttcatctgtgcatatagctatactgatttcgtcagactcacagtcaaacatgccggtcagttggcctggtgatggcgggatcgttgtatatttcttgacaccttttcggcaccgccctaaaattctgcgtcctcataatatatgaggcgatttattacgtgtttacgaagcaaaagctaaaaccaggagctatttaatgatcaaagtttaccgttatgaaatcgttaaaccgctggacctggattggaaagaattcggcaccatcctgcgtcagctgcagcaggaaacccgcttcgcgctgaacaaagcaacccagctggcgtgggaatggatgggtttcagctctgattacaaagacaaccatggcgaatacccgaaaagcaaagacatcctgggctacaccaacgttcacggttacgcataccacaccatcaaaaccaaagcttatcgtctgaacagcggcaacctgagccagaccatcaaacgtgcgaccgatcgcttcaaagcgtaccagaaagaaatcctgcgtggtgacatgtccatcccgtcttacaaacgtgatatcccgctggatctgatcaaagaaaacatcagcgttaaccgtatgaaccacggtgattatatcgcttccctgtccctgctgtctaacccggcgaaacaggaaatgaacgttaaacgtaaaatctccgtgattatcatcgttcgtggcgcgggtaaaaccatcatggatcgcatcctgagcggcgaataccaggtgagcgcgagccagatcatccacgacgaccgtaaaaacaaatggtacctgaacatctcttatgatttcgaaccgcagacccgtgttctggatctgaacaaaatcatgggcatcgatctgggtgttgcggtggcggtgtacatggcgttccagcacaccccggcgcgctacaaactggaaggcggtgaaatcgaaaacttccgtcgtcaggtggagtctcgtcgcatctccatgctgcgccagggtaaatacgcgggtggtgctcgtggcggtcacggccgtgataaacgtatcaaaccgatcgaacagctgcgtgacaaaatcgctaacttccgcgataccactaaccaccgttactctcgttacatcgttgatatggctatcaaagaaggttgcggtaccattcagatggaagatctgaccaacatccgtgatatcggctctcgtttcctgcagaactggacctactacgatctgcagcagaaaatcatctacaaagcggaagaagcgggcatcaaagttatcaaaattgatccgcagtacaccagccagcgttgcagcgaatgcggcaacatcgattccggtaaccgtatcggtcaggcgatcttcaaatgccgtgcttgcggctacgaagcgaacgcggactacaacgcagctcgtaacatcgcgatcccgaacatcgataaaatcatcgcggaaagcatcaaataatggctggttggcgtactgtt

SEQ ID NO: 41 - DNA, 783 bp, Artificial Sequence
  8_AsCas12f_sgRNAv1_PAMdep
gttaccaaaagcttgatatcttgacagctagctcagtcctaggtataatactagtattcgtcggttcagcgacgataagccgagaagtgccaataaaactgttaagtggtttggtaacgctcggtaaggtagccaaaaggctgaaactccgtgcacaaagaccgcacggacgcttcacatatagctcataaacaagggtttgcgagctagcttgtggagtgtgaactgtcctcttcctctttagcgggccggcatggtcccagcctcctcgctggcgccggctgggcaacatgcttcggcatggcgaatgggacgatctgacagctagcataaccccttggggcctctaaacgggtcttgaggggttttttggatatcgaattccgcatcctcacgataataagcttcctgctgaacatcaaaggcaagaaaacatctgttgtcaaagacagcatccttgaacaaggacaattaacagttaacaaataaaaacgcaaaagaaaatgccgatattgactaccggaagcagtgtgaccgtgtgcttctcaaatgcctgattcaggctgtctatgtgtgactgttgagctgtaacaagttgtctcaggtgttcaatttcatgttctagttgctttgttttactggtttcacctgttctattaggtgttacatgctgttcatctgttacattgtcgatctgttcatggtgaacagctttaaatgcaccaaaaactcgtaaaagctctgatgtatctatcttttttacaccgttttcatctgtgcata

SEQ ID NO: 42 - DNA, 5007 bp, Artificial Sequence
  p15a-PAMcontrol
tggctggttggcgtactgttgtggtaaatacccatatggacagttttccctttgatatgtaacggtgaacagttgttctacttttgtttgttagtcttgatgcttcactgatagatacaagagcgtcgggtgatgctgccaacttactgatttagtgtatgatggtgtttttgaggtgctccagtggcttctgtttctatcagctgtccctcctgttcagctactgacggggtggtgcgtaacggcaaaagcaccgccggacatcagcgctagcggagtgtatactggcttactatgttggcactgatgagggtgtcagtgaagtgcttcatgtggcaggagaaaaaaggctgcaccggtgcgtcagcagaatatgtgatacaggatatattccgcttcctcgctcactgactcgctacgctcggtcgttcgactgcggcgagcggaaatggcttacgaacggggcggagatttcctggaagatgccaggaagatacttaacagggaagtgagagggccgcggcaaagccgtttttccataggctccgcccccctgacaagcatcacgaaatctgacgctcaaatcagtggtggcgaaacccgacaggactataaagataccaggcgtttccccctggcggctccctcgtgcgctctcctgttcctgcctttcggtttaccggtgtcattccgctgttatggccgcgtttgtctcattccacgcctgacactcagttccgggtaggcagttcgctccaagctggactgtatgcacgaaccccccgttcagtccgaccgctgcgccttatccggtaactatcgtcttgagtccaacccggaaagacatgcaaaagcaccactggcagcagccactggtaattgatttagaggagttagtcttgaagtcatgcgccggttaaggctaaactgaaaggacaagttttggtgactgcgctcctccaagccagttacctcggttcaaagagttggtagctcagagaaccttcgaaaaaccgccctgcaaggcggttttttcgttttcagagcaagagattacgcgcagaccaaaacgatctcaagaagatcatcttattaatcagataaaatatttctagatttcagtgcaatttatctcttcaaatgtagcacctgaagtcagccccatacgatataagttgtgacgtaaaatgagacgttgatcggcacgtaagaggttccaactttcaccataatgaaataagatcactaccgggcgtattttttgagttatcgagattttcaggagctaaggaagctaaaatggagaaaaaaatcactggatataccaccgttgatatatcccaatggcatcgtaaagaacattttgaggcatttcagtcagttgctcaatgtacctataaccagaccgttcagctgggtcatccaccggatcaattcccctgctcgcgcaggctgggtgccaagctctcgggtaacatcaaggcccgatccttggagcccttgccctcccgcacgatgatcgtgccgtgatcgaaatccagatccttgacccgcagttgcaaaccctcactgatccggctcacggtaactgatgccgtatttgcagtaccagcgtacggcccacagaatgatgtcacgctgaaaatgccggcctttgaatgggttcatgtgcagctccatcagcaaaaggggatgataagtttatcaccaccgactatttgcaacagtgccgttgatcgtgctatgatcgactgatgtcatcagcggtggagtgcaatgtcgtgcaatacgaatggcgaaaagccgagctcatcggtcagcttctcaaccttggggttacccccggcggtgtgctgctggtccacagctccttccgtagcgtccggcccctcgaagatgggccacttggactgatcgaggccctgcgtgctgcgctgggtccgggagggacgctcgtcatgccctcgtggtcaggtctggacgacgagccgttcgatcctgccacgtcgcccgttacaccggaccttggagttgtctctgacacattctggcgcctgccaaatgtaaagcgcagcgcccatccatttgcctttgcggcagcggggccacaggcagagcagatcatctctgatccattgcccctgccacctcactcgcctgcaagcccggtcgcccgtgtccatgaactcgatgggcaggtacttctcctcggcgtgggacacgatgccaacacgacgctgcatcttgccgagttgatggcaaaggttccctatggggtgccgagacactgcaccattcttcaggatggcaagttggtacgcgtcgattatctcgagaatgaccactgctgtgagcgctttgccttggcggacaggtggctcaaggagaagagccttcagaaggaaggtccagtcggtcatgcctttgctcggttgatccgctcccgcgacattgtggcgacagccctgggtcaactgggccgagatccgttgatcttcctgcatccgccagaggcgggatgcgaagaatgcgatgccgctcgccagtcgattggctgagctcatgagcggagaacgagatgacgttggaggggcaaggtcgcgctgattgctggggcaacacgtgaaaggcgagatcaccaaggtagtcggcaaataatgtctaacggtacccggggatcctctagagtcgacctgcataatgtgcctgtcaaatggacgaagcagggattctgcaaaccctatgctactccgtcaagccgtcaattgtctgattcgttaccaaaagcttgatatcttgacagctagctcagtcctaggtataatactagtattcgtcggttcagcgacgataagccgagaagtgccaataaaactgttaagtggtttggtaacgctcggtaaggtagccaaaaggctgaaactccgtgcacaaagaccgcacggacgcttcacatatagctcataaacaagggtttgcgagctagcttgtggagtgtgaaccgagaccattggtctcaggccggcatggtcccagcctcctcgctggcgccggctgggcaacatgcttcggcatggcgaatgggacgatctgacagctagcataaccccttggggcctctaaacgggtcttgaggggttttttggatatcgaattccgcatcctcacgataataagcttcctgctgaacatcaaaggcaagaaaacatctgttgtcaaagacagcatccttgaacaaggacaattaacagttaacaaataaaaacgcaaaagaaaatgccgatattgactaccggaagcagtgtgaccgtgtgcttctcaaatgcctgattcaggctgtctatgtgtgactgttgagctgtaacaagttgtctcaggtgttcaatttcatgttctagttgctttgttttactggtttcacctgttctattaggtgttacatgctgttcatctgttacattgtcgatctgttcatggtgaacagctttaaatgcaccaaaaactcgtaaaagctctgatgtatctatcttttttacaccgttttcatctgtgcatatagctatactgatttcgtcagactcacagtcaaacatgccggtcagttggcctggtgatggcgggatcgttgtatatttcttgacaccttttcggcaccgccctaaaattctgcgtcctcataatatatgaggcgatttattacgtgtttacgaagcaaaagctaaaaccaggagctatttaatgatcaaagtttaccgttatgaaatcgttaaaccgctggacctggattggaaagaattcggcaccatcctgcgtcagctgcagcaggaaacccgcttcgcgctgaacaaagcaacccagctggcgtgggaatggatgggtttcagctctgattacaaagacaaccatggcgaatacccgaaaagcaaagacatcctgggctacaccaacgttcacggttacgcataccacaccatcaaaaccaaagcttatcgtctgaacagcggcaacctgagccagaccatcaaacgtgcgaccgatcgcttcaaagcgtaccagaaagaaatcctgcgtggtgacatgtccatcccgtcttacaaacgtgatatcccgctggatctgatcaaagaaaacatcagcgttaaccgtatgaaccacggtgattatatcgcttccctgtccctgctgtctaacccggcgaaacaggaaatgaacgttaaacgtaaaatctccgtgattatcatcgttcgtggcgcgggtaaaaccatcatggatcgcatcctgagcggcgaataccaggtgagcgcgagccagatcatccacgacgaccgtaaaaacaaatggtacctgaacatctcttatgatttcgaaccgcagacccgtgttctggatctgaacaaaatcatgggcatcgatctgggtgttgcggtggcggtgtacatggcgttccagcacaccccggcgcgctacaaactggaaggcggtgaaatcgaaaacttccgtcgtcaggtggagtctcgtcgcatctccatgctgcgccagggtaaatacgcgggtggtgctcgtggcggtcacggccgtgataaacgtatcaaaccgatcgaacagctgcgtgacaaaatcgctaacttccgcgataccactaaccaccgttactctcgttacatcgttgatatggctatcaaagaaggttgcggtaccattcagatggaagatctgaccaacatccgtgatatcggctctcgtttcctgcagaactggacctactacgatctgcagcagaaaatcatctacaaagcggaagaagcgggcatcaaagttatcaaaattgatccgcagtacaccagccagcgttgcagcgaatgcggcaacatcgattccggtaaccgtatcggtcaggcgatcttcaaatgccgtgcttgcggctacgaagcgaacgcggactacaacgcagctcgtaacatcgcgatcccgaacatcgataaaatcatcgcggaaagcatcaaataa

SEQ ID NO: 43 - DNA, 780 bp, Artificial Sequence
  AsCas12f_sgRNAv1_PAMcontrol
gttaccaaaagcttgatatcttgacagctagctcagtcctaggtataatactagtattcgtcggttcagcgacgataagccgagaagtgccaataaaactgttaagtggtttggtaacgctcggtaaggtagccaaaaggctgaaactccgtgcacaaagaccgcacggacgcttcacatatagctcataaacaagggtttgcgagctagcttgtggagtgtgaaccgagaccattggtctcaggccggcatggtcccagcctcctcgctggcgccggctgggcaacatgcttcggcatggcgaatgggacgatctgacagctagcataaccccttggggcctctaaacgggtcttgaggggttttttggatatcgaattccgcatcctcacgataataagcttcctgctgaacatcaaaggcaagaaaacatctgttgtcaaagacagcatccttgaacaaggacaattaacagttaacaaataaaaacgcaaaagaaaatgccgatattgactaccggaagcagtgtgaccgtgtgcttctcaaatgcctgattcaggctgtctatgtgtgactgttgagctgtaacaagttgtctcaggtgttcaatttcatgttctagttgctttgttttactggtttcacctgttctattaggtgttacatgctgttcatctgttacattgtcgatctgttcatggtgaacagctttaaatgcaccaaaaactcgtaaaagctctgatgtatctatcttttttacaccgttttcatctgtgcata

SEQ ID NO: 44 - DNA, 2707 bp, Artificial Sequence
  pUC19-6N-library
  misc_feature (222)..(227): n is a, c, g, or t
attaatgcagctggcacgacaggtttcccgactggaaagcgggcagtgagcgcaacgcaattaatgtgagttagctcactcattaggcaccccaggctttacactttatgcttccggctcgtatgttgtgtggaattgtgagcggataacaatttcacacaggaaacagctatgaccatgattacgccaagcttgtgcacgccggcgacgttgggtcaactnnnnnntgtcctcttcctctttagcgtttagaatttgtcgaattcactggccgtcgttttacaacgtcgtgactgggaaaaccctggcgttacccaacttaatcgccttgcagcacatccccctttcgccagctggcgtaatagcgaagaggcccgcaccgatcgcccttcccaacagttgcgcagcctgaatggcgaatggcgcctgatgcggtattttctccttacgcatctgtgcggtatttcacaccgcatatggtgcactctcagtacaatctgctctgatgccgcatagttaagccagccccgacacccgccaacacccgctgacgcgccctgacgggcttgtctgctcccggcatccgcttacagacaagctgtgaccgtctccgggagctgcatgtgtcagaggttttcaccgtcatcaccgaaacgcgcgagacgaaagggcctcgtgatacgcctatttttataggttaatgtcatgataataatggtttcttagacgtcaggtggcacttttcggggaaatgtgcgcggaacccctatttgtttatttttctaaatacattcaaatatgtatccgctcatgagacaataaccctgataaatgcttcaataatattgaaaaaggaagagtatgagtattcaacatttccgtgtcgcccttattcccttttttgcggcattttgccttcctgtttttgctcacccagaaacgctggtgaaagtaaaagatgctgaagatcagttgggtgcacgagtgggttacatcgaactggatctcaacagcggtaagatccttgagagttttcgccccgaagaacgttttccaatgatgagcacttttaaagttctgctatgtggcgcggtattatcccgtattgacgccgggcaagagcaactcggtcgccgcatacactattctcagaatgacttggttgagtactcaccagtcacagaaaagcatcttacggatggcatgacagtaagagaattatgcagtgctgccataaccatgagtgataacactgcggccaacttacttctgacaacgatcggaggaccgaaggagctaaccgcttttttgcacaacatgggggatcatgtaactcgccttgatcgttgggaaccggagctgaatgaagccataccaaacgacgagcgtgacaccacgatgcctgtagcaatggcaacaacgttgcgcaaactattaactggcgaactacttactctagcttcccggcaacaattaatagactggatggaggcggataaagttgcaggaccacttctgcgctcggcccttccggctggctggtttattgctgataaatctggagccggtgagcgtgggtctcgcggtatcattgcagcactggggccagatggtaagccctcccgtatcgtagttatctacacgacggggagtcaggcaactatggatgaacgaaatagacagatcgctgagataggtgcctcactgattaagcattggtaactgtcagaccaagtttactcatatatactttagattgatttaaaacttcatttttaatttaaaaggatctaggtgaagatcctttttgataatctcatgaccaaaatcccttaacgtgagttttcgttccactgagcgtcagaccccgtagaaaagatcaaaggatcttcttgagatcctttttttctgcgcgtaatctgctgcttgcaaacaaaaaaaccaccgctaccagcggtggtttgtttgccggatcaagagctaccaactctttttccgaaggtaactggcttcagcagagcgcagataccaaatactgttcttctagtgtagccgtagttaggccaccacttcaagaactctgtagcaccgcctacatacctcgctctgctaatcctgttaccagtggctgctgccagtggcgataagtcgtgtcttaccgggttggactcaagacgatagttaccggataaggcgcagcggtcgggctgaacggggggttcgtgcacacagcccagcttggagcgaacgacctacaccgaactgagatacctacagcgtgagctatgagaaagcgccacgcttcccgaagggagaaaggcggacaggtatccggtaagcggcagggtcggaacaggagagcgcacgagggagcttccagggggaaacgcctggtatctttatagtcctgtcgggtttcgccacctctgacttgagcgtcgatttttgtgatgctcgtcaggggggcggagcctatggaaaaacgccagcaacgcggcctttttacggttcctggccttttgctggccttttgctcacatgttctttcctgcgttatcccctgattctgtggataaccgtattaccgcctttgagtgagctgataccgctcgccgcagccgaacgaccgagcgcagcgagtcagtgagcgaggaagcggaagagcgcccaatacgcaaaccgcctctccccgcgcgttggccgattc

SEQ ID NO: 45 - DNA, 46 bp, Artificial Sequence
  6N-F
  misc_feature (21)..(26): n is a, c, g, or t
ccggcgacgttgggtcaactnnnnnntgtcctcttcctctttagcg

SEQ ID NO: 46 - DNA, 30 bp, Artificial Sequence
  6N-R
agttgacccaacgtcgccggcgtgcacaag

SEQ ID NO: 47 - DNA, 51 bp, Artificial Sequence
  PAM-1F
gtgactggagttcagacgtgtgctcttccgatctcaggaaacagctatgac

SEQ ID NO: 48 - DNA, 43 bp, Artificial Sequence
  PAM-1R
gttcagagttctacagtccgacgatcgtaaaacgacggccagt

SEQ ID NO: 49 - DNA, 66 bp, Artificial Sequence
  PAM-2F
caagcagaagacggcatacgagatcggttcaagtgactggagttcagacgtgtgctcttccgatct

SEQ ID NO: 50 - DNA, 63 bp, Artificial Sequence
  PAM-2R
aatgatacggcgaccaccgagatctacacgctggattgttcagagttctacagtccgacgatc

SEQ ID NO: 51 - DNA, 6926 bp, Artificial Sequence
  pET28a-SUMO-AsCas12f
tggcgaatgggacgcgccctgtagcggcgcattaagcgcggcgggtgtggtggttacgcgcagcgtgaccgctacacttgccagcgccctagcgcccgctcctttcgctttcttcccttcctttctcgccacgttcgccggctttccccgtcaagctctaaatcgggggctccctttagggttccgatttagtgctttacggcacctcgaccccaaaaaacttgattagggtgatggttcacgtagtgggccatcgccctgatagacggtttttcgccctttgacgttggagtccacgttctttaatagtggactcttgttccaaactggaacaacactcaaccctatctcggtctattcttttgatttataagggattttgccgatttcggcctattggttaaaaaatgagctgatttaacaaaaatttaacgcgaattttaacaaaatattaacgtttacaatttcaggtggcacttttcggggaaatgtgcgcggaacccctatttgtttatttttctaaatacattcaaatatgtatccgctcatgaattaattcttagaaaaactcatcgagcatcaaatgaaactgcaatttattcatatcaggattatcaataccatatttttgaaaaagccgtttctgtaatgaaggagaaaactcaccgaggcagttccataggatggcaagatcctggtatcggtctgcgattccgactcgtccaacatcaatacaacctattaatttcccctcgtcaaaaataaggttatcaagtgagaaatcaccatgagtgacgactgaatccggtgagaatggcaaaagtttatgcatttctttccagacttgttcaacaggccagccattacgctcgtcatcaaaatcactcgcatcaaccaaaccgttattcattcgtgattgcgcctgagcgagacgaaatacgcgatcgctgttaaaaggacaattacaaacaggaatcgaatgcaaccggcgcaggaacactgccagcgcatcaacaatattttcacctgaatcaggatattcttctaatacctggaatgctgttttcccggggatcgcagtggtgagtaaccatgcatcatcaggagtacggataaaatgcttgatggtcggaagaggcataaattccgtcagccagtttagtctgaccatctcatctgtaacatcattggcaacgctacctttgccatgtttcagaaacaactctggcgcatcgggcttcccatacaatcgatagattgtcgcacctgattgcccgacattatcgcgagcccatttatacccatataaatcagcatccatgttggaatttaatcgcggcctagagcaagacgtttcccgttgaatatggctcataacaccccttgtattactgtttatgtaagcagacagttttattgttcatgaccaaaatcccttaacgtgagttttcgttccactgagcgtcagaccccgtagaaaagatcaaaggatcttcttgagatcctttttttctgcgcgtaatctgctgcttgcaaacaaaaaaaccaccgctaccagcggtggtttgtttgccggatcaagagctaccaactctttttccgaaggtaactggcttcagcagagcgcagataccaaatactgtccttctagtgtagccgtagttaggccaccacttcaagaactctgtagcaccgcctacatacctcgctctgctaatcctgttaccagtggctgctgccagtggcgataagtcgtgtcttaccgggttggactcaagacgatagttaccggataaggcgcagcggtcgggctgaacggggggttcgtgcacacagcccagcttggagcgaacgacctacaccgaactgagatacctacagcgtgagctatgagaaagcgccacgcttcccgaagggagaaaggcggacaggtatccggtaagcggcagggtcggaacaggagagcgcacgagggagcttccagggggaaacgcctggtatctttatagtcctgtcgggtttcgccacctctgacttgagcgtcgatttttgtgatgctcgtcaggggggcggagcctatggaaaaacgccagcaacgcggcctttttacggttcctggccttttgctggccttttgctcacatgttctttcctgcgttatcccctgattctgtggataaccgtattaccgcctttgagtgagctgataccgctcgccgcagccgaacgaccgagcgcagcgagtcagtgagcgaggaagcggaagagcgcctgatgcggtattttctccttacgcatctgtgcggtatttcacaccgcatatatggtgcactctcagtacaatctgctctgatgccgcatagttaagccagtatacactccgctatcgctacgtgactgggtcatggctgcgccccgacacccgccaacacccgctgacgcgccctgacgggcttgtctgctcccggcatccgcttacagacaagctgtgaccgtctccgggagctgcatgtgtcagaggttttcaccgtcatcaccgaaacgcgcgaggcagctgcggtaaagctcatcagcgtggtcgtgaagcgattcacagatgtctgcctgttcatccgcgtccagctcgttgagtttctccagaagcgttaatgtctggcttctgataaagcgggccatgttaagggcggttttttcctgtttggtcactgatgcctccgtgtaagggggatttctgttcatgggggtaatgataccgatgaaacgagagaggatgctcacgatacgggttactgatgatgaacatgcccggttactggaacgttgtgagggtaaacaactggcggtatggatgcggcgggaccagagaaaaatcactcagggtcaatgccagcgcttcgttaatacagatgtaggtgttccacagggtagccagcagcatcctgcgatgcagatccggaacataatggtgcagggcgctgacttccgcgtttccagactttacgaaacacggaaaccgaagaccattcatgttgttgctcaggtcgcagacgttttgcagcagcagtcgcttcacgttcgctcgcgtatcggtgattcattctgctaaccagtaaggcaaccccgccagcctagccgggtcctcaacgacaggagcacgatcatgcgcacccgtggggccgccatgccggcgataatggcctgcttctcgccgaaacgtttggtggcgggaccagtgacgaaggcttgagcgagggcgtgcaagattccgaataccgcaagcgacaggccgatcatcgtcgcgctccagcgaaagcggtcctcgccgaaaatgacccagagcgctgccggcacctgtcctacgagttgcatgataaagaagacagtcataagtgcggcgacgatagtcatgccccgcgcccaccggaaggagctgactgggttgaaggctctcaagggcatcggtcgagatcccggtgcctaatgagtgagctaacttacattaattgcgttgcgctcactgcccgctttccagtcgggaaacctgtcgtgccagctgcattaatgaatcggccaacgcgcggggagaggcggtttgcgtattgggcgccagggtggtttttcttttcaccagtgagacgggcaacagctgattgcccttcaccgcctggccctgagagagttgcagcaagcggtccacgctggtttgccccagcaggcgaaaatcctgtttgatggtggttaacggcgggatataacatgagctgtcttcggtatcgtcgtatcccactaccgagatatccgcaccaacgcgcagcccggactcggtaatggcgcgcattgcgcccagcgccatctgatcgttggcaaccagcatcgcagtgggaacgatgccctcattcagcatttgcatggtttgttgaaaaccggacatggcactccagtcgccttcccgttccgctatcggctgaatttgattgcgagtgagatatttatgccagccagccagacgcagacgcgccgagacagaacttaatgggcccgctaacagcgcgatttgctggtgacccaatgcgaccagatgctccacgcccagtcgcgtaccgtcttcatgggagaaaataatactgttgatgggtgtctggtcagagacatcaagaaataacgccggaacattagtgcaggcagcttccacagcaatggcatcctggtcatccagcggatagttaatgatcagcccactgacgcgttgcgcgagaagattgtgcaccgccgctttacaggcttcgacgccgcttcgttctaccatcgacaccaccacgctggcacccagttgatcggcgcgagatttaatcgccgcgacaatttgcgacggcgcgtgcagggccagactggaggtggcaacgccaatcagcaacgactgtttgcccgccagttgttgtgccacgcggttgggaatgtaattcagctccgccatcgccgcttccactttttcccgcgttttcgcagaaacgtggctggcctggttcaccacgcgggaaacggtctgataagagacaccggcatactctgcgacatcgtataacgttactggtttcacattcaccaccctgaattgactctcttccgggcgctatcatgccataccgcgaaaggttttgcgccattcgatggtgtccgggatctcgacgctctcccttatgcgactcctgcattaggaagcagcccagtagtaggttgaggccgttgagcaccgccgccgcaaggaatggtgcatgcaaggagatggcgcccaacagtcccccggccacggggcctgccaccatacccacgccgaaacaagcgctcatgagcccgaagtggcgagcccgatcttccccatcggtgatgtcggcgatataggcgccagcaaccgcacctgtggcgccggtgatgccggccacgatgcgtccggcgtagaggatcgagatctcgatcccgcgaaattaatacgactcactataggggaattgtgagcggataacaattcccctctagaaataattttgtttaactttaagaaggagatataccatgggcagcagccatcatcatcatcatcacagcagcggcctggtgccgcgcggcagcatgtcggactcagaagtcaatcaagaagctaagccagaggtcaagccagaagtcaagcctgagactcacatcaatttaaaggtgtccgatggatcttcagagatcttcttcaagatcaaaaagaccactcctttaagaaggctgatggaagcgttcgctaaaagacagggtaaggaaatggactccttaagattcttgtacgacggtattagaattcaagctgatcagacccctgaagatttggacatggaggataacgatattattgaggctcacagagaacagattggtggtcatagtagtcttgaagtcctctttcagggacccatgatcaaagtttaccgttatgaaatcgttaaaccgctggacctggattggaaagaattcggcaccatcctgcgtcagctgcagcaggaaacccgcttcgcgctgaacaaagcaacccagctggcgtgggaatggatgggtttcagctctgattacaaagacaaccatggcgaatacccgaaaagcaaagacatcctgggctacaccaacgttcacggttacgcataccacaccatcaaaaccaaagcttatcgtctgaacagcggcaacctgagccagaccatcaaacgtgcgaccgatcgcttcaaagcgtaccagaaagaaatcctgcgtggtgacatgtccatcccgtcttacaaacgtgatatcccgctggatctgatcaaagaaaacatcagcgttaaccgtatgaaccacggtgattatatcgcttccctgtccctgctgtctaacccggcgaaacaggaaatgaacgttaaacgtaaaatctccgtgattatcatcgttcgtggcgcgggtaaaaccatcatggatcgcatcctgagcggcgaataccaggtgagcgcgagccagatcatccacgacgaccgtaaaaacaaatggtacctgaacatctcttatgatttcgaaccgcagacccgtgttctggatctgaacaaaatcatgggcatcgatctgggtgttgcggtggcggtgtacatggcgttccagcacaccccggcgcgctacaaactggaaggcggtgaaatcgaaaacttccgtcgtcaggtggagtctcgtcgcatctccatgctgcgccagggtaaatacgcgggtggtgctcgtggcggtcacggccgtgataaacgtatcaaaccgatcgaacagctgcgtgacaaaatcgctaacttccgcgataccactaaccaccgttactctcgttacatcgttgatatggctatcaaagaaggttgcggtaccattcagatggaagatctgaccaacatccgtgatatcggctctcgtttcctgcagaactggacctactacgatctgcagcagaaaatcatctacaaagcggaagaagcgggcatcaaagttatcaaaattgatccgcagtacaccagccagcgttgcagcgaatgcggcaacatcgattccggtaaccgtatcggtcaggcgatcttcaaatgccgtgcttgcggctacgaagcgaacgcggactacaacgcagctcgtaacatcgcgatcccgaacatcgataaaatcatcgcggaaagcatcaaataagcttaagaattcgagctccgtcgacaagcttgcggccgcactcgagcaccaccaccaccaccactgagatccggctgctaacaaagcccgaaaggaagctgagttggctgctgccaccgctgagcaataactagcataaccccttggggcctctaaacgggtcttgaggggttttttgctgaaaggaggaactatatccggat

SEQ ID NO: 52 - DNA, 20 bp, Artificial Sequence
  28a-F
gcttaagaattcgagctccg

SEQ ID NO: 53 - DNA, 20 bp, Artificial Sequence
  28a-R
gctgccgcgcggcaccaggc

SEQ ID NO: 54 - DNA, 1636 bp, Artificial Sequence
  SUMO-AsCas12f
gcctggtgccgcgcggcagcatgtcggactcagaagtcaatcaagaagctaagccagaggtcaagccagaagtcaagcctgagactcacatcaatttaaaggtgtccgatggatcttcagagatcttcttcaagatcaaaaagaccactcctttaagaaggctgatggaagcgttcgctaaaagacagggtaaggaaatggactccttaagattcttgtacgacggtattagaattcaagctgatcagacccctgaagatttggacatggaggataacgatattattgaggctcacagagaacagattggtggtcatagtagtcttgaagtcctctttcagggacccatgatcaaagtttaccgttatgaaatcgttaaaccgctggacctggattggaaagaattcggcaccatcctgcgtcagctgcagcaggaaacccgcttcgcgctgaacaaagcaacccagctggcgtgggaatggatgggtttcagctctgattacaaagacaaccatggcgaatacccgaaaagcaaagacatcctgggctacaccaacgttcacggttacgcataccacaccatcaaaaccaaagcttatcgtctgaacagcggcaacctgagccagaccatcaaacgtgcgaccgatcgcttcaaagcgtaccagaaagaaatcctgcgtggtgacatgtccatcccgtcttacaaacgtgatatcccgctggatctgatcaaagaaaacatcagcgttaaccgtatgaaccacggtgattatatcgcttccctgtccctgctgtctaacccggcgaaacaggaaatgaacgttaaacgtaaaatctccgtgattatcatcgttcgtggcgcgggtaaaaccatcatggatcgcatcctgagcggcgaataccaggtgagcgcgagccagatcatccacgacgaccgtaaaaacaaatggtacctgaacatctcttatgatttcgaaccgcagacccgtgttctggatctgaacaaaatcatgggcatcgatctgggtgttgcggtggcggtgtacatggcgttccagcacaccccggcgcgctacaaactggaaggcggtgaaatcgaaaacttccgtcgtcaggtggagtctcgtcgcatctccatgctgcgccagggtaaatacgcgggtggtgctcgtggcggtcacggccgtgataaacgtatcaaaccgatcgaacagctgcgtgacaaaatcgctaacttccgcgataccactaaccaccgttactctcgttacatcgttgatatggctatcaaagaaggttgcggtaccattcagatggaagatctgaccaacatccgtgatatcggctctcgtttcctgcagaactggacctactacgatctgcagcagaaaatcatctacaaagcggaagaagcgggcatcaaagttatcaaaattgatccgcagtacaccagccagcgttgcagcgaatgcggcaacatcgattccggtaaccgtatcggtcaggcgatcttcaaatgccgtgcttgcggctacgaagcgaacgcggactacaacgcagctcgtaacatcgcgatcccgaacatcgataaaatcatcgcggaaagcatcaaataagcttaagaattcgagctccg

SEQ ID NO: 55 - DNA, 215 bp, Artificial Sequence
  sgRNAv1-pUC19
aagctaatacgactcactatagggattcgtcggttcagcgacgataagccgagaagtgccaataaaactgttaagtggtttggtaacgctcggtaaggtagccaaaaggctgaaactccgtgcacaaagaccgcacggacgcttcacatatagctcataaacaagggtttgcgagctagcttgtggagtgtgaacctggcgtttttccataggct

SEQ ID NO: 56 - DNA, 26 bp, Artificial Sequence
  UC-F
cagtctattaattgttgccgggaagc

SEQ ID NO: 57 - DNA, 23 bp, Artificial Sequence
  UC-R
gatggaggcggataaagttgcag

SEQ ID NO: 58 - DNA, 56 bp, Artificial Sequence
  56-bp DNA substrate
aaggccgcgttgctggcgtttttccataggctccgcccccctgacgagcatcacaa

SEQ ID NO: 59 - DNA, 36 bp, Artificial Sequence
  D225A-F
atcatgggcatcgctctgggtgttgcggtggcggtg

SEQ ID NO: 60 - DNA, 36 bp, Artificial Sequence
  D225A-R
acccagagcgatgcccatgattttgttcagatccag

SEQ ID NO: 61 - DNA, 35 bp, Artificial Sequence
  E324A-F
taccattcagatggcagatctgaccaacatccgtg

SEQ ID NO: 62 - DNA, 35 bp, Artificial Sequence
  E324A-R
ggtcagatctgccatctgaatggtaccgcaacctt

SEQ ID NO: 63 - DNA, 35 bp, Artificial Sequence
  R383A-F
tcgattccggtaacgctatcggtcaggcgatcttc

SEQ ID NO: 64 - DNA, 35 bp, Artificial Sequence
  R383A-R
ctgaccgatagcgttaccggaatcgatgttgccgc

SEQ ID NO: 65 - DNA, 37 bp, Artificial Sequence
  D401A-F
cgaagcgaacgcggcctacaacgcagctcgtaacatc

SEQ ID NO: 66 - DNA, 37 bp, Artificial Sequence
  D401A-R
cgttgtaggccgcgttcgcttcgtagccgcaagcacg

SEQ ID NO: 67 - DNA, 6926 bp, Artificial Sequence
  pET28a-SUMO-AsCas12f-D225A
tggcgaatgggacgcgccctgtagcggcgcattaagcgcggcgggtgtggtggttacgcgcagcgtgaccgctacacttgccagcgccctagcgcccgctcctttcgctttcttcccttcctttctcgccacgttcgccggctttccccgtcaagctctaaatcgggggctccctttagggttccgatttagtgctttacggcacctcgaccccaaaaaacttgattagggtgatggttcacgtagtgggccatcgccctgatagacggtttttcgccctttgacgttggagtccacgttctttaatagtggactcttgttccaaactggaacaacactcaaccctatctcggtctattcttttgatttataagggattttgccgatttcggcctattggttaaaaaatgagctgatttaacaaaaatttaacgcgaattttaacaaaatattaacgtttacaatttcaggtggcacttttcggggaaatgtgcgcggaacccctatttgtttatttttctaaatacattcaaatatgtatccgctcatgaattaattcttagaaaaactcatcgagcatcaaatgaaactgcaatttattcatatcaggattatcaataccatatttttgaaaaagccgtttctgtaatgaaggagaaaactcaccgaggcagttccataggatggcaagatcctggtatcggtctgcgattccgactcgtccaacatcaatacaacctattaatttcccctcgtcaaaaataaggttatcaagtgagaaatcaccatgagtgacgactgaatccggtgagaatggcaaaagtttatgcatttctttccagacttgttcaacaggccagccattacgctcgtcatcaaaatcactcgcatcaaccaaaccgttattcattcgtgattgcgcctgagcgagacgaaatacgcgatcgctgttaaaaggacaattacaaacaggaatcgaatgcaaccggcgcaggaacactgccagcgcatcaacaatattttcacctgaatcaggatattcttctaatacctggaatgctgttttcccggggatcgcagtggtgagtaaccatgcatcatcaggagtacggataaaatgcttgatggtcggaagaggcataaattccgtcagccagtttagtctgaccatctcatctgtaacatcattggcaacgctacctttgccatgtttcagaaacaactctggcgcatcgggcttcccatacaatcgatagattgtcgcacctgattgcccgacattatcgcgagcccatttatacccatataaatcagcatccatgttggaatttaatcgcggcctagagcaagacgtttcccgttgaatatggctcataacaccccttgtattactgtttatgtaagcagacagttttattgttcatgaccaaaatcccttaacgtgagttttcgttccactgagcgtcagaccccgtagaaaagatcaaaggatcttcttgagatcctttttttctgcgcgtaatctgctgcttgcaaacaaaaaaaccaccgctaccagcggtggtttgtttgccggatcaagagctaccaactctttttccgaaggtaactggcttcagcagagcgcagataccaaatactgtccttctagtgtagccgtagttaggccaccacttcaagaactctgtagcaccgcctacatacctcgctctgctaatcctgttaccagtggctgctgccagtggcgataagtcgtgtcttaccgggttggactcaagacgatagttaccggataaggcgcagcggtcgggctgaacggggggttcgtgcacacagcccagcttggagcgaacgacctacaccgaactgagatacctacagcgtgagctatgagaaagcgccacgcttcccgaagggagaaaggcggacaggtatccggtaagcggcagggtcggaacaggagagcgcacgagggagcttccagggggaaacgcctggtatctttatagtcctgtcgggtttcgccacctctgacttgagcgtcgatttttgtgatgctcgtcaggggggcggagcctatggaaaaacgccagcaacgcggcctttttacggttcctggccttttgctggccttttgctcacatgttctttcctgcgttatcccctgattctgtggataaccgtattaccgcctttgagtgagctgataccgctcgccgcagccgaacgaccgagcgcagcgagtcagtgagcgaggaagcggaagagcgcctgatgcggtattttctccttacgcatctgtgcggtatttcacaccgcatatatggtgcactctcagtacaatctgctctgatgccgcatagttaagccagtatacactccgctatcgctacgtgactgggtcatggctgcgccccgacacccgccaacacccgctgacgcgccctgacgggcttgtctgctcccggcatccgcttacagacaagctgtgaccgtctccgggagctgcatgtgtcagaggttttcaccgtcatcaccgaaacgcgcgaggcagctgcggtaaagctcatcagcgtggtcgtgaagcgattcacagatgtctgcctgttcatccgcgtccagctcgttgagtttctccagaagcgttaatgtctggcttctgataaagcgggccatgttaagggcggttttttcctgtttggtcactgatgcctccgtgtaagggggatttctgttcatgggggtaatgataccgatgaaacgagagaggatgctcacgatacgggttactgatgatgaacatgcccggttactggaacgttgtgagggtaaacaactggcggtatggatgcggcgggaccagagaaaaatcactcagggtcaatgccagcgcttcgttaatacagatgtaggtgttccacagggtagccagcagcatcctgcgatgcagatccggaacataatggtgcagggcgctgacttccgcgtttccagactttacgaaacacggaaaccgaagaccattcatgttgttgctcaggtcgcagacgttttgcagcagcagtcgcttcacgttcgctcgcgtatcggtgattcattctgctaaccagtaaggcaaccccgccagcctagccgggtcctcaacgacaggagcacgatcatgcgcacccgtggggccgccatgccggcgataatggcctgcttctcgccgaaacgtttggtggcgggaccagtgacgaaggcttgagcgagggcgtgcaagattccgaataccgcaagcgacaggccgatcatcgtcgcgctccagcgaaagcggtcctcgccgaaaatgacccagagcgctgccggcacctgtcctacgagttgcatgataaagaagacagtcataagtgcggcgacgatagtcatgccccgcgcccaccggaaggagctgactgggttgaaggctctcaagggcatcggtcgagatcccggtgcctaatgagtgagctaacttacattaattgcgttgcgctcactgcccgctttccagtcgggaaacctgtcgtgccagctgcattaatgaatcggccaacgcgcggggagaggcggtttgcgtattgggcgccagggtggtttttcttttcaccagtgagacgggcaacagctgattgcccttcaccgcctggccctgagagagttgcagcaagcggtccacgctggtttgccccagcaggcgaaaatcctgtttgatggtggttaacggcgggatataacatgagctgtcttcggtatcgtcgtatcccactaccgagatatccgcaccaacgcgcagcccggactcggtaatggcgcgcattgcgcccagcgccatctgatcgttggcaaccagcatcgcagtgggaacgatgccctcattcagcatttgcatggtttgttgaaaaccggacatggcactccagtcgccttcccgttccgctatcggctgaatttgattgcgagtgagatatttatgccagccagccagacgcagacgcgccgagacagaacttaatgggcccgctaacagcgcgatttgctggtgacccaatgcgaccagatgctccacgcccagtcgcgtaccgtcttcatgggagaaaataatactgttgatgggtgtctggtcagagacatcaagaaataacgccggaacattagtgcaggcagcttccacagcaatggcatcctggtcatccagcggatagttaatgatcagcccactgacgcgttgcgcgagaagattgtgcaccgccgctttacaggcttcgacgccgcttcgttctaccatcgacaccaccacgctggcacccagttgatcggcgcgagatttaatcgccgcgacaatttgcgacggcgcgtgcagggccagactggaggtggcaacgccaatcagcaacgactgtttgcccgccagttgttgtgccacgcggttgggaatgtaattcagctccgccatcgccgcttccactttttcccgcgttttcgcagaaacgtggctggcctggttcaccacgcgggaaacggtctgataagagacaccggcatactctgcgacatcgtataacgttactggtttcacattcaccaccctgaattgactctcttccgggcgctatcatgccataccgcgaaaggttttgcgccattcgatggtgtccgggatctcgacgctctcccttatgcgactcctgcattaggaagcagcccagtagtaggttgaggccgttgagcaccgccgccgcaaggaatggtgcatgcaaggagatggcgcccaacagtcccccggccacggggcctgccaccatacccacgccgaaacaagcgctcatgagcccgaagtggcgagcccgatcttccccatcggtgatgtcggcgatataggcgccagcaaccgcacctgtggcgccggtgatgccggccacgatgcgtccggcgtagaggatcgagatctcgatcccgcgaaattaatacgactcactataggggaattgtgagcggataacaattcccctctagaaataattttgtttaactttaagaaggagatataccatgggcagcagccatcatcatcatcatcacagcagcggcctggtgccgcgcggcagcatgtcggactcagaagtcaatcaagaagctaagccagaggtcaagccagaagtcaagcctgagactcacatcaatttaaaggtgtccgatggatcttcagagatcttcttcaagatcaaaaagaccactcctttaagaaggctgatggaagcgttcgctaaaagacaggggaaggaaatggactccttaagattcttgtacgacggtattagaattcaagctgatcagacccctgaagatttggacatggaggataacgatattattgaggctcacagagaaaagattggtggtcatagtagtcttgaagtcctctttcagggacccatgatcaaagtttaccgttatgaaatcgttaaaccgctggacctggattggaaagaattcggcaccatcctgcgtcagctgcagcaggaaacccgcttcgcgctgaacaaagcaacccagctggcgtgggaatggatgggtttcagctctgattacaaagacaaccatggcgaatacccgaaaagcaaagacatcctgggctacaccaacgttcacggttacgcataccacaccatcaaaaccaaagcttatcgtctgaacagcggcaacctgagccagaccatcaaacgtgcgaccgatcgcttcaaagcgtaccagaaagaaatcctgcgtggtgacatgtccatcccgtcttacaaacgtgatatcccgctggatctgatcaaagaaaacatcagcgttaaccgtatgaaccacggtgattatatcgcttccctgtccctgctgtctaacccggcgaaacaggaaatgaacgttaaacgtaaaatctccgtgattatcatcgttcgtggcgcgggtaaaaccatcatggatcgcatcctgagcggcgaataccaggtgagcgcgagccagatcatccacgacgaccgtaaaaacaaatggtacctgaacatctcttatgatttcgaaccgcagacccgtgttctggatctgaacaaaatcatgggcatcgctctgggtgttgcggtggcggtgtacatggcgttccagcacaccccggcgcgctacaaactggaaggcggtgaaatcgaaaacttccgtcgtcaggtggagtctcgtcgcatctccatgctgcgccagggtaaatacgcgggtggtgctcgtggcggtcacggccgtgataaacgtatcaaaccgatcgaacagctgcgtgacaaaatcgctaacttccgcgataccactaaccaccgttactctcgttacatcgttgatatggctatcaaagaaggttgcggtaccattcagatggaagatctgaccaacatccgtgatatcggctctcgtttcctgcagaactggacctactacgatctgcagcagaaaatcatctacaaagcggaagaagcgggcatcaaagttatcaaaattgatccgcagtacaccagccagcgttgcagcgaatgcggcaacatcgattccggtaaccgtatcggtcaggcgatcttcaaatgccgtgcttgcggctacgaagcgaacgcggactacaacgcagctcgtaacatcgcgatcccgaacatcgataaaatcatcgcggaaagcatcaaataagcttaagaattcgagctccgtcgacaagcttgcggccgcactcgagcaccaccaccaccaccactgagatccggctgctaacaaagcccgaaaggaagctgagttggctgctgccaccgctgagcaataactagcataaccccttggggcctctaaacgggtcttgaggggttttttgctgaaaggaggaactatatccggat

SEQ ID NO: 68 - DNA, 6926 bp, Artificial Sequence
  pET28a-SUMO-AsCas12f-E324A
tggcgaatgggacgcgccctgtagcggcgcattaagcgcggcgggtgtggtggttacgcgcagcgtgaccgctacacttgccagcgccctagcgcccgctcctttcgctttcttcccttcctttctcgccacgttcgccggctttccccgtcaagctctaaatcgggggctccctttagggttccgatttagtgctttacggcacctcgaccccaaaaaacttgattagggtgatggttcacgtagtgggccatcgccctgatagacggtttttcgccctttgacgttggagtccacgttctttaatagtggactcttgttccaaactggaacaacactcaaccctatctcggtctattcttttgatttataagggattttgccgatttcggcctattggttaaaaaatgagctgatttaacaaaaatttaacgcgaattttaacaaaatattaacgtttacaatttcaggtggcacttttcggggaaatgtgcgcggaacccctatttgtttatttttctaaatacattcaaatatgtatccgctcatgaattaattcttagaaaaactcatcgagcatcaaatgaaactgcaatttattcatatcaggattatcaataccatatttttgaaaaagccgtttctgtaatgaaggagaaaactcaccgaggcagttccataggatggcaagatcctggtatcggtctgcgattccgactcgtccaacatcaatacaacctattaatttcccctcgtcaaaaataaggttatcaagtgagaaatcaccatgagtgacgactgaatccggtgagaatggcaaaagtttatgcatttctttccagacttgttcaacaggccagccattacgctcgtcatcaaaatcactcgcatcaaccaaaccgttattcattcgtgattgcgcctgagcgagacgaaatacgcgatcgctgttaaaaggacaattacaaacaggaatcgaatgcaaccggcgcaggaacactgccagcgcatcaacaatattttcacctgaatcaggatattcttctaatacctggaatgctgttttcccggggatcgcagtggtgagtaaccatgcatcatcaggagtacggataaaatgcttgatggtcggaagaggcataaattccgtcagccagtttagtctgaccatctcatctgtaacatcattggcaacgctacctttgccatgtttcagaaacaactctggcgcatcgggcttcccatacaatcgatagattgtcgcacctgattgcccgacattatcgcgagcccatttatacccatataaatcagcatccatgttggaatttaatcgcggcctagagcaagacgtttcccgttgaatatggctcataacaccccttgtattactgtttatgtaagcagacagttttattgttcatgaccaaaatcccttaacgtgagttttcgttccactgagcgtcagaccccgtagaaaagatcaaaggatcttcttgagatcctttttttctgcgcgtaatctgctgcttgcaaacaaaaaaaccaccgctaccagcggtggtttgtttgccggatcaagagctaccaactctttttccgaaggtaactggcttcagcagagcgcagataccaaatactgtccttctagtgtagccgtagttaggccaccacttcaagaactctgtagcaccgcctacatacctcgctctgctaatcctgttaccagtggctgctgccagtggcgataagtcgtgtcttaccgggttggactcaagacgatagttaccggataaggcgcagcggtcgggctgaacggggggttcgtgcacacagcccagcttggagcgaacgacctacaccgaactgagatacctacagcgtgagctatgagaaagcgccacgcttcccgaagggagaaaggcggacaggtatccggtaagcggcagggtcggaacaggagagcgcacgagggagcttccagggggaaacgcctggtatctttatagtcctgtcgggtttcgccacctctgacttgagcgtcgatttttgtgatgctcgtcaggggggcggagcctatggaaaaacgccagcaacgcggcctttttacggttcctggccttttgctggccttttgctcacatgttctttcctgcgttatcccctgattctgtggataaccgtattaccgcctttgagtgagctgataccgctcgccgcagccgaacgaccgagcgcagcgagtcagtgagcgaggaagcggaagagcgcctgatgcggtattttctccttacgcatctgtgcggtatttcacaccgcatatatggtgcactctcagtacaatctgctctgatgccgcatagttaagccagtatacactccgctatcgctacgtgactgggtcatggctgcgccccgacacccgccaacacccgctgacgcgccctgacgggcttgtctgctcccggcatccgcttacagacaagctgtgaccgtctccgggagctgcatgtgtcagaggttttcaccgtcatcaccgaaacgcgcgaggcagctgcggtaaagctcatcagcgtggtcgtgaagcgattcacagatgtctgcctgttcatccgcgtccagctcgttgagtttctccagaagcgttaatgtctggcttctgataaagcgggccatgttaagggcggttttttcctgtttggtcactgatgcctccgtgtaagggggatttctgttcatgggggtaatgataccgatgaaacgagagaggatgctcacgatacgggttactgatgatgaacatgcccggttactggaacgttgtgagggtaaacaactggcggtatggatgcggcgggaccagagaaaaatcactcagggtcaatgccagcgcttcgttaatacagatgtaggtgttccacagggtagccagcagcatcctgcgatgcagatccggaacataatggtgcagggcgctgacttccgcgtttccagactttacgaaacacggaaaccgaagaccattcatgttgttgctcaggtcgcagacgttttgcagcagcagtcgcttcacgttcgctcgcgtatcggtgattcattctgctaaccagtaaggcaaccccgccagcctagccgggtcctcaacgacaggagcacgatcatgcgcacccgtggggccgccatgccggcgataatggcctgcttctcgccgaaacgtttggtggcgggaccagtgacgaaggcttgagcgagggcgtgcaagattccgaataccgcaagcgacaggccgatcatcgtcgcgctccagcgaaagcggtcctcgccgaaaatgacccagagcgctgccggcacctgtcctacgagttgcatgataaagaagacagtcataagtgcggcgacgatagtcatgccccgcgcccaccggaaggagctgactgggttgaaggctctcaagggcatcggtcgagatcccggtgcctaatgagtgagctaacttacattaattgcgttgcgctcactgcccgctttccagtcgggaaacctgtcgtgccagctgcattaatgaatcggccaacgcgcggggagaggcggtttgcgtattgggcgccagggtggtttttcttttcaccagtgagacgggcaacagctgattgcccttcaccgcctggccctgagagagttgcagcaagcggtccacgctggtttgccccagcaggcgaaaatcctgtttgatggtggttaacggcgggatataacatgagctgtcttcggtatcgtcgtatcccactaccgagatatccgcaccaacgcgcagcccggactcggtaatggcgcgcattgcgcccagcgccatctgatcgttggcaaccagcatcgcagtgggaacgatgccctcattcagcatttgcatggtttgttgaaaaccggacatggcactccagtcgccttcccgttccgctatcggctgaatttgattgcgagtgagatatttatgccagccagccagacgcagacgcgccgagacagaacttaatgggcccgctaacagcgcgatttgctggtgacccaatgcgaccagatgctccacgcccagtcgcgtaccgtcttcatgggagaaaataatactgttgatgggtgtctggtcagagacatcaagaaataacgccggaacattagtgcaggcagcttccacagcaatggcatcctggtcatccagcggatagttaatgatcagcccactgacgcgttgcgcgagaagattgtgcaccgccgctttacaggcttcgacgccgcttcgttctaccatcgacaccaccacgctggcacccagttgatcggcgcgagatttaatcgccgcgacaatttgcgacggcgcgtgcagggccagactggaggtggcaacgccaatcagcaacgactgtttgcccgccagttgttgtgccacgcggttgggaatgtaattcagctccgccatcgccgcttccactttttcccgcgttttcgcagaaacgtggctggcctggttcaccacgcgggaaacggtctgataagagacaccggcatactctgcgacatcgtataacgttactggtttcacattcaccaccctgaattgactctcttccgggcgctatcatgccataccgcgaaaggttttgcgccattcgatggtgtccgggatctcgacgctctcccttatgcgactcctgcattaggaagcagcccagtagtaggttgaggccgttgagcaccgccgccgcaaggaatggtgcatgcaaggagatggcgcccaacagtcccccggccacggggcctgccaccatacccacgccgaaacaagcgctcatgagcccgaagtggcgagcccgatcttccccatcggtgatgtcggcgatataggcgccagcaaccgcacctgtggcgccggtgatgccggccacgatgcgtccggcgtagaggatcgagatctcgatcccgcgaaattaatacgactcactataggggaattgtgagcggataacaattcccctctagaaataattttgtttaactttaagaaggagatataccatgggcagcagccatcatcatcatcatcacagcagcggcctggtgccgcgcggcagcatgtcggactcagaagtcaatcaagaagctaagccagaggtcaagccagaagtcaagcctgagactcacatcaatttaaaggtgtccgatggatcttcagagatcttcttcaagatcaaaaagaccactcctttaagaaggctgatggaagcgttcgctaaaagacaggggaaggaaatggactccttaagattcttgtacgacggtattagaattcaagctgatcagacccctgaagatttggacatggaggataacgatattattgaggctcacagagaaaagattggtggtcatagtagtcttgaagtcctctttcagggacccatgatcaaagtttaccgttatgaaatcgttaaaccgctggacctggattggaaagaattcggcaccatcctgcgtcagctgcagcaggaaacccgcttcgcgctgaacaaagcaacccagctggcgtgggaatggatgggtttcagctctgattacaaagacaaccatggcgaatacccgaaaagcaaagacatcctgggctacaccaacgttcacggttacgcataccacaccatcaaaaccaaagcttatcgtctgaacagcggcaacctgagccagaccatcaaacgtgcgaccgatcgcttcaaagcgtaccagaaagaaatcctgcgtggtgacatgtccatcccgtcttacaaacgtgatatcccgctggatctgatcaaagaaaacatcagcgttaaccgtatgaaccacggtgattatatcgcttccctgtccctgctgtctaacccggcgaaacaggaaatgaacgttaaacgtaaaatctccgtgattatcatcgttcgtggcgcgggtaaaaccatcatggatcgcatcctgagcggcgaataccaggtgagcgcgagccagatcatccacgacgaccgtaaaaacaaatggtacctgaacatctcttatgatttcgaaccgcagacccgtgttctggatctgaacaaaatcatgggcatcgatctgggtgttgcggtggcggtgtacatggcgttccagcacaccccggcgcgctacaaactggaaggcggtgaaatcgaaaacttccgtcgtcaggtggagtctcgtcgcatctccatgctgcgccagggtaaatacgcgggtggtgctcgtggcggtcacggccgtgataaacgtatcaaaccgatcgaacagctgcgtgacaaaatcgctaacttccgcgataccactaaccaccgttactctcgttacatcgttgatatggctatcaaagaaggttgcggtaccattcagatggcagatctgaccaacatccgtgatatcggctctcgtttcctgcagaactggacctactacgatctgcagcagaaaatcatctacaaagcggaagaagcgggcatcaaagttatcaaaattgatccgcagtacaccagccagcgttgcagcgaatgcggcaacatcgattccggtaaccgtatcggtcaggcgatcttcaaatgccgtgcttgcggctacgaagcgaacgcggactacaacgcagctcgtaacatcgcgatcccgaacatcgataaaatcatcgcggaaagcatcaaataagcttaagaattcgagctccgtcgacaagcttgcggccgcactcgagcaccaccaccaccaccactgagatccggctgctaacaaagcccgaaaggaagctgagttggctgctgccaccgctgagcaataactagcataaccccttggggcctctaaacgggtcttgaggggttttttgctgaaaggaggaactatatccggat

SEQ ID NO: 69 - DNA, 6926 bp, Artificial Sequence
  pET28a-SUMO-AsCas12f-R383A
tggcgaatgggacgcgccctgtagcggcgcattaagcgcggcgggtgtggtggttacgcgcagcgtgaccgctacacttgccagcgccctagcgcccgctcctttcgctttcttcccttcctttctcgccacgttcgccggctttccccgtcaagctctaaatcgggggctccctttagggttccgatttagtgctttacggcacctcgaccccaaaaaacttgattagggtgatggttcacgtagtgggccatcgccctgatagacggtttttcgccctttgacgttggagtccacgttctttaatagtggactcttgttccaaactggaacaacactcaaccctatctcggtctattcttttgatttataagggattttgccgatttcggcctattggttaaaaaatgagctgatttaacaaaaatttaacgcgaattttaacaaaatattaacgtttacaatttcaggtggcacttttcggggaaatgtgcgcggaacccctatttgtttatttttctaaatacattcaaatatgtatccgctcatgaattaattcttagaaaaactcatcgagcatcaaatgaaactgcaatttattcatatcaggattatcaataccatatttttgaaaaagccgtttctgtaatgaaggagaaaactcaccgaggcagttccataggatggcaagatcctggtatcggtctgcgattccgactcgtccaacatcaatacaacctattaatttcccctcgtcaaaaataaggttatcaagtgagaaatcaccatgagtgacgactgaatccggtgagaatggcaaaagtttatgcatttctttccagacttgttcaacaggccagccattacgctcgtcatcaaaatcactcgcatcaaccaaaccgttattcattcgtgattgcgcctgagcgagacgaaatacgcgatcgctgttaaaaggacaattacaaacaggaatcgaatgcaaccggcgcaggaacactgccagcgcatcaacaatattttcacctgaatcaggatattcttctaatacctggaatgctgttttcccggggatcgcagtggtgagtaaccatgcatcatcaggagtacggataaaatgcttgatggtcggaagaggcataaattccgtcagccagtttagtctgaccatctcatctgtaacatcattggcaacgctacctttgccatgtttcagaaacaactctggcgcatcgggcttcccatacaatcgatagattgtcgcacctgattgcccgacattatcgcgagcccatttatacccatataaatcagcatccatgttggaatttaatcgcggcctagagcaagacgtttcccgttgaatatggctcataacaccccttgtattactgtttatgtaagcagacagttttattgttcatgaccaaaatcccttaacgtgagttttcgttccactgagcgtcagaccccgtagaaaagatcaaaggatcttcttgagatcctttttttctgcgcgtaatctgctgcttgcaaacaaaaaaaccaccgctaccagcggtggtttgtttgccggatcaagagctaccaactctttttccgaaggtaactggcttcagcagagcgcagataccaaatactgtccttctagtgtagccgtagttaggccaccacttcaagaactctgtagcaccgcctacatacctcgctctgctaatcctgttaccagtggctgctgccagtggcgataagtcgtgtcttaccgggttggactcaagacgatagttaccggataaggcgcagcggtcgggctgaacggggggttcgtgcacacagcccagcttggagcgaacgacctacaccgaactgagatacctacagcgtgagctatgagaaagcgccacgcttcccgaagggagaaaggcggacaggtatccggtaagcggcagggtcggaacaggagagcgcacgagggagcttccagggggaaacgcctggtatctttatagtcctgtcgggtttcgccacctctgacttgagcgtcgatttttgtgatgctcgtcaggggggcggagcctatggaaaaacgccagcaacgcggcctttttacggttcctggccttttgctggccttttgctcacatgttctttcctgcgttatcccctgattctgtggataaccgtattaccgcctttgagtgagctgataccgctcgccgcagccgaacgaccgagcgcagcgagtcagtgagcgaggaagcggaagagcgcctgatgcggtattttctccttacgcatctgtgcggtatttcacaccgcatatatggtgcactctcagtacaatctgctctgatgccgcatagttaagccagtatacactccgctatcgctacgtgactgggtcatggctgcgccccgacacccgccaacacccgctgacgcgccctgacgggcttgtctgctcccggcatccgcttacagacaagctgtgaccgtctccgggagctgcatgtgtcagaggttttcaccgtcatcaccgaaacgcgcgaggcagctgcggtaaagctcatcagcgtggtcgtgaagcgattcacagatgtctgcctgttcatccgcgtccagctcgttgagtttctccagaagcgttaatgtctggcttctgataaagcgggccatgttaagggcggttttttcctgtttggtcactgatgcctccgtgtaagggggatttctgttcatgggggtaatgataccgatgaaacgagagaggatgctcacgatacgggttactgatgatgaacatgcccggttactggaacgttgtgagggtaaacaactggcggtatggatgcggcgggaccagagaaaaatcactcagggtcaatgccagcgcttcgttaatacagatgtaggtgttccacagggtagccagcagcatcctgcgatgcagatccggaacataatggtgcagggcgctgacttccgcgtttccagactttacgaaacacggaaaccgaagaccattcatgttgttgctcaggtcgcagacgttttgcagcagcagtcgcttcacgttcgctcgcgtatcggtgattcattctgctaaccagtaaggcaaccccgccagcctagccgggtcctcaacgacaggagcacgatcatgcgcacccgtggggccgccatgccggcgataatggcctgcttctcgccgaaacgtttggtggcgggaccagtgacgaaggcttgagcgagggcgtgcaagattccgaataccgcaagcgacaggccgatcatcgtcgcgctccagcgaaagcggtcctcgccgaaaatgacccagagcgctgccggcacctgtcctacgagttgcatgataaagaagacagtcataagtgcggcgacgatagtcatgccccgcgcccaccggaaggagctgactgggttgaaggctctcaagggcatcggtcgagatcccggtgcctaatgagtgagctaacttacattaattgcgttgcgctcactgcccgctttccagtcgggaaacctgtcgtgccagctgcattaatgaatcggccaacgcgcggggagaggcggtttgcgtattgggcgccagggtggtttttcttttcaccagtgagacgggcaacagctgattgcccttcaccgcctggccctgagagagttgcagcaagcggtccacgctggtttgccccagcaggcgaaaatcctgtttgatggtggttaacggcgggatataacatgagctgtcttcggtatcgtcgtatcccactaccgagatatccgcaccaacgcgcagcccggactcggtaatggcgcgcattgcgcccagcgccatctgatcgttggcaaccagcatcgcagtgggaacgatgccctcattcagcatttgcatggtttgttgaaaaccggacatggcactccagtcgccttcccgttccgctatcggctgaatttgattgcgagtgagatatttatgccagccagccagacgcagacgcgccgagacagaacttaatgggcccgctaacagcgcgatttgctggtgacccaatgcgaccagatgctccacgcccagtcgcgtaccgtcttcatgggagaaaataatactgttgatgggtgtctggtcagagacatcaagaaataacgccggaacattagtgcaggcagcttccacagcaatggcatcctggtcatccagcggatagttaatgatcagcccactgacgcgttgcgcgagaagattgtgcaccgccgctttacaggcttcgacgccgcttcgttctaccatcgacaccaccacgctggcacccagttgatcggcgcgagatttaatcgccgcgacaatttgcgacggcgcgtgcagggccagactggaggtggcaacgccaatcagcaacgactgtttgcccgccagttgttgtgccacgcggttgggaatgtaattcagctccgccatcgccgcttccactttttcccgcgttttcgcagaaacgtggctggcctggttcaccacgcgggaaacggtctgataagagacaccggcatactctgcgacatcgtataacgttactggtttcacattcaccaccctgaattgactctcttccgggcgctatcatgccataccgcgaaaggttttgcgccattcgatggtgtccgggatctcgacgctctcccttatgcgactcctgcattaggaagcagcccagtagtaggttgaggccgttgagcaccgccgccgcaaggaatggtgcatgcaaggagatggcgcccaacagtcccccggccacggggcctgccaccatacccacgccgaaacaagcgctcatgagcccgaagtggcgagcccgatcttccccatcggtgatgtcggcgatataggcgccagcaaccgcacctgtggcgccggtgatgccggccacgatgcgtccggcgtagaggatcgagatctcgatcccgcgaaattaatacgactcactataggggaattgtgagcggataacaattcccctctagaaataattttgtttaactttaagaaggagatataccatgggcagcagccatcatcatcatcatcacagcagcggcctggtgccgcgcggcagcatgtcggactcagaagtcaatcaagaagctaagccagaggtcaagccagaagtcaagcctgagactcacatcaatttaaaggtgtccgatggatcttcagagatcttcttcaagatcaaaaagaccactcctttaagaaggctgatggaagcgttcgctaaaagacaggggaaggaaatggactccttaagattcttgtacgacggtattagaattcaagctgatcagacccctgaagatttggacatggaggataacgatattattgaggctcacagagaaaagattggtggtcatagtagtcttgaagtcctctttcagggacccatgatcaaagtttaccgttatgaaatcgttaaaccgctggacctggattggaaagaattcggcaccatcctgcgtcagctgcagcaggaaacccgcttcgcgctgaacaaagcaacccagctggcgtgggaatggatgggtttcagctctgattacaaagacaaccatggcgaatacccgaaaagcaaagacatcctgggctacaccaacgttcacggttacgcataccacaccatcaaaaccaaagcttatcgtctgaacagcggcaacctgagccagaccatcaaacgtgcgaccgatcgcttcaaagcgtaccagaaagaaatcctgcgtggtgacatgtccatcccgtcttacaaacgtgatatcccgctggatctgatcaaagaaaacatcagcgttaaccgtatgaaccacggtgattatatcgcttccctgtccctgctgtctaacccggcgaaacaggaaatgaacgttaaacgtaaaatctccgtgattatcatcgttcgtggcgcgggtaaaaccatcatggatcgcatcctgagcggcgaataccaggtgagcgcgagccagatcatccacgacgaccgtaaaaacaaatggtacctgaacatctcttatgatttcgaaccgcagacccgtgttctggatctgaacaaaatcatgggcatcgatctgggtgttgcggtggcggtgtacatggcgttccagcacaccccggcgcgctacaaactggaaggcggtgaaatcgaaaacttccgtcgtcaggtggagtctcgtcgcatctccatgctgcgccagggtaaatacgcgggtggtgctcgtggcggtcacggccgtgataaacgtatcaaaccgatcgaacagctgcgtgacaaaatcgctaacttccgcgataccactaaccaccgttactctcgttacatcgttgatatggctatcaaagaaggttgcggtaccattcagatggaagatctgaccaacatccgtgatatcggctctcgtttcctgcagaactggacctactacgatctgcagcagaaaatcatctacaaagcggaagaagcgggcatcaaagttatcaaaattgatccgcagtacaccagccagcgttgcagcgaatgcggcaacatcgattccggtaacgctatcggtcaggcgatcttcaaatgccgtgcttgcggctacgaagcgaacgcggactacaacgcagctcgtaacatcgcgatcccgaacatcgataaaatcatcgcggaaagcatcaaataagcttaagaattcgagctccgtcgacaagcttgcggccgcactcgagcaccaccaccaccaccactgagatccggctgctaacaaagcccgaaaggaagctgagttggctgctgccaccgctgagcaataactagcataaccccttggggcctctaaacgggtcttgaggggttttttgctgaaaggaggaactatatccggat

SEQ ID NO: 70 - DNA, 6926 bp, Artificial Sequence
  pET28a-SUMO-AsCas12f-D401A
tggcgaatgggacgcgccctgtagcggcgcattaagcgcggcgggtgtggtggttacgcgcagcgtgaccgctacacttgccagcgccctagcgcccgctcctttcgctttcttcccttcctttctcgccacgttcgccggctttccccgtcaagctctaaatcgggggctccctttagggttccgatttagtgctttacggcacctcgaccccaaaaaacttgattagggtgatggttcacgtagtgggccatcgccctgatagacggtttttcgccctttgacgttggagtccacgttctttaatagtggactcttgttccaaactggaacaacactcaaccctatctcggtctattcttttgatttataagggattttgccgatttcggcctattggttaaaaaatgagctgatttaacaaaaatttaacgcgaattttaacaaaatattaacgtttacaatttcaggtggcacttttcggggaaatgtgcgcggaacccctatttgtttatttttctaaatacattcaaatatgtatccgctcatgaattaattcttagaaaaactcatcgagcatcaaatgaaactgcaatttattcatatcaggattatcaataccatatttttgaaaaagccgtttctgtaatgaaggagaaaactcaccgaggcagttccataggatggcaagatcctggtatcggtctgcgattccgactcgtccaacatcaatacaacctattaatttcccctcgtcaaaaataaggttatcaagtgagaaatcaccatgagtgacgactgaatccggtgagaatggcaaaagtttatgcatttctttccagacttgttcaacaggccagccattacgctcgtcatcaaaatcactcgcatcaaccaaaccgttattcattcgtgattgcgcctgagcgagacgaaatacgcgatcgctgttaaaaggacaattacaaacaggaatcgaatgcaaccggcgcaggaacactgccagcgcatcaacaatattttcacctgaatcaggatattcttctaatacctggaatgctgttttcccggggatcgcagtggtgagtaaccatgcatcatcaggagtacggataaaatgcttgatggtcggaagaggcataaattccgtcagccagtttagtctgaccatctcatctgtaacatcattggcaacgctacctttgccatgtttcagaaacaactctggcgcatcgggcttcccatacaatcgatagattgtcgcacctgattgcccgacattatcgcgagcccatttatacccatataaatcagcatccatgttggaatttaatcgcggcctagagcaagacgtttcccgttgaatatggctcataacaccccttgtattactgtttatgtaagcagacagttttattgttcatgaccaaaatcccttaacgtgagttttcgttccactgagcgtcagaccccgtagaaaagatcaaaggatcttcttgagatcctttttttctgcgcgtaatctgctgcttgcaaacaaaaaaaccaccgctaccagcggtggtttgtttgccggatcaagagctaccaactctttttccgaaggtaactggcttcagcagagcgcagataccaaatactgtccttctagtgtagccgtagttaggccaccacttcaagaactctgtagcaccgcctacatacctcgctctgctaatcctgttaccagtggctgctgccagtggcgataagtcgtgtcttaccgggttggactcaagacgatagttaccggataaggcgcagcggtcgggctgaacggggggttcgtgcacacagcccagcttggagcgaacgacctacaccgaactgagatacctacagcgtgagctatgagaaagcgccacgcttcccgaagggagaaaggcggacaggtatccggtaagcggcagggtcggaacaggagagcgcacgagggagcttccagggggaaacgcctggtatctttatagtcctgtcgggtttcgccacctctgacttgagcgtcgatttttgtgatgctcgtcaggggggcggagcctatggaaaaacgccagcaacgcggcctttttacggttcctggccttttgctggccttttgctcacatgttctttcctgcgttatcccctgattctgtggataaccgtattaccgcctttgagtgagctgataccgctcgccgcagccgaacgaccgagcgcagcgagtcagtgagcgaggaagcggaagagcgcctgatgcggtattttctccttacgcatctgtgcggtatttcacaccgcatatatggtgcactctcagtacaatctgctctgatgccgcatagttaagccagtatacactccgctatcgctacgtgactgggtcatggctgcgccccgacacccgccaacacccgctgacgcgccctgacgggcttgtctgctcccggcatccgcttacagacaagctgtgaccgtctccgggagctgcatgtgtcagaggttttcaccgtcatcaccgaaacgcgcgaggcagctgcggtaaagctcatcagcgtggtcgtgaagcgattcacagatgtctgcctgttcatccgcgtccagctcgttgagtttctccagaagcgttaatgtctggcttctgataaagcgggccatgttaagggcggttttttcctgtttggtcactgatgcctccgtgtaagggggatttctgttcatgggggtaatgataccgatgaaacgagagaggatgctcacgatacgggttactgatgatgaacatgcccggttactggaacgttgtgagggtaaacaactggcggtatggatgcggcgggaccagagaaaaatcactcagggtcaatgccagcgcttcgttaatacagatgtaggtgttccacagggtagccagcagcatcctgcgatgcagatccggaacataatggtgcagggcgctgacttccgcgtttccagactttacgaaacacggaaaccgaagaccattcatgttgttgctcaggtcgcagacgttttgcagcagcagtcgcttcacgttcgctcgcgtatcggtgattcattctgctaaccagtaaggcaaccccgccagcctagccgggtcctcaacgacaggagcacgatcatgcgcacccgtggggccgccatgccggcgataatggcctgcttctcgccgaaacgtttggtggcgggaccagtgacgaaggcttgagcgagggcgtgcaagattccgaataccgcaagcgacaggccgatcatcgtcgcgctccagcgaaagcggtcctcgccgaaaatgacccagagcgctgccggcacctgtcctacgagttgcatgataaagaagacagtcataagtgcggcgacgatagtcatgccccgcgcccaccggaaggagctgactgggttgaaggctctcaagggcatcggtcgagatcccggtgcctaatgagtgagctaacttacattaattgcgttgcgctcactgcccgctttccagtcgggaaacctgtcgtgccagctgcattaatgaatcggccaacgcgcggggagaggcggtttgcgtattgggcgccagggtggtttttcttttcaccagtgagacgggcaacagctgattgcccttcaccgcctggccctgagagagttgcagcaagcggtccacgctggtttgccccagcaggcgaaaatcctgtttgatggtggttaacggcgggatataacatgagctgtcttcggtatcgtcgtatcccactaccgagatatccgcaccaacgcgcagcccggactcggtaatggcgcgcattgcgcccagcgccatctgatcgttggcaaccagcatcgcagtgggaacgatgccctcattcagcatttgcatggtttgttgaaaaccggacatggcactccagtcgccttcccgttccgctatcggctgaatttgattgcgagtgagatatttatgccagccagccagacgcagacgcgccgagacagaacttaatgggcccgctaacagcgcgatttgctggtgacccaatgcgaccagatgctccacgcccagtcgcgtaccgtcttcatgggagaaaataatactgttgatgggtgtctggtcagagacatcaagaaataacgccggaacattagtgcaggcagcttccacagcaatggcatcctggtcatccagcggatagttaatgatcagcccactgacgcgttgcgcgagaagattgtgcaccgccgctttacaggcttcgacgccgcttcgttctaccatcgacaccaccacgctggcacccagttgatcggcgcgagatttaatcgccgcgacaatttgcgacggcgcgtgcagggccagactggaggtggcaacgccaatcagcaacgactgtttgcccgccagttgttgtgccacgcggttgggaatgtaattcagctccgccatcgccgcttccactttttcccgcgttttcgcagaaacgtggctggcctggttcaccacgcgggaaacggtctgataagagacaccggcatactctgcgacatcgtataacgttactggtttcacattcaccaccctgaattgactctcttccgggcgctatcatgccataccgcgaaaggttttgcgccattcgatggtgtccgggatctcgacgctctcccttatgcgactcctgcattaggaagcagcccagtagtaggttgaggccgttgagcaccgccgccgcaaggaatggtgcatgcaaggagatggcgcccaacagtcccccggccacggggcctgccaccatacccacgccgaaacaagcgctcatgagcccgaagtggcgagcccgatcttccccatcggtgatgtcggcgatataggcgccagcaaccgcacctgtggcgccggtgatgccggccacgatgcgtccggcgtagaggatcgagatctcgatcccgcgaaattaatacgactcactataggggaattgtgagcggataacaattcccctctagaaataattttgtttaactttaagaaggagatataccatgggcagcagccatcatcatcatcatcacagcagcggcctggtgccgcgcggcagcatgtcggactcagaagtcaatcaagaagctaagccagaggtcaagccagaagtcaagcctgagactcacatcaatttaaaggtgtccgatggatcttcagagatcttcttcaagatcaaaaagaccactcctttaagaaggctgatggaagcgttcgctaaaagacaggggaaggaaatggactccttaagattcttgtacgacggtattagaattcaagctgatcagacccctgaagatttggacatggaggataacgatattattgaggctcacagagaaaagattggtggtcatagtagtcttgaagtcctctttcagggacccatgatcaaagtttaccgttatgaaatcgttaaaccgctggacctggattggaaagaattcggcaccatcctgcgtcagctgcagcaggaaacccgcttcgcgctgaacaaagcaacccagctggcgtgggaatggatgggtttcagctctgattacaaagacaaccatggcgaatacccgaaaagcaaagacatcctgggctacaccaacgttcacggttacgcataccacaccatcaaaaccaaagcttatcgtctgaacagcggcaacctgagccagaccatcaaacgtgcgaccgatcgcttcaaagcgtaccagaaagaaatcctgcgtggtgacatgtccatcccgtcttacaaacgtgatatcccgctggatctgatcaaagaaaacatcagcgttaaccgtatgaaccacggtgattatatcgcttccctgtccctgctgtctaacccggcgaaacaggaaatgaacgttaaacgtaaaatctccgtgattatcatcgttcgtggcgcgggtaaaaccatcatggatcgcatcctgagcggcgaataccaggtgagcgcgagccagatcatccacgacgaccgtaaaaacaaatggtacctgaacatctcttatgatttcgaaccgcagacccgtgttctggatctgaacaaaatcatgggcatcgatctgggtgttgcggtggcggtgtacatggcgttccagcacaccccggcgcgctacaaactggaaggcggtgaaatcgaaaacttccgtcgtcaggtggagtctcgtcgcatctccatgctgcgccagggtaaatacgcgggtggtgctcgtggcggtcacggccgtgataaacgtatcaaaccgatcgaacagctgcgtgacaaaatcgctaacttccgcgataccactaaccaccgttactctcgttacatcgttgatatggctatcaaagaaggttgcggtaccattcagatggaagatctgaccaacatccgtgatatcggctctcgtttcctgcagaactggacctactacgatctgcagcagaaaatcatctacaaagcggaagaagcgggcatcaaagttatcaaaattgatccgcagtacaccagccagcgttgcagcgaatgcggcaacatcgattccggtaaccgtatcggtcaggcgatcttcaaatgccgtgcttgcggctacgaagcgaacgcggcctacaacgcagctcgtaacatcgcgatcccgaacatcgataaaatcatcgcggaaagcatcaaataagcttaagaattcgagctccgtcgacaagcttgcggccgcactcgagcaccaccaccaccaccactgagatccggctgctaacaaagcccgaaaggaagctgagttggctgctgccaccgctgagcaataactagcataaccccttggggcctctaaacgggtcttgaggggttttttgctgaaaggaggaactatatccggat

SEQ ID NO: 71 - DNA, 7767 bp, Artificial Sequence
  p15a-AsCas12f
tggctggttggcgtactgttgtggtaaatacccatatggacagttttccctttgatatgtaacggtgaacagttgttctacttttgtttgttagtcttgatgcttcactgatagatacaagagcgtcgggtgatgctgccaacttactgatttagtgtatgatggtgtttttgaggtgctccagtggcttctgtttctatcagctgtccctcctgttcagctactgacggggtggtgcgtaacggcaaaagcaccgccggacatcagcgctagcggagtgtatactggcttactatgttggcactgatgagggtgtcagtgaagtgcttcatgtggcaggagaaaaaaggctgcaccggtgcgtcagcagaatatgtgatacaggatatattccgcttcctcgctcactgactcgctacgctcggtcgttcgactgcggcgagcggaaatggcttacgaacggggcggagatttcctggaagatgccaggaagatacttaacagggaagtgagagggccgcggcaaagccgtttttccataggctccgcccccctgacaagcatcacgaaatctgacgctcaaatcagtggtggcgaaacccgacaggactataaagataccaggcgtttccccctggcggctccctcgtgcgctctcctgttcctgcctttcggtttaccggtgtcattccgctgttatggccgcgtttgtctcattccacgcctgacactcagttccgggtaggcagttcgctccaagctggactgtatgcacgaaccccccgttcagtccgaccgctgcgccttatccggtaactatcgtcttgagtccaacccggaaagacatgcaaaagcaccactggcagcagccactggtaattgatttagaggagttagtcttgaagtcatgcgccggttaaggctaaactgaaaggacaagttttggtgactgcgctcctccaagccagttacctcggttcaaagagttggtagctcagagaaccttcgaaaaaccgccctgcaaggcggttttttcgttttcagagcaagagattacgcgcagaccaaaacgatctcaagaagatcatcttattaatcagataaaatatttctagatttcagtgcaatttatctcttcaaatgtagcacctgaagtcagccccatacgatataagttgtgacgtaaaatgagacgttgatcggcacgtaagaggttccaactttcaccataatgaaataagatcactaccgggcgtattttttgagttatcgagattttcaggagctaaggaagctaaaatggagaaaaaaatcactggatataccaccgttgatatatcccaatggcatcgtaaagaacattttgaggcatttcagtcagttgctcaatgtacctataaccagaccgttcagctgggtcatccaccggatcaattcccctgctcgcgcaggctgggtgccaagctctcgggtaacatcaaggcccgatccttggagcccttgccctcccgcacgatgatcgtgccgtgatcgaaatccagatccttgacccgcagttgcaaaccctcactgatccggctcacggtaactgatgccgtatttgcagtaccagcgtacggcccacagaatgatgtcacgctgaaaatgccggcctttgaatgggttcatgtgcagctccatcagcaaaaggggatgataagtttatcaccaccgactatttgcaacagtgccgttgatcgtgctatgatcgactgatgtcatcagcggtggagtgcaatgtcgtgcaatacgaatggcgaaaagccgagctcatcggtcagcttctcaaccttggggttacccccggcggtgtgctgctggtccacagctccttccgtagcgtccggcccctcgaagatgggccacttggactgatcgaggccctgcgtgctgcgctgggtccgggagggacgctcgtcatgccctcgtggtcaggtctggacgacgagccgttcgatcctgccacgtcgcccgttacaccggaccttggagttgtctctgacacattctggcgcctgccaaatgtaaagcgcagcgcccatccatttgcctttgcggcagcggggccacaggcagagcagatcatctctgatccattgcccctgccacctcactcgcctgcaagcccggtcgcccgtgtccatgaactcgatgggcaggtacttctcctcggcgtgggacacgatgccaacacgacgctgcatcttgccgagttgatggcaaaggttccctatggggtgccgagacactgcaccattcttcaggatggcaagttggtacgcgtcgattatctcgagaatgaccactgctgtgagcgctttgccttggcggacaggtggctcaaggagaagagccttcagaaggaaggtccagtcggtcatgcctttgctcggttgatccgctcccgcgacattgtggcgacagccctgggtcaactgggccgagatccgttgatcttcctgcatccgccagaggcgggatgcgaagaatgcgatgccgctcgccagtcgattggctgagctcatgagcggagaacgagatgacgttggaggggcaaggtcgcgctgattgctggggcaacacgtgaaaggcgagatcaccaaggtagtcggcaaataatgtctaacggtacccggggatcctctagagtcgacctgcataatgtgcctgtcaaatggacgaagcagggattctgcaaaccctatgctactccgtcaagccgtcaattgtctgattcgttaccaattatgacaacttgacggctacatcattcactttttcttcacaaccggcacggaactcgctcgggctggccccggtgcattttttaaatacccgcgagaaatagagttgatcgtcaaaaccaacattgcgaccgacggtggcgataggcatccgggtggtgctcaaaagcagcttcgcctggctgatacgttggtcctcgcgccagcttaagacgctaatccctaactgctggcggaaaagatgtgacagacgcgacggcgacaagcaaacatgctgtgcgacgctggcgatatcaaaattgctgtctgccaggtgatcgctgatgtactgacaagcctcgcgtacccgattatccatcggtggatggagcgactcgttaatcgcttccatgcgccgcagtaacaattgctcaagcagatttatcgccagcagctccgaatagcgcccttccccttgcccggcgttaatgatttgcccaaacaggtcgctgaaatgcggctggtgcgcttcatccgggcgaaagaaccccgtattggcaaatattgacggccagttaagccattcatgccagtaggcgcgcggacgaaagtaaacccactggtgataccattcgcgagcctccggatgacgaccgtagtgatgaatctctcctggcgggaacagcaaaatatcacccggtcggcaaacaaattctcgtccctgatttttcaccaccccctgaccgcgaatggtgagattgagaatataacctttcattcccagcggtcggtcgataaaaaaatcgagataaccgttggcctcaatcggcgttaaacccgccaccagatgggcattaaacgagtatcccggcagcaggggatcattttgcgcttcagccatacttttcatactcccgccattcagagaagaaaccaattgtccatattgcatcagacattgccgtcactgcgtcttttactggctcttctcgctaaccaaaccggtaaccccgcttattaaaagcattctgtaacaaagcgggaccaaagccatgacaaaaacgcgtaacaaaagtgtctataatcacggcagaaaagtccacattgattatttgcacggcgtcacactttgctatgccatagcatttttatccataagattagcggatcctacctgacgctttttatcgcaactctctactgtttctccatacccgtttttttgggctagcgaaaagatgtttcgtgaagccgtcgacgcttataaaaaatggatattaatactgaaactgagatcaagcaaaagcattcactaaccccctttcctgttttcctaatcagcccggcatttcgcgggcgatattttcacagctatttcaggagttcagccatgaacgcttattacattcaggatcgtcttgaggctcagagctgggcgcgtcactaccagcagctcgcccgtgaagagaaagaggcagaactggcagacgacatggaaaaaggcctgccccagcacctgtttgaatcgctatgcatcgatcatttgcaacgccacggggccagcaaaaaatccattacccgtgcgtttgatgacgatgttgagtttcaggagcgcatggcagaacacatccggtacatggttgaaaccattgctcaccaccaggttgatattgattcagaggtataaaacgaatgagtactgcactcgcaacgctggctgggaagctggctgaacgtgtcggcatggattctgtcgacccacaggaactgatcaccactcttcgccagacggcatttaaaggtgatgccagcgatgcgcagttcatcgcattactgatcgttgccaaccagtacggccttaatccgtggacgaaagaaatttacgcctttcctgataagcagaatggcatcgttccggtggtgggcgttgatggctggtcccgcatcatcaatgaaaaccagcagtttgatggcatggactttgagcaggacaatgaatcctgtacatgccggatttaccgcaaggaccgtaatcatccgatctgcgttaccgaatggatggatgaatgccgccgcgaaccattcaaaactcgcgaaggcagagaaatcacggggccgtggcagtcgcatcccaaacggatgttacgtcataaagccatgattcagtgtgcccgtctggccttcggatttgctggtatctatgacaaggatgaagccgagcgcattgtcgaaaatactgcatacactgcagaacgtcagccggaacgcgacatcactccggttaacgatgaaaccatgcaggagattaacactctgctgatcgccctggataaaacatgggatgacgacttattgccgctctgttcccagatatttcgccgcgacattcgtgcatcgtcagaactgacacaggccgaagcagtaaaagctcttggattcctgaaacagaaagccgcagagcagaaggtggcagcatgacaccggacattatcctgcagcgtaccgggatcgatgtgagagctgtcgaacagggggatgatgcgtggcacaaattacggctcggcgtcatcaccgcttcagaagttcacaacgtgatagcaaaaccccgctccggaaagaagtggcctgacatgaaaatgtcctacttccacaccctgcttgctgaggtttgcaccggtgtggctccggaagttaacgctaaagcactggcctggggaaaacagtacgagaacgacgccagaaccctgtttgaattcacttccggcgtgaatgttactgaatccccgatcatctatcgcgacgaaagtatgcgtaccgcctgctctcccgatggtttatgcagtgacggcaacggccttgaactgaaatgcccgtttacctcccgggatttcatgaagttccggctcggtggtttcgaggccataaagtcagcttacatggcccaggtgcagtacagcatgtgggtgacgcgaaaaaatgcctggtactttgccaactatgacccgcgtatgaagcgtgaaggcctgcattatgtcgtgattgagcgggatgaaaagtacatggcgagttttgacgagatcgtgccggagttcatcgaaaaaatggacgaggcactggctgaaattggttttgtatttggggagcaatggcgatgacgcatcctcacgataataagcttcctgctgaacatcaaaggcaagaaaacatctgttgtcaaagacagcatccttgaacaaggacaattaacagttaacaaataaaaacgcaaaagaaaatgccgatattgactaccggaagcagtgtgaccgtgtgcttctcaaatgcctgattcaggctgtctatgtgtgactgttgagctgtaacaagttgtctcaggtgttcaatttcatgttctagttgctttgttttactggtttcacctgttctattaggtgttacatgctgttcatctgttacattgtcgatctgttcatggtgaacagctttaaatgcaccaaaaactcgtaaaagctctgatgtatctatcttttttacaccgttttcatctgtgcatatagctatactgatttcgtcagactcacagtcaaacatgccggtcagttggcctggtgatggcgggatcgttgtatatttcttgacaccttttcggcaccgccctaaaattctgcgtcctcataatatatgaggcgatttattacgtgtttacgaagcaaaagctaaaaccaggagctatttaatgatcaaagtttaccgttatgaaatcgttaaaccgctggacctggattggaaagaattcggcaccatcctgcgtcagctgcagcaggaaacccgcttcgcgctgaacaaagcaacccagctggcgtgggaatggatgggtttcagctctgattacaaagacaaccatggcgaatacccgaaaagcaaagacatcctgggctacaccaacgttcacggttacgcataccacaccatcaaaaccaaagcttatcgtctgaacagcggcaacctgagccagaccatcaaacgtgcgaccgatcgcttcaaagcgtaccagaaagaaatcctgcgtggtgacatgtccatcccgtcttacaaacgtgatatcccgctggatctgatcaaagaaaacatcagcgttaaccgtatgaaccacggtgattatatcgcttccctgtccctgctgtctaacccggcgaaacaggaaatgaacgttaaacgtaaaatctccgtgattatcatcgttcgtggcgcgggtaaaaccatcatggatcgcatcctgagcggcgaataccaggtgagcgcgagccagatcatccacgacgaccgtaaaaacaaatggtacctgaacatctcttatgatttcgaaccgcagacccgtgttctggatctgaacaaaatcatgggcatcgatctgggtgttgcggtggcggtgtacatggcgttccagcacaccccggcgcgctacaaactggaaggcggtgaaatcgaaaacttccgtcgtcaggtggagtctcgtcgcatctccatgctgcgccagggtaaatacgcgggtggtgctcgtggcggtcacggccgtgataaacgtatcaaaccgatcgaacagctgcgtgacaaaatcgctaacttccgcgataccactaaccaccgttactctcgttacatcgttgatatggctatcaaagaaggttgcggtaccattcagatggaagatctgaccaacatccgtgatatcggctctcgtttcctgcagaactggacctactacgatctgcagcagaaaatcatctacaaagcggaagaagcgggcatcaaagttatcaaaattgatccgcagtacaccagccagcgttgcagcgaatgcggcaacatcgattccggtaaccgtatcggtcaggcgatcttcaaatgccgtgcttgcggctacgaagcgaacgcggactacaacgcagctcgtaacatcgcgatcccgaacatcgataaaatcatcgcggaaagcatcaaataa

SEQ ID NO: 72 - DNA, 3552 bp, Artificial Sequence
  lambda-red
attgtctgattcgttaccaattatgacaacttgacggctacatcattcactttttcttcacaaccggcacggaactcgctcgggctggccccggtgcattttttaaatacccgcgagaaatagagttgatcgtcaaaaccaacattgcgaccgacggtggcgataggcatccgggtggtgctcaaaagcagcttcgcctggctgatacgttggtcctcgcgccagcttaagacgctaatccctaactgctggcggaaaagatgtgacagacgcgacggcgacaagcaaacatgctgtgcgacgctggcgatatcaaaattgctgtctgccaggtgatcgctgatgtactgacaagcctcgcgtacccgattatccatcggtggatggagcgactcgttaatcgcttccatgcgccgcagtaacaattgctcaagcagatttatcgccagcagctccgaatagcgcccttccccttgcccggcgttaatgatttgcccaaacaggtcgctgaaatgcggctggtgcgcttcatccgggcgaaagaaccccgtattggcaaatattgacggccagttaagccattcatgccagtaggcgcgcggacgaaagtaaacccactggtgataccattcgcgagcctccggatgacgaccgtagtgatgaatctctcctggcgggaacagcaaaatatcacccggtcggcaaacaaattctcgtccctgatttttcaccaccccctgaccgcgaatggtgagattgagaatataacctttcattcccagcggtcggtcgataaaaaaatcgagataaccgttggcctcaatcggcgttaaacccgccaccagatgggcattaaacgagtatcccggcagcaggggatcattttgcgcttcagccatacttttcatactcccgccattcagagaagaaaccaattgtccatattgcatcagacattgccgtcactgcgtcttttactggctcttctcgctaaccaaaccggtaaccccgcttattaaaagcattctgtaacaaagcgggaccaaagccatgacaaaaacgcgtaacaaaagtgtctataatcacggcagaaaagtccacattgattatttgcacggcgtcacactttgctatgccatagcatttttatccataagattagcggatcctacctgacgctttttatcgcaactctctactgtttctccatacccgtttttttgggctagcgaaaagatgtttcgtgaagccgtcgacgcttataaaaaatggatattaatactgaaactgagatcaagcaaaagcattcactaaccccctttcctgttttcctaatcagcccggcatttcgcgggcgatattttcacagctatttcaggagttcagccatgaacgcttattacattcaggatcgtcttgaggctcagagctgggcgcgtcactaccagcagctcgcccgtgaagagaaagaggcagaactggcagacgacatggaaaaaggcctgccccagcacctgtttgaatcgctatgcatcgatcatttgcaacgccacggggccagcaaaaaatccattacccgtgcgtttgatgacgatgttgagtttcaggagcgcatggcagaacacatccggtacatggttgaaaccattgctcaccaccaggttgatattgattcagaggtataaaacgaatgagtactgcactcgcaacgctggctgggaagctggctgaacgtgtcggcatggattctgtcgacccacaggaactgatcaccactcttcgccagacggcatttaaaggtgatgccagcgatgcgcagttcatcgcattactgatcgttgccaaccagtacggccttaatccgtggacgaaagaaatttacgcctttcctgataagcagaatggcatcgttccggtggtgggcgttgatggctggtcccgcatcatcaatgaaaaccagcagtttgatggcatggactttgagcaggacaatgaatcctgtacatgccggatttaccgcaaggaccgtaatcatccgatctgcgttaccgaatggatggatgaatgccgccgcgaaccattcaaaactcgcgaaggcagagaaatcacggggccgtggcagtcgcatcccaaacggatgttacgtcataaagccatgattcagtgtgcccgtctggccttcggatttgctggtatctatgacaaggatgaagccgagcgcattgtcgaaaatactgcatacactgcagaacgtcagccggaacgcgacatcactccggttaacgatgaaaccatgcaggagattaacactctgctgatcgccctggataaaacatgggatgacgacttattgccgctctgttcccagatatttcgccgcgacattcgtgcatcgtcagaactgacacaggccgaagcagtaaaagctcttggattcctgaaacagaaagccgcagagcagaaggtggcagcatgacaccggacattatcctgcagcgtaccgggatcgatgtgagagctgtcgaacagggggatgatgcgtggcacaaattacggctcggcgtcatcaccgcttcagaagttcacaacgtgatagcaaaaccccgctccggaaagaagtggcctgacatgaaaatgtcctacttccacaccctgcttgctgaggtttgcaccggtgtggctccggaagttaacgctaaagcactggcctggggaaaacagtacgagaacgacgccagaaccctgtttgaattcacttccggcgtgaatgttactgaatccccgatcatctatcgcgacgaaagtatgcgtaccgcctgctctcccgatggtttatgcagtgacggcaacggccttgaactgaaatgcccgtttacctcccgggatttcatgaagttccggctcggtggtttcgaggccataaagtcagcttacatggcccaggtgcagtacagcatgtgggtgacgcgaaaaaatgcctggtactttgccaactatgacccgcgtatgaagcgtgaaggcctgcattatgtcgtgattgagcgggatgaaaagtacatggcgagttttgacgagatcgtgccggagttcatcgaaaaaatggacgaggcactggctgaaattggttttgtatttggggagcaatggcgatgacgcatcctcacgataataagcttcctgctgaacatcaaaggcaagaaaacatctgttgtcaaagacagcatccttgaacaaggacaattaacagttaacaaataaaaacgcaaaagaaaatgccgatattgactaccggaagcagtgtgaccgtgtgcttctcaaatgcctgattcaggctgtctatgtgtgactgttgagctgtaacaagttgtctcaggtgttcaatttcatgttctagttgctttgttttactggtttcacctgttctattaggtgttacatgctgttcatctgttacattgtcgatctgttcatggtgaacagctttaaatgcaccaaaaactcgtaaaagctctgatgtatctatcttttttacaccgttttcatctgtgcata

SEQ ID NO: 73 - DNA, 4943 bp, Artificial Sequence
  psgRNAv1
tcttccgcttcctcgctcactgactcgctgcgctcggtcgttcggctgcggcgagcggtatcagctcactcaaaggcggtaatacggttatccacagaatcaggggataacgcaggaaagaacatgtgagcaaaaggccagcaaaaggccaggaaccgtaaaaaggccgcgttgctggcgtttttccataggctccgcccccctgacgagcatcacaaaaatcgacgctcaagtcagaggtggcgaaacccgacaggactataaagataccaggcgtttccccctggaagctccctcgtgcgctctcctgttccgaccctgccgcttaccggatacctgtccgcctttctcccttcgggaagcgtggcgctttctcatagctcacgctgtaggtatctcagttcggtgtaggtcgttcgctccaagctgggctgtgtgcacgaaccccccgttcagcccgaccgctgcgccttatccggtaactatcgtcttgagtccaacccggtaagacacgacttatcgccactggcagcagccactggtaacaggattagcagagcgaggtatgtaggcggtgctacagagttcttgaagtggtggcctaactacggctacactagaagaacagtatttggtatctgcgctctgctgaagccagttaccttcggaaaaagagttggtagctcttgatccggcaaacaaaccaccgctggtagcggtggtttttttgtttgcaagcagcagattacgcgcagaaaaaaaggatctcaagaagatcctttgatcttttctacggggtctgacgctcagtggaacgaaaactcacgttaagggattttggtcatgagattatcaaaaaggatcttcacctagatccttttaaattaaaaatgaagttttaaatcaatctaaagtatatatgagtaaacttggtctgacagttagaaaaactcatcgagcatcaaatgaaactgcaatttattcatatcaggattatcaataccatatttttgaaaaagccgtttctgtaatgaaggagaaaactcaccgaggcagttccataggatggcaagatcctggtatcggtctgcgattccgactcgtccaacatcaatacaacctattaatttcccctcgtcaaaaataaggttatcaagtgagaaatcaccatgagtgacgactgaatccggtgagaatggcaaaagtttatgcatttctttccagacttgttcaacaggccagccattacgctcgtcatcaaaatcactcgcatcaaccaaaccgttattcattcgtgattgcgcctgagcgagacgaaatacgcgatcgctgttaaaaggacaattacaaacaggaatcgaatgcaaccggcgcaggaacactgccagcgcatcaacaatattttcacctgaatcaggatattcttctaatacctggaatgctgttttcccagggatcgcagtggtgagtaaccatgcatcatcaggagtacggataaaatgcttgatggtcggaagaggcataaattccgtcagccagtttagtctgaccatctcatctgtaacatcattggcaacgctacctttgccatgtttcagaaacaactctggcgcatcgggcttcccatacaatcgatagattgtcgcacctgattgcccgacattatcgcgagcccatttatacccatataaatcagcatccatgttggaatttaatcgcggcctagagcaagacgtttcccgttgaatatggctcatactcttcctttttcaatattattgaagcatttatcagggttattgtctcatgagcggatacatatttgaatgtatttagaaaaataaacaaataggggttccgcgcacatttccccgaaaagtgccacctgacgtctaagaaaccattattatcatgacattaacctataaaaataggcgtatcacgaggccctttcgtctcgcgcgtttcggtgatgacggtgaaaacctctgacacatgcagctcccggagacggtcacagcttgtctgtaagcggatgccgggagcagacaagcccgtcagggcgcgtcagcgggtgttggcgggtgtcggggctggcttaactatgcggcatcagagcagattgtactgagagtgcaccatatgcggtgtgaaataccgcacagatgcgtaaggagaaaataccgcatcaggcgccattcgccattcaggctgcgcaactgttgggaagggcgatcggtgcgggcctcttcgctattacgccagctggcgaaagggggatgtgctgcaaggcgattaagttgggtaacgccagggttttcccagtcacgacgttgtaaaacgacggccagtgaattgacgcgtattgggatggtaccgggccccccctcgaggtcgacggtatcgatacggcatcagagcagattgtactgagagtgcaccataatcggcattttcttttgcgtttttatttgttaactgttaattgtccttgttcaaggatgctgtctttgacaacagatgttttcttgcctttgatgttcagcaggaagctaggcgcaaacgttgattgtttgtctgcgtagaatcctctgtttgtcatatagcttgtaatcacgacattgtttcctttcgcttgaggtacagcgaagtgtgagtaagtaaaggttacatcgttaggatcaagatccatttttaacacaaggccagttttgttcagcggcttgtatgggccagttaaagaattagaaacataaccaagcatgtaaatatcgttagacgtaatgccgtcaatcgtcatttttgatccgcgggagtcagtgaacagataccatttgccgttcattttaaagacgttcgcgcgttcaatttcatctgttactgtgttagatgcaatcagcggtttcatcacttttttcagtgtgtaatcatcgtttagctcaatcataccgagagcgccgtttgctaactcagccgtgcgttttttatcgctttgcagaagtttttgactttcttgacggaagaatgatgtgcttttgccatagtatgctttgttaaataaagattcttcgccttggtagccatcttcagttccagtgtttgcttcaaatactaagtatttgtggcctttatcttctacgtagtgaggatctctcagcgtatggttgtcgcctgagctgtagttgccttcatcgatgaactgctgtacattttgatacgtttttccgtcaccgtcaaagattgatttataatcctctacaccgttgatgttcaaagagctgtctgatgctgatacgttaacttgtgcagttgtcagtgtttgtttgccgtaatgtttaccggagaaatcagtgtagaataaacggatttttccgtcagatgtaaatgtggctgaacctgaccattcttgtgtttggtcttttaggatagaatcatttgcatcgaatttgtcgctgtctttaaagacgcggccagcgtttttccagctgtcaatagaagtttcgccgactttttgatagaacatgtaaatcgatgtgtcatccgcatttttaggatctccggctaatgcaaagacgatgtggtagccgtgatagtttgcgacagtgccgtcagcgttttgtaatggccagctgtcccaaacgtccaggccttttgcagaagagatatttttaattgtggacgaatcgaactcaggaacttgatatttttcatttttttgctgttcagggatttgcagcatatcatggcgtgtaatatgggaaatgccgtatgtttccttatatggcttttggttcgtttctttcgcaaacgcttgagttgcgcctcctgccagcagtgcggtagtaaaggttaatactgttgcttgttttgcaaactttttgatgttcatcgttcatgtctccttttttatgtactgtgttagcggtctgcttcttccagccctcctgtttgaagatggcaagttagttacgcacaataaaaaaagacctaaaatatgtaaggggtgacgccaaagtatacactttgccctttacacattttaggtcttgcctgctttatcagtaacaaacccgcgcgatttacttttcgacctcattctattagactctcgtttggattgcaactggtctattttcctcttttgtttgatagaaaatcataaaaggatttgcagactacgggcctaaagaactaaaaaatctatctgtttcttttcattctctgtattttttatagtttctgttgcatgggcataaagttgcaagcttgatatcttgacagctagctcagtcctaggtataatactagtattcgtcggttcagcgacgataagccgagaagtgccaataaaactgttaagtggtttggtaacgctcggtaaggtagccaaaaggctgaaactccgtgcacaaagaccgcacggacgcttcacatatagctcataaacaagggtttgcgagctagcttgtggagtgtgaaccgagaccattggtctcaggccggcatggtcccagcctcctcgctggcgccggctgggcaacatgcttcggcatggcgaatgggacgatctgacagctagcataaccccttggggcctctaaacgggtcttgaggggttttttggatatcgaattcctgcagcccgggggatccactagttctagagcggccgccaccgcggtggagctcatcccaatggcgcgccgagcttggctcgagcatggtcatagctgtttcctgtgtgaaattgttatccgctcacaattccacacaacatacgagccggaagcataaagtgtaaagcctggggtgcctaatgagtgagctaactcacattaattgcgttgcgctcactgcccgctttccagtcgggaaacctgtcgtgccagctgcattaatgaatcggccaacgcgcggggagaggcggtttgcgtattgggcgc

SEQ ID NO: 74 - DNA, 20 bp, Artificial Sequence
  SGKP-F
gatctgacagctagcataac

SEQ ID NO: 75 - DNA, 20 bp, Artificial Sequence
  SGKP-R
gatatcaagcttgcaacttt

SEQ ID NO: 76 - DNA, 331 bp, Artificial Sequence
  sgRNAv1-2Bsa1
aaagttgcaagcttgatatcttgacagctagctcagtcctaggtataatactagtattcgtcggttcagcgacgataagccgagaagtgccaataaaactgttaagtggtttggtaacgctcggtaaggtagccaaaaggctgaaactccgtgcacaaagaccgcacggacgcttcacatatagctcataaacaagggtttgcgagctagcttgtggagtgtgaaccgagaccattggtctcaggccggcatggtcccagcctcctcgctggcgccggctgggcaacatgcttcggcatggcgaatgggacgatctgacagctagcataac

SEQ ID NO: 77 - DNA, 24 bp, Artificial Sequence
  hisD-F
gaacctgacgcccgatgctgatat

SEQ ID NO: 78 - DNA, 24 bp, Artificial Sequence
  hisD-R
ggccatatcagcatcgggcgtcag

SEQ ID NO: 79 - DNA, 24 bp, Artificial Sequence
  pyrF-F
gaacagtttcacgatattcccaac

SEQ ID NO: 80 - DNA, 24 bp, Artificial Sequence
  pyrF-R
ggccgttgggaatatcgtgaaact

SEQ ID NO: 81 - DNA, 4946 bp, Artificial Sequence
  psgRNAv1-hisD
tcttccgcttcctcgctcactgactcgctgcgctcggtcgttcggctgcggcgagcggtatcagctcactcaaaggcggtaatacggttatccacagaatcaggggataacgcaggaaagaacatgtgagcaaaaggccagcaaaaggccaggaaccgtaaaaaggccgcgttgctggcgtttttccataggctccgcccccctgacgagcatcacaaaaatcgacgctcaagtcagaggtggcgaaacccgacaggactataaagataccaggcgtttccccctggaagctccctcgtgcgctctcctgttccgaccctgccgcttaccggatacctgtccgcctttctcccttcgggaagcgtggcgctttctcatagctcacgctgtaggtatctcagttcggtgtaggtcgttcgctccaagctgggctgtgtgcacgaaccccccgttcagcccgaccgctgcgccttatccggtaactatcgtcttgagtccaacccggtaagacacgacttatcgccactggcagcagccactggtaacaggattagcagagcgaggtatgtaggcggtgctacagagttcttgaagtggtggcctaactacggctacactagaagaacagtatttggtatctgcgctctgctgaagccagttaccttcggaaaaagagttggtagctcttgatccggcaaacaaaccaccgctggtagcggtggtttttttgtttgcaagcagcagattacgcgcagaaaaaaaggatctcaagaagatcctttgatcttttctacggggtctgacgctcagtggaacgaaaactcacgttaagggattttggtcatgagattatcaaaaaggatcttcacctagatccttttaaattaaaaatgaagttttaaatcaatctaaagtatatatgagtaaacttggtctgacagttagaaaaactcatcgagcatcaaatgaaactgcaatttattcatatcaggattatcaataccatatttttgaaaaagccgtttctgtaatgaaggagaaaactcaccgaggcagttccataggatggcaagatcctggtatcggtctgcgattccgactcgtccaacatcaatacaacctattaatttcccctcgtcaaaaataaggttatcaagtgagaaatcaccatgagtgacgactgaatccggtgagaatggcaaaagtttatgcatttctttccagacttgttcaacaggccagccattacgctcgtcatcaaaatcactcgcatcaaccaaaccgttattcattcgtgattgcgcctgagcgagacgaaatacgcgatcgctgttaaaaggacaattacaaacaggaatcgaatgcaaccggcgcaggaacactgccagcgcatcaacaatattttcacctgaatcaggatattcttctaatacctggaatgctgttttcccagggatcgcagtggtgagtaaccatgcatcatcaggagtacggataaaatgcttgatggtcggaagaggcataaattccgtcagccagtttagtctgaccatctcatctgtaacatcattggcaacgctacctttgccatgtttcagaaacaactctggcgcatcgggcttcccatacaatcgatagattgtcgcacctgattgcccgacattatcgcgagcccatttatacccatataaatcagcatccatgttggaatttaatcgcggcctagagcaagacgtttcccgttgaatatggctcatactcttcctttttcaatattattgaagcatttatcagggttattgtctcatgagcggatacatatttgaatgtatttagaaaaataaacaaataggggttccgcgcacatttccccgaaaagtgccacctgacgtctaagaaaccattattatcatgacattaacctataaaaataggcgtatcacgaggccctttcgtctcgcgcgtttcggtgatgacggtgaaaacctctgacacatgcagctcccggagacggtcacagcttgtctgtaagcggatgccgggagcagacaagcccgtcagggcgcgtcagcgggtgttggcgggtgtcggggctggcttaactatgcggcatcagagcagattgtactgagagtgcaccatatgcggtgtgaaataccgcacagatgcgtaaggagaaaataccgcatcaggcgccattcgccattcaggctgcgcaactgttgggaagggcgatcggtgcgggcctcttcgctattacgccagctggcgaaagggggatgtgctgcaaggcgattaagttgggtaacgccagggttttcccagtcacgacgttgtaaaacgacggccagtgaattgacgcgtattgggatggtaccgggccccccctcgaggtcgacggtatcgatacggcatcagagcagattgtactgagagtgcaccataatcggcattttcttttgcgtttttatttgttaactgttaattgtccttgttcaaggatgctgtctttgacaacagatgttttcttgcctttgatgttcagcaggaagctaggcgcaaacgttgattgtttgtctgcgtagaatcctctgtttgtcatatagcttgtaatcacgacattgtttcctttcgcttgaggtacagcgaagtgtgagtaagtaaaggttacatcgttaggatcaagatccatttttaacacaaggccagttttgttcagcggcttgtatgggccagttaaagaattagaaacataaccaagcatgtaaatatcgttagacgtaatgccgtcaatcgtcatttttgatccgcgggagtcagtgaacagataccatttgccgttcattttaaagacgttcgcgcgttcaatttcatctgttactgtgttagatgcaatcagcggtttcatcacttttttcagtgtgtaatcatcgtttagctcaatcataccgagagcgccgtttgctaactcagccgtgcgttttttatcgctttgcagaagtttttgactttcttgacggaagaatgatgtgcttttgccatagtatgctttgttaaataaagattcttcgccttggtagccatcttcagttccagtgtttgcttcaaatactaagtatttgtggcctttatcttctacgtagtgaggatctctcagcgtatggttgtcgcctgagctgtagttgccttcatcgatgaactgctgtacattttgatacgtttttccgtcaccgtcaaagattgatttataatcctctacaccgttgatgttcaaagagctgtctgatgctgatacgttaacttgtgcagttgtcagtgtttgtttgccgtaatgtttaccggagaaatcagtgtagaataaacggatttttccgtcagatgtaaatgtggctgaacctgaccattcttgtgtttggtcttttaggatagaatcatttgcatcgaatttgtcgctgtctttaaagacgcggccagcgtttttccagctgtcaatagaagtttcgccgactttttgatagaacatgtaaatcgatgtgtcatccgcatttttaggatctccggctaatgcaaagacgatgtggtagccgtgatagtttgcgacagtgccgtcagcgttttgtaatggccagctgtcccaaacgtccaggccttttgcagaagagatatttttaattgtggacgaatcgaactcaggaacttgatatttttcatttttttgctgttcagggatttgcagcatatcatggcgtgtaatatgggaaatgccgtatgtttccttatatggcttttggttcgtttctttcgcaaacgcttgagttgcgcctcctgccagcagtgcggtagtaaaggttaatactgttgcttgttttgcaaactttttgatgttcatcgttcatgtctccttttttatgtactgtgttagcggtctgcttcttccagccctcctgtttgaagatggcaagttagttacgcacaataaaaaaagacctaaaatatgtaaggggtgacgccaaagtatacactttgccctttacacattttaggtcttgcctgctttatcagtaacaaacccgcgcgatttacttttcgacctcattctattagactctcgtttggattgcaactggtctattttcctcttttgtttgatagaaaatcataaaaggatttgcagactacgggcctaaagaactaaaaaatctatctgtttcttttcattctctgtattttttatagtttctgttgcatgggcataaagttgcaagcttgatatcttgacagctagctcagtcctaggtataatactagtattcgtcggttcagcgacgataagccgagaagtgccaataaaactgttaagtggtttggtaacgctcggtaaggtagccaaaaggctgaaactccgtgcacaaagaccgcacggacgcttcacatatagctcataaacaagggtttgcgagctagcttgtggagtgtgaacctgacgcccgatgctgatatggccggcatggtcccagcctcctcgctggcgccggctgggcaacatgcttcggcatggcgaatgggacgatctgacagctagcataaccccttggggcctctaaacgggtcttgaggggttttttggatatcgaattcctgcagcccgggggatccactagttctagagcggccgccaccgcggtggagctcatcccaatggcgcgccgagcttggctcgagcatggtcatagctgtttcctgtgtgaaattgttatccgctcacaattccacacaacatacgagccggaagcataaagtgtaaagcctggggtgcctaatgagtgagctaactcacattaattgcgttgcgctcactgcccgctttccagtcgggaaacctgtcgtgccagctgcattaatgaatcggccaacgcgcggggagaggcggtttgcgtattgggcgc

SEQ ID NO: 82 - DNA, 4946 bp, Artificial Sequence
  psgRNAv1-pyrF
tcttccgcttcctcgctcactgactcgctgcgctcggtcgttcggctgcggcgagcggtatcagctcactcaaaggcggtaatacggttatccacagaatcaggggataacgcaggaaagaacatgtgagcaaaaggccagcaaaaggccaggaaccgtaaaaaggccgcgttgctggcgtttttccataggctccgcccccctgacgagcatcacaaaaatcgacgctcaagtcagaggtggcgaaacccgacaggactataaagataccaggcgtttccccctggaagctccctcgtgcgctctcctgttccgaccctgccgcttaccggatacctgtccgcctttctcccttcgggaagcgtggcgctttctcatagctcacgctgtaggtatctcagttcggtgtaggtcgttcgctccaagctgggctgtgtgcacgaaccccccgttcagcccgaccgctgcgccttatccggtaactatcgtcttgagtccaacccggtaagacacgacttatcgccactggcagcagccactggtaacaggattagcagagcgaggtatgtaggcggtgctacagagttcttgaagtggtggcctaactacggctacactagaagaacagtatttggtatctgcgctctgctgaagccagttaccttcggaaaaagagttggtagctcttgatccggcaaacaaaccaccgctggtagcggtggtttttttgtttgcaagcagcagattacgcgcagaaaaaaaggatctcaagaagatcctttgatcttttctacggggtctgacgctcagtggaacgaaaactcacgttaagggattttggtcatgagattatcaaaaaggatcttcacctagatccttttaaattaaaaatgaagttttaaatcaatctaaagtatatatgagtaaacttggtctgacagttagaaaaactcatcgagcatcaaatgaaactgcaatttattcatatcaggattatcaataccatatttttgaaaaagccgtttctgtaatgaaggagaaaactcaccgaggcagttccataggatggcaagatcctggtatcggtctgcgattccgactcgtccaacatcaatacaacctattaatttcccctcgtcaaaaataaggttatcaagtgagaaatcaccatgagtgacgactgaatccggtgagaatggcaaaagtttatgcatttctttccagacttgttcaacaggccagccattacgctcgtcatcaaaatcactcgcatcaaccaaaccgttattcattcgtgattgcgcctgagcgagacgaaatacgcgatcgctgttaaaaggacaattacaaacaggaatcgaatgcaaccggcgcaggaacactgccagcgcatcaacaatattttcacctgaatcaggatattcttctaatacctggaatgctgttttcccagggatcgcagtggtgagtaaccatgcatcatcaggagtacggataaaatgcttgatggtcggaagaggcataaattccgtcagccagtttagtctgaccatctcatctgtaacatcattggcaacgctacctttgccatgtttcagaaacaactctggcgcatcgggcttcccatacaatcgatagattgtcgcacctgattgcccgacattatcgcgagcccatttatacccatataaatcagcatccatgttggaatttaatcgcggcctagagcaagacgtttcccgttgaatatggctcatactcttcctttttcaatattattgaagcatttatcagggttattgtctcatgagcggatacatatttgaatgtatttagaaaaataaacaaataggggttccgcgcacatttccccgaaaagtgccacctgacgtctaagaaaccattattatcatgacattaacctataaaaataggcgtatcacgaggccctttcgtctcgcgcgtttcggtgatgacggtgaaaacctctgacacatgcagctcccggagacggtcacagcttgtctgtaagcggatgccgggagcagacaagcccgtcagggcgcgtcagcgggtgttggcgggtgtcggggctggcttaactatgcggcatcagagcagattgtactgagagtgcaccatatgcggtgtgaaataccgcacagatgcgtaaggagaaaataccgcatcaggcgccattcgccattcaggctgcgcaactgttgggaagggcgatcggtgcgggcctcttcgctattacgccagctggcgaaagggggatgtgctgcaaggcgattaagttgggtaacgccagggttttcccagtcacgacgttgtaaaacgacggccagtgaattgacgcgtattgggatggtaccgggccccccctcgaggtcgacggtatcgatacggcatcagagcagattgtactgagagtgcaccataatcggcattttcttttgcgtttttatttgttaactgttaattgtccttgttcaaggatgctgtctttgacaacagatgttttcttgcctttgatgttcagcaggaagctaggcgcaaacgttgattgtttgtctgcgtagaatcctctgtttgtcatatagcttgtaatcacgacattgtttcctttcgcttgaggtacagcgaagtgtgagtaagtaaaggttacatcgttaggatcaagatccatttttaacacaaggccagttttgttcagcggcttgtatgggccagttaaagaattagaaacataaccaagcatgtaaatatcgttagacgtaatgccgtcaatcgtcatttttgatccgcgggagtcagtgaacagataccatttgccgttcattttaaagacgttcgcgcgttcaatttcatctgttactgtgttagatgcaatcagcggtttcatcacttttttcagtgtgtaatcatcgtttagctcaatcataccgagagcgccgtttgctaactcagccgtgcgttttttatcgctttgcagaagtttttgactttcttgacggaagaatgatgtgcttttgccatagtatgctttgttaaataaagattcttcgccttggtagccatcttcagttccagtgtttgcttcaaatactaagtatttgtggcctttatcttctacgtagtgaggatctctcagcgtatggttgtcgcctgagctgtagttgccttcatcgatgaactgctgtacattttgatacgtttttccgtcaccgtcaaagattgatttataatcctctacaccgttgatgttcaaagagctgtctgatgctgatacgttaacttgtgcagttgtcagtgtttgtttgccgtaatgtttaccggagaaatcagtgtagaataaacggatttttccgtcagatgtaaatgtggctgaacctgaccattcttgtgtttggtcttttaggatagaatcatttgcatcgaatttgtcgctgtctttaaagacgcggccagcgtttttccagctgtcaatagaagtttcgccgactttttgatagaacatgtaaatcgatgtgtcatccgcatttttaggatctccggctaatgcaaagacgatgtggtagccgtgatagtttgcgacagtgccgtcagcgttttgtaatggccagctgtcccaaacgtccaggccttttgcagaagagatatttttaattgtggacgaatcgaactcaggaacttgatatttttcatttttttgctgttcagggatttgcagcatatcatggcgtgtaatatgggaaatgccgtatgtttccttatatggcttttggttcgtttctttcgcaaacgcttgagttgcgcctcctgccagcagtgcggtagtaaaggttaatactgttgcttgttttgcaaactttttgatgttcatcgttcatgtctccttttttatgtactgtgttagcggtctgcttcttccagccctcctgtttgaagatggcaagttagttacgcacaataaaaaaagacctaaaatatgtaaggggtgacgccaaagtatacactttgccctttacacattttaggtcttgcctgctttatcagtaacaaacccgcgcgatttacttttcgacctcattctattagactctcgtttggattgcaactggtctattttcctcttttgtttgatagaaaatcataaaaggatttgcagactacgggcctaaagaactaaaaaatctatctgtttcttttcattctctgtattttttatagtttctgttgcatgggcataaagttgcaagcttgatatcttgacagctagctcagtcctaggtataatactagtattcgtcggttcagcgacgataagccgagaagtgccaataaaactgttaagtggtttggtaacgctcggtaaggtagccaaaaggctgaaactccgtgcacaaagaccgcacggacgcttcacatatagctcataaacaagggtttgcgagctagcttgtggagtgtgaacagtttcacgatattcccaacggccggcatggtcccagcctcctcgctggcgccggctgggcaacatgcttcggcatggcgaatgggacgatctgacagctagcataaccccttggggcctctaaacgggtcttgaggggttttttggatatcgaattcctgcagcccgggggatccactagttctagagcggccgccaccgcggtggagctcatcccaatggcgcgccgagcttggctcgagcatggtcatagctgtttcctgtgtgaaattgttatccgctcacaattccacacaacatacgagccggaagcataaagtgtaaagcctggggtgcctaatgagtgagctaactcacattaattgcgttgcgctcactgcccgctttccagtcgggaaacctgtcgtgccagctgcattaatgaatcggccaacgcgcggggagaggcggtttgcgtattgggcgc

SEQ ID NO: 83 - DNA, 90 bp, Artificial Sequence
  hisD-RT
gctggtgattgctgacagcggcgctacgccggatttcgtggcttccaggcactgagcaccagccgcctgatcgtgaccaacgatttagcg

SEQ ID NO: 84 - DNA, 90 bp, Artificial Sequence
  pyrF-RT
gccgcctgaaggtgggcaaagagatgttcaccctgctgggaccgcatgaccgcggcgcgcgaagcgctgctgccctttggtcaagacgcg

SEQ ID NO: 85 - DNA, 1266 bp, Artificial Sequence
  AsCas12f1 encoding gene with condon optimization for human
atgatcaaggtgtacagatacgagatcgtgaagcctctggacctggactggaaggagttcggcaccatcctgagacagctgcagcaggaaaccagattcgccctgaataaggccacacagctggcctgggagtggatgggcttcagcagcgactacaaggataaccacggcgagtaccccaagagcaaggacatcctgggctacaccaacgtgcacggctacgcctaccacaccatcaagacaaaggcctacagactgaactctggaaatctgagccagaccatcaagagagccacagacaggttcaaggcctaccagaaggagatcctgcgcggcgacatgtctatccccagctacaagagggacatccccctggacctgatcaaggagaacatctccgtgaacaggatgaatcacggcgactacatcgccagcctgtctctgctgagcaaccccgccaagcaggagatgaacgtgaagagaaagatctccgtgatcatcatcgtgaggggcgccggcaagaccatcatggacagaatcctgtccggcgagtaccaggtgagcgccagccagattatccacgacgaccggaagaacaagtggtacctgaacatcagctacgacttcgagccacagaccagagtgctggacctgaacaagatcatgggcattgacctgggcgtggccgtggccgtgtacatggccttccagcacacccccgccaggtacaagctggagggcggcgagattgagaacttcaggaggcaggtggagagccggcgcatctccatgctgagacagggcaagtacgccggcggcgccaggggcggccacggcagagacaagagaatcaagcccattgagcagctgagggataagatcgccaatttcagagacaccaccaatcaccggtacagcagatacatcgtggacatggccatcaaggagggctgcggcacaatccagatggaggatctgacaaacatcagagacatcggcagcagattcctgcagaactggacctactacgacctgcagcagaagatcatctacaaggccgaggaggccggcatcaaagtgatcaagatcgacccccagtacaccagccagagatgctccgagtgcggcaacatcgactccggcaacagaatcggccaggccatctttaagtgccgggcctgcggctacgaggccaacgccgactacaacgccgcccggaatatcgccatccccaacatcgacaagatcatcgccgagagcattaag

SEQ ID NO: 86 - DNA, 6842 bp, Artificial Sequence
  pAsCas12fHs
ggtaccgattagtgaacggatctcgacggtatcgatcacgagactagcctcgagcggccgcccccttcaccgagggcctatttcccatgattccttcatatttgcatatacgatacaaggctgttagagagataattggaattaatttgactgtaaacacaaagatattagtacaaaatacgtgacgtagaaagtaataatttcttgggtagtttgcagttttaaaattatgttttaaaatggactatcatatgcttaccgtaacttgaaagtatttcgatttcttggctttatatatcttgtggaaaggacgaaacaccgattcgtcggttcagcgacgataagccgagaagtgccaataaaactgttaagtggtttggtaacgctcggtaaggtagccaaaaggctgaaactccgtgcacaaagaccgcacggacgcttcacatatagctcataaacaagggtttgcgagctagcttgtggagtgtgaaccgagacccgagagagggtcggtctcctttttttgaattctcgacctcgagacaaatggcagtattcatccacaattttaaaagaaaaggggggattggggggtacagtgcaggggaaagaatagtagacataatagcaacagacatacaaactaaagaattacaaaaacaaattacaaaaattcaaaattttcgggtttattacagggacagcagagatccactttggccgcggctcgagggggttggggttgcgccttttccaaggcagccctgggtttgcgcagggacgcggctgctctgggcgtggttccgggaaacgcagcggcgccgaccctgggactcgcacattcttcacgtccgttcgcagcgtcacccggatcttcgccgctacccttgtgggccccccggcgacgcttcctgctccgcccctaagtcgggaaggttccttgcggttcgcggcgtgccggacgtgacaaacggaagccgcacgtctcactagtaccctcgcagacggacagcgccagggagcaatggcagcgcgccgaccgcgatgggctgtggccaatagcggctgctcagcagggcgcgccgagagcagcggccgggaaggggcggtgcgggaggcggggtgtggggcggtagtgtgggccctgttcctgcccgcgcggtgttccgcattctgcaagcctccggagcgcacgtcggcagtcggctccctcgttgaccgaatcaccgacctctctccccagggggatccaccggagcttaccatgaccgagtacaagcccacggtgcgcctcgccacccgcgacgacgtccccagggccgtacgcaccctcgccgccgcgttcgccgactaccccgccacgcgccacaccgtcgatccggaccgccacatcgagcgggtcaccgagctgcaagaactcttcctcacgcgcgtcgggctcgacatcggcaaggtgtgggtcgcggacgacggcgccgcggtggcggtctggaccacgccggagagcgtcgaagcgggggcggtgttcgccgagatcggcccgcgcatggccgagttgagcggttcccggctggccgcgcagcaacagatggaaggcctcctggcgccgcaccggcccaaggagcccgcgtggttcctggccaccgtcggcgtctcgcccgaccaccagggcaagggtctgggcagcgccgtcgtgctccccggagtggaggcggccgagcgcgccggggtgcccgccttcctggaaacctccgcgccccgcaacctccccttctacgagcggctcggcttcaccgtcaccgccgacgtcgaggtgcccgaaggaccgcgcacctggtgcatgacccgcaagcccggtgcctgacgcccgccccacgacccgcagcgcccgaccgaaaggagcgcacgaccccatgcatcggtacctttaagaccaatgacttacaaggcagctgtagatcttagccactttctagagtcggggcggccggccgcttcgagcagacatgataagatacattgatgagtttggacaaaccacaactagaatgcagtgaaaaaaatgctttatttgtgaaatttgtgatgctattgctttatttgtaaccattataagctgcaataaacaagttaacaacaacaattgcattcattttatgtttcaggttcagggggaggtgtgggaggttttttaaagcaagtaaaacctctacaaatgtggtaaaatcgataaggatccgtcgaccgatgcccttgagagccttcaacccagtcagctccttccggtgggcgcggggcatgactatcgtcgccgcacttatgactgtcttctttatcatgcaactcgtaggacaggtgccggcagcgctcttccgcttcctcgctcactgactcgctgcgctcggtcgttcggctgcggcgagcggtatcagctcactcaaaggcggtaatacggttatccacagaatcaggggataacgcaggaaagaacatgtgagcaaaaggccagcaaaaggccaggaaccgtaaaaaggccgcgttgctggcgtttttccataggctccgcccccctgacgagcatcacaaaaatcgacgctcaagtcagaggtggcgaaacccgacaggactataaagataccaggcgtttccccctggaagctccctcgtgcgctctcctgttccgaccctgccgcttaccggatacctgtccgcctttctcccttcgggaagcgtggcgctttctcaatgctcacgctgtaggtatctcagttcggtgtaggtcgttcgctccaagctgggctgtgtgcacgaaccccccgttcagcccgaccgctgcgccttatccggtaactatcgtcttgagtccaacccggtaagacacgacttatcgccactggcagcagccactggtaacaggattagcagagcgaggtatgtaggcggtgctacagagttcttgaagtggtggcctaactacggctacactagaaggacagtatttggtatctgcgctctgctgaagccagttaccttcggaaaaagagttggtagctcttgatccggcaaacaaaccaccgctggtagcggtggtttttttgtttgcaagcagcagattacgcgcagaaaaaaaggatctcaagaagatcctttgatcttttctacggggtctgacgctcagtggaacgaaaactcacgttaagggattttggtcatgagattatcaaaaaggatcttcacctagatccttttaaattaaaaatgaagttttaaatcaatctaaagtatatatgagtaaacttggtctgacagttaccaatgcttaatcagtgaggcacctatctcagcgatctgtctatttcgttcatccatagttgcctgactccccgtcgtgtagataactacgatacgggagggcttaccatctggccccagtgctgcaatgataccgcgggacccacgctcaccggctccagatttatcagcaataaaccagccagccggaagggccgagcgcagaagtggtcctgcaactttatccgcctccatccagtctattaattgttgccgggaagctagagtaagtagttcgccagttaatagtttgcgcaacgttgttgccattgctacaggcatcgtggtgtcacgctcgtcgtttggtatggcttcattcagctccggttcccaacgatcaaggcgagttacatgatcccccatgttgtgcaaaaaagcggttagctccttcggtcctccgatcgttgtcagaagtaagttggccgcagtgttatcactcatggttatggcagcactgcataattctcttactgtcatgccatccgtaagatgcttttctgtgactggtgagtactcaaccaagtcattctgagaatagtgtatgcggcgaccgagttgctcttgcccggcgtcaatacgggataataccgcgccacatagcagaactttaaaagtgctcatcattggaaaacgttcttcggggcgaaaactctcaaggatcttaccgctgttgagatccagttcgatgtaacccactcgtgcacccaactgatcttcagcatcttttactttcaccagcgtttctgggtgagcaaaaacaggaaggcaaaatgccgcaaaaaagggaataagggcgacacggaaatgttgaatactcatactcttcctttttcaatattattgaagcatttatcagggttattgtctcatgagcggatacatatttgaatgtatttagaaaaataaacaaataggggttccgcgcacatttccccgaaaagtgccacctgcaggaaacagctatgaccatgattacgccaagctctagctagaggtcgacggtatcgagccccagctggttctttccgcctcagaagccatagagcccaccgcatccccagcatgcctgctattgtcttcccaatcctcccccttgctgtcctgccccaccccaccccccagaatagaatgacacctactcagacaatgcgatgcaatttcctcattttattaggaaaggacagtgggagtggcaccttccagggtcaaggaaggcacgggggaggggcaaacaacagatggctggcaactagaaggcacagtcgaggctgatcagcgggtttaaactcaatggtgatggtgatgatgaccggttagactttcctcttcttcttgggagaaccaccagacttaatgctctcggcgatgatcttgtcgatgttggggatggcgatattccgggcggcgttgtagtcggcgttggcctcgtagccgcaggcccggcacttaaagatggcctggccgattctgttgccggagtcgatgttgccgcactcggagcatctctggctggtgtactgggggtcgatcttgatcactttgatgccggcctcctcggccttgtagatgatcttctgctgcaggtcgtagtaggtccagttctgcaggaatctgctgccgatgtctctgatgtttgtcagatcctccatctggattgtgccgcagccctccttgatggccatgtccacgatgtatctgctgtaccggtgattggtggtgtctctgaaattggcgatcttatccctcagctgctcaatgggcttgattctcttgtctctgccgtggccgcccctggcgccgccggcgtacttgccctgtctcagcatggagatgcgccggctctccacctgcctcctgaagttctcaatctcgccgccctccagcttgtacctggcgggggtgtgctggaaggccatgtacacggccacggccacgcccaggtcaatgcccatgatcttgttcaggtccagcactctggtctgtggctcgaagtcgtagctgatgttcaggtaccacttgttcttccggtcgtcgtggataatctggctggcgctcacctggtactcgccggacaggattctgtccatgatggtcttgccggcgcccctcacgatgatgatcacggagatctttctcttcacgttcatctcctgcttggcggggttgctcagcagagacaggctggcgatgtagtcgccgtgattcatcctgttcacggagatgttctccttgatcaggtccagggggatgtccctcttgtagctggggatagacatgtcgccgcgcaggatctccttctggtaggccttgaacctgtctgtggctctcttgatggtctggctcagatttccagagttcagtctgtaggcctttgtcttgatggtgtggtaggcgtagccgtgcacgttggtgtagcccaggatgtccttgctcttggggtactcgccgtggttatccttgtagtcgctgctgaagcccatccactcccaggccagctgtgtggccttattcagggcgaatctggtttcctgctgcagctgtctcaggatggtgccgaactccttccagtccaggtccagaggcttcacgatctcgtatctgtacaccttgatcatgactttcctcttcttcttgggcatggtggcggctctccctatagtgagtcgtattagcggccgcggatctctagcggatctgacggttcactaaaccagctctgcttatatagacctcccaccgtacacgcctaccgcccatttgcgtcaatggggcggagttgttacgacattttggaaagtcccgttgattttggtgccaaaacaaactcccattgacgtcaatggggtggagacttggaaatccccgtgagtcaaaccgctatccacgcccattgatgtactgccaaaaccgcatcaccatggtaatagcgatgactaatacgtagatgtactgccaagtaggaaagtcccataaggtcatgtactgggcataatgccaggcgggccatttaccgtcattgacgtcaatagggggcgtacttggcatatgatacacttgatgtactgccaagtgggcagtttaccgtaaatactccacccattgacgtcaatggaaagtccctattggcgttactatgggaacatacgtcattattgacgtcaatgggcgggggtcgttgggcggtcagccaggcgggccatttaccgtaagttatgtaacgcggaactccatatatgggctatgaactaatgaccccgtaattgattactattaataactagtcaataatcaatgtcaacgcgtatatctggcccgtacatcgcgaagcagcgcaaaacgcctaaccctaagcagattcttcatgcaattgtcggtcaagaatcgatagtactaacatacgctctccatcaaaacaaaacgaaacaaaacaaactagcaaaataggctgtccccagtgcaagtgcaggtgccagaacatttctctatcgata

SEQ ID NO: 87 - DNA, 2256 bp, Artificial Sequence
  53_human vector backbone
aacaacaacaattgcattcattttatgtttcaggttcagggggaggtgtgggaggttttttaaagcaagtaaaacctctacaaatgtggtaaaatcgataaggatccgtcgaccgatgcccttgagagccttcaacccagtcagctccttccggtgggcgcggggcatgactatcgtcgccgcacttatgactgtcttctttatcatgcaactcgtaggacaggtgccggcagcgctcttccgcttcctcgctcactgactcgctgcgctcggtcgttcggctgcggcgagcggtatcagctcactcaaaggcggtaatacggttatccacagaatcaggggataacgcaggaaagaacatgtgagcaaaaggccagcaaaaggccaggaaccgtaaaaaggccgcgttgctggcgtttttccataggctccgcccccctgacgagcatcacaaaaatcgacgctcaagtcagaggtggcgaaacccgacaggactataaagataccaggcgtttccccctggaagctccctcgtgcgctctcctgttccgaccctgccgcttaccggatacctgtccgcctttctcccttcgggaagcgtggcgctttctcaatgctcacgctgtaggtatctcagttcggtgtaggtcgttcgctccaagctgggctgtgtgcacgaaccccccgttcagcccgaccgctgcgccttatccggtaactatcgtcttgagtccaacccggtaagacacgacttatcgccactggcagcagccactggtaacaggattagcagagcgaggtatgtaggcggtgctacagagttcttgaagtggtggcctaactacggctacactagaaggacagtatttggtatctgcgctctgctgaagccagttaccttcggaaaaagagttggtagctcttgatccggcaaacaaaccaccgctggtagcggtggtttttttgtttgcaagcagcagattacgcgcagaaaaaaaggatctcaagaagatcctttgatcttttctacggggtctgacgctcagtggaacgaaaactcacgttaagggattttggtcatgagattatcaaaaaggatcttcacctagatccttttaaattaaaaatgaagttttaaatcaatctaaagtatatatgagtaaacttggtctgacagttaccaatgcttaatcagtgaggcacctatctcagcgatctgtctatttcgttcatccatagttgcctgactccccgtcgtgtagataactacgatacgggagggcttaccatctggccccagtgctgcaatgataccgcgggacccacgctcaccggctccagatttatcagcaataaaccagccagccggaagggccgagcgcagaagtggtcctgcaactttatccgcctccatccagtctattaattgttgccgggaagctagagtaagtagttcgccagttaatagtttgcgcaacgttgttgccattgctacaggcatcgtggtgtcacgctcgtcgtttggtatggcttcattcagctccggttcccaacgatcaaggcgagttacatgatcccccatgttgtgcaaaaaagcggttagctccttcggtcctccgatcgttgtcagaagtaagttggccgcagtgttatcactcatggttatggcagcactgcataattctcttactgtcatgccatccgtaagatgcttttctgtgactggtgagtactcaaccaagtcattctgagaatagtgtatgcggcgaccgagttgctcttgcccggcgtcaatacgggataataccgcgccacatagcagaactttaaaagtgctcatcattggaaaacgttcttcggggcgaaaactctcaaggatcttaccgctgttgagatccagttcgatgtaacccactcgtgcacccaactgatcttcagcatcttttactttcaccagcgtttctgggtgagcaaaaacaggaaggcaaaatgccgcaaaaaagggaataagggcgacacggaaatgttgaatactcatactcttcctttttcaatattattgaagcatttatcagggttattgtctcatgagcggatacatatttgaatgtatttagaaaaataaacaaataggggttccgcgcacatttccccgaaaagtgccacctgcaggaaacagctatgaccatgattacgccaagctctagctagaggtcgacggtatcgagccccagctggttctttccgcctcagaag

SEQ ID NO: 88 - DNA, 1440 bp, Artificial Sequence
  puromycin
cactttggccgcggctcgagggggttggggttgcgccttttccaaggcagccctgggtttgcgcagggacgcggctgctctgggcgtggttccgggaaacgcagcggcgccgaccctgggactcgcacattcttcacgtccgttcgcagcgtcacccggatcttcgccgctacccttgtgggccccccggcgacgcttcctgctccgcccctaagtcgggaaggttccttgcggttcgcggcgtgccggacgtgacaaacggaagccgcacgtctcactagtaccctcgcagacggacagcgccagggagcaatggcagcgcgccgaccgcgatgggctgtggccaatagcggctgctcagcagggcgcgccgagagcagcggccgggaaggggcggtgcgggaggcggggtgtggggcggtagtgtgggccctgttcctgcccgcgcggtgttccgcattctgcaagcctccggagcgcacgtcggcagtcggctccctcgttgaccgaatcaccgacctctctccccagggggatccaccggagcttaccatgaccgagtacaagcccacggtgcgcctcgccacccgcgacgacgtccccagggccgtacgcaccctcgccgccgcgttcgccgactaccccgccacgcgccacaccgtcgatccggaccgccacatcgagcgggtcaccgagctgcaagaactcttcctcacgcgcgtcgggctcgacatcggcaaggtgtgggtcgcggacgacggcgccgcggtggcggtctggaccacgccggagagcgtcgaagcgggggcggtgttcgccgagatcggcccgcgcatggccgagttgagcggttcccggctggccgcgcagcaacagatggaaggcctcctggcgccgcaccggcccaaggagcccgcgtggttcctggccaccgtcggcgtctcgcccgaccaccagggcaagggtctgggcagcgccgtcgtgctccccggagtggaggcggccgagcgcgccggggtgcccgccttcctggaaacctccgcgccccgcaacctccccttctacgagcggctcggcttcaccgtcaccgccgacgtcgaggtgcccgaaggaccgcgcacctggtgcatgacccgcaagcccggtgcctgacgcccgccccacgacccgcagcgcccgaccgaaaggagcgcacgaccccatgcatcggtacctttaagaccaatgacttacaaggcagctgtagatcttagccactttctagagtcggggcggccggccgcttcgagcagacatgataagatacattgatgagtttggacaaaccacaactagaatgcagtgaaaaaaatgctttatttgtgaaatttgtgatgctattgctttatttgtaaccattataagctgcaataaacaagttaacaacaacaattgcattca

SEQ ID NO: 89 - DNA, 2299 bp, Artificial Sequence
  CMV-AsCas12f
ggttctttccgcctcagaagccatagagcccaccgcatccccagcatgcctgctattgtcttcccaatcctcccccttgctgtcctgccccaccccaccccccagaatagaatgacacctactcagacaatgcgatgcaatttcctcattttattaggaaaggacagtgggagtggcaccttccagggtcaaggaaggcacgggggaggggcaaacaacagatggctggcaactagaaggcacagtcgaggctgatcagcgggtttaaactcaatggtgatggtgatgatgaccggttagactttcctcttcttcttgggagaaccaccagacttaatgctctcggcgatgatcttgtcgatgttggggatggcgatattccgggcggcgttgtagtcggcgttggcctcgtagccgcaggcccggcacttaaagatggcctggccgattctgttgccggagtcgatgttgccgcactcggagcatctctggctggtgtactgggggtcgatcttgatcactttgatgccggcctcctcggccttgtagatgatcttctgctgcaggtcgtagtaggtccagttctgcaggaatctgctgccgatgtctctgatgtttgtcagatcctccatctggattgtgccgcagccctccttgatggccatgtccacgatgtatctgctgtaccggtgattggtggtgtctctgaaattggcgatcttatccctcagctgctcaatgggcttgattctcttgtctctgccgtggccgcccctggcgccgccggcgtacttgccctgtctcagcatggagatgcgccggctctccacctgcctcctgaagttctcaatctcgccgccctccagcttgtacctggcgggggtgtgctggaaggccatgtacacggccacggccacgcccaggtcaatgcccatgatcttgttcaggtccagcactctggtctgtggctcgaagtcgtagctgatgttcaggtaccacttgttcttccggtcgtcgtggataatctggctggcgctcacctggtactcgccggacaggattctgtccatgatggtcttgccggcgcccctcacgatgatgatcacggagatctttctcttcacgttcatctcctgcttggcggggttgctcagcagagacaggctggcgatgtagtcgccgtgattcatcctgttcacggagatgttctccttgatcaggtccagggggatgtccctcttgtagctggggatagacatgtcgccgcgcaggatctccttctggtaggccttgaacctgtctgtggctctcttgatggtctggctcagatttccagagttcagtctgtaggcctttgtcttgatggtgtggtaggcgtagccgtgcacgttggtgtagcccaggatgtccttgctcttggggtactcgccgtggttatccttgtagtcgctgctgaagcccatccactcccaggccagctgtgtggccttattcagggcgaatctggtttcctgctgcagctgtctcaggatggtgccgaactccttccagtccaggtccagaggcttcacgatctcgtatctgtacaccttgatcatgactttcctcttcttcttgggcatggtggcggctctccctatagtgagtcgtattagcggccgcggatctctagcggatctgacggttcactaaaccagctctgcttatatagacctcccaccgtacacgcctaccgcccatttgcgtcaatggggcggagttgttacgacattttggaaagtcccgttgattttggtgccaaaacaaactcccattgacgtcaatggggtggagacttggaaatccccgtgagtcaaaccgctatccacgcccattgatgtactgccaaaaccgcatcaccatggtaatagcgatgactaatacgtagatgtactgccaagtaggaaagtcccataaggtcatgtactgggcataatgccaggcgggccatttaccgtcattgacgtcaatagggggcgtacttggcatatgatacacttgatgtactgccaagtgggcagtttaccgtaaatactccacccattgacgtcaatggaaagtccctattggcgttactatgggaacatacgtcattattgacgtcaatgggcgggggtcgttgggcggtcagccaggcgggccatttaccgtaagttatgtaacgcggaactccatatatgggctatgaactaatgaccccgtaattgattactattaataactagtcaataatcaatgtcaacgcgtatatctggcccgt

SEQ ID NO: 90 - DNA, 927 bp, Artificial Sequence
  Human_sgRNAv1
aacgcgtatatctggcccgtacatcgcgaagcagcgcaaaacgcctaaccctaagcagattcttcatgcaattgtcggtcaagaatcgatagtactaacatacgctctccatcaaaacaaaacgaaacaaaacaaactagcaaaataggctgtccccagtgcaagtgcaggtgccagaacatttctctatcgataggtaccgattagtgaacggatctcgacggtatcgatcacgagactagcctcgagcggccgcccccttcaccgagggcctatttcccatgattccttcatatttgcatatacgatacaaggctgttagagagataattggaattaatttgactgtaaacacaaagatattagtacaaaatacgtgacgtagaaagtaataatttcttgggtagtttgcagttttaaaattatgttttaaaatggactatcatatgcttaccgtaacttgaaagtatttcgatttcttggctttatatatcttgtggaaaggacgaaacaccgattcgtcggttcagcgacgataagccgagaagtgccaataaaactgttaagtggtttggtaacgctcggtaaggtagccaaaaggctgaaactccgtgcacaaagaccgcacggacgcttcacatatagctcataaacaagggtttgcgagctagcttgtggagtgtgaaccgagacccgagagagggtcggtctcctttttttgaattctcgacctcgagacaaatggcagtattcatccacaattttaaaagaaaaggggggattggggggtacagtgcaggggaaagaatagtagacataatagcaacagacatacaaactaaagaattacaaaaacaaattacaaaaattcaaaattttcgggtttattacagggacagcagagatccactttggccgcggctcgag

SEQ ID NO: 91 - DNA, 6977 bp, Artificial Sequence
  pET28a-SUMO-AsCas12f-2NLS
tggcgaatgggacgcgccctgtagcggcgcattaagcgcggcgggtgtggtggttacgcgcagcgtgaccgctacacttgccagcgccctagcgcccgctcctttcgctttcttcccttcctttctcgccacgttcgccggctttccccgtcaagctctaaatcgggggctccctttagggttccgatttagtgctttacggcacctcgaccccaaaaaacttgattagggtgatggttcacgtagtgggccatcgccctgatagacggtttttcgccctttgacgttggagtccacgttctttaatagtggactcttgttccaaactggaacaacactcaaccctatctcggtctattcttttgatttataagggattttgccgatttcggcctattggttaaaaaatgagctgatttaacaaaaatttaacgcgaattttaacaaaatattaacgtttacaatttcaggtggcacttttcggggaaatgtgcgcggaacccctatttgtttatttttctaaatacattcaaatatgtatccgctcatgaattaattcttagaaaaactcatcgagcatcaaatgaaactgcaatttattcatatcaggattatcaataccatatttttgaaaaagccgtttctgtaatgaaggagaaaactcaccgaggcagttccataggatggcaagatcctggtatcggtctgcgattccgactcgtccaacatcaatacaacctattaatttcccctcgtcaaaaataaggttatcaagtgagaaatcaccatgagtgacgactgaatccggtgagaatggcaaaagtttatgcatttctttccagacttgttcaacaggccagccattacgctcgtcatcaaaatcactcgcatcaaccaaaccgttattcattcgtgattgcgcctgagcgagacgaaatacgcgatcgctgttaaaaggacaattacaaacaggaatcgaatgcaaccggcgcaggaacactgccagcgcatcaacaatattttcacctgaatcaggatattcttctaatacctggaatgctgttttcccggggatcgcagtggtgagtaaccatgcatcatcaggagtacggataaaatgcttgatggtcggaagaggcataaattccgtcagccagtttagtctgaccatctcatctgtaacatcattggcaacgctacctttgccatgtttcagaaacaactctggcgcatcgggcttcccatacaatcgatagattgtcgcacctgattgcccgacattatcgcgagcccatttatacccatataaatcagcatccatgttggaatttaatcgcggcctagagcaagacgtttcccgttgaatatggctcataacaccccttgtattactgtttatgtaagcagacagttttattgttcatgaccaaaatcccttaacgtgagttttcgttccactgagcgtcagaccccgtagaaaagatcaaaggatcttcttgagatcctttttttctgcgcgtaatctgctgcttgcaaacaaaaaaaccaccgctaccagcggtggtttgtttgccggatcaagagctaccaactctttttccgaaggtaactggcttcagcagagcgcagataccaaatactgtccttctagtgtagccgtagttaggccaccacttcaagaactctgtagcaccgcctacatacctcgctctgctaatcctgttaccagtggctgctgccagtggcgataagtcgtgtcttaccgggttggactcaagacgatagttaccggataaggcgcagcggtcgggctgaacggggggttcgtgcacacagcccagcttggagcgaacgacctacaccgaactgagatacctacagcgtgagctatgagaaagcgccacgcttcccgaagggagaaaggcggacaggtatccggtaagcggcagggtcggaacaggagagcgcacgagggagcttccagggggaaacgcctggtatctttatagtcctgtcgggtttcgccacctctgacttgagcgtcgatttttgtgatgctcgtcaggggggcggagcctatggaaaaacgccagcaacgcggcctttttacggttcctggccttttgctggccttttgctcacatgttctttcctgcgttatcccctgattctgtggataaccgtattaccgcctttgagtgagctgataccgctcgccgcagccgaacgaccgagcgcagcgagtcagtgagcgaggaagcggaagagcgcctgatgcggtattttctccttacgcatctgtgcggtatttcacaccgcatatatggtgcactctcagtacaatctgctctgatgccgcatagttaagccagtatacactccgctatcgctacgtgactgggtcatggctgcgccccgacacccgccaacacccgctgacgcgccctgacgggcttgtctgctcccggcatccgcttacagacaagctgtgaccgtctccgggagctgcatgtgtcagaggttttcaccgtcatcaccgaaacgcgcgaggcagctgcggtaaagctcatcagcgtggtcgtgaagcgattcacagatgtctgcctgttcatccgcgtccagctcgttgagtttctccagaagcgttaatgtctggcttctgataaagcgggccatgttaagggcggttttttcctgtttggtcactgatgcctccgtgtaagggggatttctgttcatgggggtaatgataccgatgaaacgagagaggatgctcacgatacgggttactgatgatgaacatgcccggttactggaacgttgtgagggtaaacaactggcggtatggatgcggcgggaccagagaaaaatcactcagggtcaatgccagcgcttcgttaatacagatgtaggtgttccacagggtagccagcagcatcctgcgatgcagatccggaacataatggtgcagggcgctgacttccgcgtttccagactttacgaaacacggaaaccgaagaccattcatgttgttgctcaggtcgcagacgttttgcagcagcagtcgcttcacgttcgctcgcgtatcggtgattcattctgctaaccagtaaggcaaccccgccagcctagccgggtcctcaacgacaggagcacgatcatgcgcacccgtggggccgccatgccggcgataatggcctgcttctcgccgaaacgtttggtggcgggaccagtgacgaaggcttgagcgagggcgtgcaagattccgaataccgcaagcgacaggccgatcatcgtcgcgctccagcgaaagcggtcctcgccgaaaatgacccagagcgctgccggcacctgtcctacgagttgcatgataaagaagacagtcataagtgcggcgacgatagtcatgccccgcgcccaccggaaggagctgactgggttgaaggctctcaagggcatcggtcgagatcccggtgcctaatgagtgagctaacttacattaattgcgttgcgctcactgcccgctttccagtcgggaaacctgtcgtgccagctgcattaatgaatcggccaacgcgcggggagaggcggtttgcgtattgggcgccagggtggtttttcttttcaccagtgagacgggcaacagctgattgcccttcaccgcctggccctgagagagttgcagcaagcggtccacgctggtttgccccagcaggcgaaaatcctgtttgatggtggttaacggcgggatataacatgagctgtcttcggtatcgtcgtatcccactaccgagatatccgcaccaacgcgcagcccggactcggtaatggcgcgcattgcgcccagcgccatctgatcgttggcaaccagcatcgcagtgggaacgatgccctcattcagcatttgcatggtttgttgaaaaccggacatggcactccagtcgccttcccgttccgctatcggctgaatttgattgcgagtgagatatttatgccagccagccagacgcagacgcgccgagacagaacttaatgggcccgctaacagcgcgatttgctggtgacccaatgcgaccagatgctccacgcccagtcgcgtaccgtcttcatgggagaaaataatactgttgatgggtgtctggtcagagacatcaagaaataacgccggaacattagtgcaggcagcttccacagcaatggcatcctggtcatccagcggatagttaatgatcagcccactgacgcgttgcgcgagaagattgtgcaccgccgctttacaggcttcgacgccgcttcgttctaccatcgacaccaccacgctggcacccagttgatcggcgcgagatttaatcgccgcgacaatttgcgacggcgcgtgcagggccagactggaggtggcaacgccaatcagcaacgactgtttgcccgccagttgttgtgccacgcggttgggaatgtaattcagctccgccatcgccgcttccactttttcccgcgttttcgcagaaacgtggctggcctggttcaccacgcgggaaacggtctgataagagacaccggcatactctgcgacatcgtataacgttactggtttcacattcaccaccctgaattgactctcttccgggcgctatcatgccataccgcgaaaggttttgcgccattcgatggtgtccgggatctcgacgctctcccttatgcgactcctgcattaggaagcagcccagtagtaggttgaggccgttgagcaccgccgccgcaaggaatggtgcatgcaaggagatggcgcccaacagtcccccggccacggggcctgccaccatacccacgccgaaacaagcgctcatgagcccgaagtggcgagcccgatcttccccatcggtgatgtcggcgatataggcgccagcaaccgcacctgtggcgccggtgatgccggccacgatgcgtccggcgtagaggatcgagatctcgatcccgcgaaattaatacgactcactataggggaattgtgagcggataacaattcccctctagaaataattttgtttaactttaagaaggagatataccatgggcagcagccatcatcatcatcatcacagcagcggcctggtgccgcgcggcagcatgtcggactcagaagtcaatcaagaagctaagccagaggtcaagccagaagtcaagcctgagactcacatcaatttaaaggtgtccgatggatcttcagagatcttcttcaagatcaaaaagaccactcctttaagaaggctgatggaagcgttcgctaaaagacaggggaaggaaatggactccttaagattcttgtacgacggtattagaattcaagctgatcagacccctgaagatttggacatggaggataacgatattattgaggctcacagagaaaagattggtggtcatagtagtcttgaagtcctctttcagggacccaagaagaagaggaaagtcatgatcaaagtttaccgttatgaaatcgttaaaccgctggacctggattggaaagaattcggcaccatcctgcgtcagctgcagcaggaaacccgcttcgcgctgaacaaagcaacccagctggcgtgggaatggatgggtttcagctctgattacaaagacaaccatggcgaatacccgaaaagcaaagacatcctgggctacaccaacgttcacggttacgcataccacaccatcaaaaccaaagcttatcgtctgaacagcggcaacctgagccagaccatcaaacgtgcgaccgatcgcttcaaagcgtaccagaaagaaatcctgcgtggtgacatgtccatcccgtcttacaaacgtgatatcccgctggatctgatcaaagaaaacatcagcgttaaccgtatgaaccacggtgattatatcgcttccctgtccctgctgtctaacccggcgaaacaggaaatgaacgttaaacgtaaaatctccgtgattatcatcgttcgtggcgcgggtaaaaccatcatggatcgcatcctgagcggcgaataccaggtgagcgcgagccagatcatccacgacgaccgtaaaaacaaatggtacctgaacatctcttatgatttcgaaccgcagacccgtgttctggatctgaacaaaatcatgggcatcgatctgggtgttgcggtggcggtgtacatggcgttccagcacaccccggcgcgctacaaactggaaggcggtgaaatcgaaaacttccgtcgtcaggtggagtctcgtcgcatctccatgctgcgccagggtaaatacgcgggtggtgctcgtggcggtcacggccgtgataaacgtatcaaaccgatcgaacagctgcgtgacaaaatcgctaacttccgcgataccactaaccaccgttactctcgttacatcgttgatatggctatcaaagaaggttgcggtaccattcagatggaagatctgaccaacatccgtgatatcggctctcgtttcctgcagaactggacctactacgatctgcagcagaaaatcatctacaaagcggaagaagcgggcatcaaagttatcaaaattgatccgcagtacaccagccagcgttgcagcgaatgcggcaacatcgattccggtaaccgtatcggtcaggcgatcttcaaatgccgtgcttgcggctacgaagcgaacgcggactacaacgcagctcgtaacatcgcgatcccgaacatcgataaaatcatcgcggaaagcatcaaatctggtggttctcccaagaagaagaggaaagtctaagcttaagaattcgagctccgtcgacaagcttgcggccgcactcgagcaccaccaccaccaccactgagatccggctgctaacaaagcccgaaaggaagctgagttggctgctgccaccgctgagcaataactagcataaccccttggggcctctaaacgggtcttgaggggttttttgctgaaaggaggaactatatccggat

SEQ ID NO: 92 - DNA, 1687 bp, Artificial Sequence
  SUMO-AsCas12f-2NLS
gcctggtgccgcgcggcagcatgtcggactcagaagtcaatcaagaagctaagccagaggtcaagccagaagtcaagcctgagactcacatcaatttaaaggtgtccgatggatcttcagagatcttcttcaagatcaaaaagaccactcctttaagaaggctgatggaagcgttcgctaaaagacaggggaaggaaatggactccttaagattcttgtacgacggtattagaattcaagctgatcagacccctgaagatttggacatggaggataacgatattattgaggctcacagagaaaagattggtggtcatagtagtcttgaagtcctctttcagggacccaagaagaagaggaaagtcatgatcaaagtttaccgttatgaaatcgttaaaccgctggacctggattggaaagaattcggcaccatcctgcgtcagctgcagcaggaaacccgcttcgcgctgaacaaagcaacccagctggcgtgggaatggatgggtttcagctctgattacaaagacaaccatggcgaatacccgaaaagcaaagacatcctgggctacaccaacgttcacggttacgcataccacaccatcaaaaccaaagcttatcgtctgaacagcggcaacctgagccagaccatcaaacgtgcgaccgatcgcttcaaagcgtaccagaaagaaatcctgcgtggtgacatgtccatcccgtcttacaaacgtgatatcccgctggatctgatcaaagaaaacatcagcgttaaccgtatgaaccacggtgattatatcgcttccctgtccctgctgtctaacccggcgaaacaggaaatgaacgttaaacgtaaaatctccgtgattatcatcgttcgtggcgcgggtaaaaccatcatggatcgcatcctgagcggcgaataccaggtgagcgcgagccagatcatccacgacgaccgtaaaaacaaatggtacctgaacatctcttatgatttcgaaccgcagacccgtgttctggatctgaacaaaatcatgggcatcgatctgggtgttgcggtggcggtgtacatggcgttccagcacaccccggcgcgctacaaactggaaggcggtgaaatcgaaaacttccgtcgtcaggtggagtctcgtcgcatctccatgctgcgccagggtaaatacgcgggtggtgctcgtggcggtcacggccgtgataaacgtatcaaaccgatcgaacagctgcgtgacaaaatcgctaacttccgcgataccactaaccaccgttactctcgttacatcgttgatatggctatcaaagaaggttgcggtaccattcagatggaagatctgaccaacatccgtgatatcggctctcgtttcctgcagaactggacctactacgatctgcagcagaaaatcatctacaaagcggaagaagcgggcatcaaagttatcaaaattgatccgcagtacaccagccagcgttgcagcgaatgcggcaacatcgattccggtaaccgtatcggtcaggcgatcttcaaatgccgtgcttgcggctacgaagcgaacgcggactacaacgcagctcgtaacatcgcgatcccgaacatcgataaaatcatcgcggaaagcatcaaatctggtggttctcccaagaagaagaggaaagtctaagcttaagaattcgagctccg

SEQ ID NO: 93 - DNA, 24 bp, Artificial Sequence
  Guide1-F
gaacctctcaagacccacaatcca

SEQ ID NO: 94 - DNA, 24 bp, Artificial Sequence
  Guide1-R
aaaatggattgtgggtcttgagag

SEQ ID NO: 95 - DNA, 24 bp, Artificial Sequence
  Guide2-F
gaacaagaagggatgtggtgcatt

SEQ ID NO: 96 - DNA, 24 bp, Artificial Sequence
  Guide2-R
aaaaaatgcaccacatcccttctt

SEQ ID NO: 97 - DNA, 24 bp, Artificial Sequence
  Guide3-F
gaacgctggggagaggagctggtg

SEQ ID NO: 98 - DNA, 24 bp, Artificial Sequence
  Guide3-R
aaaacaccagctcctctccccagc

SEQ ID NO: 99 - DNA, 24 bp, Artificial Sequence
  Guide4-F
gaacaggcatcactgccccctgat

SEQ ID NO: 100 - DNA, 24 bp, Artificial Sequence
  Guide4-R
aaaaatcagggggcagtgatgcct

SEQ ID NO: 101 - DNA, 24 bp, Artificial Sequence
  Guide5-F
gaacagtatacgcttccacagaaa

SEQ ID NO: 102 - DNA, 24 bp, Artificial Sequence
  Guide5-R
aaaatttctgtggaagcgtatact

SEQ ID NO: 103 - DNA, 24 bp, Artificial Sequence
  Guide6-F
gaactggccacatggagtgacctg

SEQ ID NO: 104 - DNA, 24 bp, Artificial Sequence
  Guide6-R
aaaacaggtcactccatgtggcca

SEQ ID NO: 105 - DNA, 24 bp, Artificial Sequence
  Guide7-F
gaacctgtgagctctagtccccac

SEQ ID NO: 106 - DNA, 24 bp, Artificial Sequence
  Guide7-R
aaaagtggggactagagctcacag

SEQ ID NO: 107 - DNA, 6836 bp, Artificial Sequence
  pAsCas12fHs-1
ggtaccgattagtgaacggatctcgacggtatcgatcacgagactagcctcgagcggccgcccccttcaccgagggcctatttcccatgattccttcatatttgcatatacgatacaaggctgttagagagataattggaattaatttgactgtaaacacaaagatattagtacaaaatacgtgacgtagaaagtaataatttcttgggtagtttgcagttttaaaattatgttttaaaatggactatcatatgcttaccgtaacttgaaagtatttcgatttcttggctttatatatcttgtggaaaggacgaaacaccgattcgtcggttcagcgacgataagccgagaagtgccaataaaactgttaagtggtttggtaacgctcggtaaggtagccaaaaggctgaaactccgtgcacaaagaccgcacggacgcttcacatatagctcataaacaagggtttgcgagctagcttgtggagtgtgaacctctcaagacccacaatccatttttttgaattctcgacctcgagacaaatggcagtattcatccacaattttaaaagaaaaggggggattggggggtacagtgcaggggaaagaatagtagacataatagcaacagacatacaaactaaagaattacaaaaacaaattacaaaaattcaaaattttcgggtttattacagggacagcagagatccactttggccgcggctcgagggggttggggttgcgccttttccaaggcagccctgggtttgcgcagggacgcggctgctctgggcgtggttccgggaaacgcagcggcgccgaccctgggactcgcacattcttcacgtccgttcgcagcgtcacccggatcttcgccgctacccttgtgggccccccggcgacgcttcctgctccgcccctaagtcgggaaggttccttgcggttcgcggcgtgccggacgtgacaaacggaagccgcacgtctcactagtaccctcgcagacggacagcgccagggagcaatggcagcgcgccgaccgcgatgggctgtggccaatagcggctgctcagcagggcgcgccgagagcagcggccgggaaggggcggtgcgggaggcggggtgtggggcggtagtgtgggccctgttcctgcccgcgcggtgttccgcattctgcaagcctccggagcgcacgtcggcagtcggctccctcgttgaccgaatcaccgacctctctccccagggggatccaccggagcttaccatgaccgagtacaagcccacggtgcgcctcgccacccgcgacgacgtccccagggccgtacgcaccctcgccgccgcgttcgccgactaccccgccacgcgccacaccgtcgatccggaccgccacatcgagcgggtcaccgagctgcaagaactcttcctcacgcgcgtcgggctcgacatcggcaaggtgtgggtcgcggacgacggcgccgcggtggcggtctggaccacgccggagagcgtcgaagcgggggcggtgttcgccgagatcggcccgcgcatggccgagttgagcggttcccggctggccgcgcagcaacagatggaaggcctcctggcgccgcaccggcccaaggagcccgcgtggttcctggccaccgtcggcgtctcgcccgaccaccagggcaagggtctgggcagcgccgtcgtgctccccggagtggaggcggccgagcgcgccggggtgcccgccttcctggaaacctccgcgccccgcaacctccccttctacgagcggctcggcttcaccgtcaccgccgacgtcgaggtgcccgaaggaccgcgcacctggtgcatgacccgcaagcccggtgcctgacgcccgccccacgacccgcagcgcccgaccgaaaggagcgcacgaccccatgcatcggtacctttaagaccaatgacttacaaggcagctgtagatcttagccactttctagagtcggggcggccggccgcttcgagcagacatgataagatacattgatgagtttggacaaaccacaactagaatgcagtgaaaaaaatgctttatttgtgaaatttgtgatgctattgctttatttgtaaccattataagctgcaataaacaagttaacaacaacaattgcattcattttatgtttcaggttcagggggaggtgtgggaggttttttaaagcaagtaaaacctctacaaatgtggtaaaatcgataaggatccgtcgaccgatgcccttgagagccttcaacccagtcagctccttccggtgggcgcggggcatgactatcgtcgccgcacttatgactgtcttctttatcatgcaactcgtaggacaggtgccggcagcgctcttccgcttcctcgctcactgactcgctgcgctcggtcgttcggctgcggcgagcggtatcagctcactcaaaggcggtaatacggttatccacagaatcaggggataacgcaggaaagaacatgtgagcaaaaggccagcaaaaggccaggaaccgtaaaaaggccgcgttgctggcgtttttccataggctccgcccccctgacgagcatcacaaaaatcgacgctcaagtcagaggtggcgaaacccgacaggactataaagataccaggcgtttccccctggaagctccctcgtgcgctctcctgttccgaccctgccgcttaccggatacctgtccgcctttctcccttcgggaagcgtggcgctttctcaatgctcacgctgtaggtatctcagttcggtgtaggtcgttcgctccaagctgggctgtgtgcacgaaccccccgttcagcccgaccgctgcgccttatccggtaactatcgtcttgagtccaacccggtaagacacgacttatcgccactggcagcagccactggtaacaggattagcagagcgaggtatgtaggcggtgctacagagttcttgaagtggtggcctaactacggctacactagaaggacagtatttggtatctgcgctctgctgaagccagttaccttcggaaaaagagttggtagctcttgatccggcaaacaaaccaccgctggtagcggtggtttttttgtttgcaagcagcagattacgcgcagaaaaaaaggatctcaagaagatcctttgatcttttctacggggtctgacgctcagtggaacgaaaactcacgttaagggattttggtcatgagattatcaaaaaggatcttcacctagatccttttaaattaaaaatgaagttttaaatcaatctaaagtatatatgagtaaacttggtctgacagttaccaatgcttaatcagtgaggcacctatctcagcgatctgtctatttcgttcatccatagttgcctgactccccgtcgtgtagataactacgatacgggagggcttaccatctggccccagtgctgcaatgataccgcgggacccacgctcaccggctccagatttatcagcaataaaccagccagccggaagggccgagcgcagaagtggtcctgcaactttatccgcctccatccagtctattaattgttgccgggaagctagagtaagtagttcgccagttaatagtttgcgcaacgttgttgccattgctacaggcatcgtggtgtcacgctcgtcgtttggtatggcttcattcagctccggttcccaacgatcaaggcgagttacatgatcccccatgttgtgcaaaaaagcggttagctccttcggtcctccgatcgttgtcagaagtaagttggccgcagtgttatcactcatggttatggcagcactgcataattctcttactgtcatgccatccgtaagatgcttttctgtgactggtgagtactcaaccaagtcattctgagaatagtgtatgcggcgaccgagttgctcttgcccggcgtcaatacgggataataccgcgccacatagcagaactttaaaagtgctcatcattggaaaacgttcttcggggcgaaaactctcaaggatcttaccgctgttgagatccagttcgatgtaacccactcgtgcacccaactgatcttcagcatcttttactttcaccagcgtttctgggtgagcaaaaacaggaaggcaaaatgccgcaaaaaagggaataagggcgacacggaaatgttgaatactcatactcttcctttttcaatattattgaagcatttatcagggttattgtctcatgagcggatacatatttgaatgtatttagaaaaataaacaaataggggttccgcgcacatttccccgaaaagtgccacctgcaggaaacagctatgaccatgattacgccaagctctagctagaggtcgacggtatcgagccccagctggttctttccgcctcagaagccatagagcccaccgcatccccagcatgcctgctattgtcttcccaatcctcccccttgctgtcctgccccaccccaccccccagaatagaatgacacctactcagacaatgcgatgcaatttcctcattttattaggaaaggacagtgggagtggcaccttccagggtcaaggaaggcacgggggaggggcaaacaacagatggctggcaactagaaggcacagtcgaggctgatcagcgggtttaaactcaatggtgatggtgatgatgaccggttagactttcctcttcttcttgggagaaccaccagacttaatgctctcggcgatgatcttgtcgatgttggggatggcgatattccgggcggcgttgtagtcggcgttggcctcgtagccgcaggcccggcacttaaagatggcctggccgattctgttgccggagtcgatgttgccgcactcggagcatctctggctggtgtactgggggtcgatcttgatcactttgatgccggcctcctcggccttgtagatgatcttctgctgcaggtcgtagtaggtccagttctgcaggaatctgctgccgatgtctctgatgtttgtcagatcctccatctggattgtgccgcagccctccttgatggccatgtccacgatgtatctgctgtaccggtgattggtggtgtctctgaaattggcgatcttatccctcagctgctcaatgggcttgattctcttgtctctgccgtggccgcccctggcgccgccggcgtacttgccctgtctcagcatggagatgcgccggctctccacctgcctcctgaagttctcaatctcgccgccctccagcttgtacctggcgggggtgtgctggaaggccatgtacacggccacggccacgcccaggtcaatgcccatgatcttgttcaggtccagcactctggtctgtggctcgaagtcgtagctgatgttcaggtaccacttgttcttccggtcgtcgtggataatctggctggcgctcacctggtactcgccggacaggattctgtccatgatggtcttgccggcgcccctcacgatgatgatcacggagatctttctcttcacgttcatctcctgcttggcggggttgctcagcagagacaggctggcgatgtagtcgccgtgattcatcctgttcacggagatgttctccttgatcaggtccagggggatgtccctcttgtagctggggatagacatgtcgccgcgcaggatctccttctggtaggccttgaacctgtctgtggctctcttgatggtctggctcagatttccagagttcagtctgtaggcctttgtcttgatggtgtggtaggcgtagccgtgcacgttggtgtagcccaggatgtccttgctcttggggtactcgccgtggttatccttgtagtcgctgctgaagcccatccactcccaggccagctgtgtggccttattcagggcgaatctggtttcctgctgcagctgtctcaggatggtgccgaactccttccagtccaggtccagaggcttcacgatctcgtatctgtacaccttgatcatgactttcctcttcttcttgggcatggtggcggctctccctatagtgagtcgtattagcggccgcggatctctagcggatctgacggttcactaaaccagctctgcttatatagacctcccaccgtacacgcctaccgcccatttgcgtcaatggggcggagttgttacgacattttggaaagtcccgttgattttggtgccaaaacaaactcccattgacgtcaatggggtggagacttggaaatccccgtgagtcaaaccgctatccacgcccattgatgtactgccaaaaccgcatcaccatggtaatagcgatgactaatacgtagatgtactgccaagtaggaaagtcccataaggtcatgtactgggcataatgccaggcgggccatttaccgtcattgacgtcaatagggggcgtacttggcatatgatacacttgatgtactgccaagtgggcagtttaccgtaaatactccacccattgacgtcaatggaaagtccctattggcgttactatgggaacatacgtcattattgacgtcaatgggcgggggtcgttgggcggtcagccaggcgggccatttaccgtaagttatgtaacgcggaactccatatatgggctatgaactaatgaccccgtaattgattactattaataactagtcaataatcaatgtcaacgcgtatatctggcccgtacatcgcgaagcagcgcaaaacgcctaaccctaagcagattcttcatgcaattgtcggtcaagaatcgatagtactaacatacgctctccatcaaaacaaaacgaaacaaaacaaactagcaaaataggctgtccccagtgcaagtgcaggtgccagaacatttctctatcgata

SEQ ID NO: 108 - DNA, 6836 bp, Artificial Sequence
  pAsCas12fHs-2
ggtaccgattagtgaacggatctcgacggtatcgatcacgagactagcctcgagcggccgcccccttcaccgagggcctatttcccatgattccttcatatttgcatatacgatacaaggctgttagagagataattggaattaatttgactgtaaacacaaagatattagtacaaaatacgtgacgtagaaagtaataatttcttgggtagtttgcagttttaaaattatgttttaaaatggactatcatatgcttaccgtaacttgaaagtatttcgatttcttggctttatatatcttgtggaaaggacgaaacaccgattcgtcggttcagcgacgataagccgagaagtgccaataaaactgttaagtggtttggtaacgctcggtaaggtagccaaaaggctgaaactccgtgcacaaagaccgcacggacgcttcacatatagctcataaacaagggtttgcgagctagcttgtggagtgtgaacaagaagggatgtggtgcatttttttttgaattctcgacctcgagacaaatggcagtattcatccacaattttaaaagaaaaggggggattggggggtacagtgcaggggaaagaatagtagacataatagcaacagacatacaaactaaagaattacaaaaacaaattacaaaaattcaaaattttcgggtttattacagggacagcagagatccactttggccgcggctcgagggggttggggttgcgccttttccaaggcagccctgggtttgcgcagggacgcggctgctctgggcgtggttccgggaaacgcagcggcgccgaccctgggactcgcacattcttcacgtccgttcgcagcgtcacccggatcttcgccgctacccttgtgggccccccggcgacgcttcctgctccgcccctaagtcgggaaggttccttgcggttcgcggcgtgccggacgtgacaaacggaagccgcacgtctcactagtaccctcgcagacggacagcgccagggagcaatggcagcgcgccgaccgcgatgggctgtggccaatagcggctgctcagcagggcgcgccgagagcagcggccgggaaggggcggtgcgggaggcggggtgtggggcggtagtgtgggccctgttcctgcccgcgcggtgttccgcattctgcaagcctccggagcgcacgtcggcagtcggctccctcgttgaccgaatcaccgacctctctccccagggggatccaccggagcttaccatgaccgagtacaagcccacggtgcgcctcgccacccgcgacgacgtccccagggccgtacgcaccctcgccgccgcgttcgccgactaccccgccacgcgccacaccgtcgatccggaccgccacatcgagcgggtcaccgagctgcaagaactcttcctcacgcgcgtcgggctcgacatcggcaaggtgtgggtcgcggacgacggcgccgcggtggcggtctggaccacgccggagagcgtcgaagcgggggcggtgttcgccgagatcggcccgcgcatggccgagttgagcggttcccggctggccgcgcagcaacagatggaaggcctcctggcgccgcaccggcccaaggagcccgcgtggttcctggccaccgtcggcgtctcgcccgaccaccagggcaagggtctgggcagcgccgtcgtgctccccggagtggaggcggccgagcgcgccggggtgcccgccttcctggaaacctccgcgccccgcaacctccccttctacgagcggctcggcttcaccgtcaccgccgacgtcgaggtgcccgaaggaccgcgcacctggtgcatgacccgcaagcccggtgcctgacgcccgccccacgacccgcagcgcccgaccgaaaggagcgcacgaccccatgcatcggtacctttaagaccaatgacttacaaggcagctgtagatcttagccactttctagagtcggggcggccggccgcttcgagcagacatgataagatacattgatgagtttggacaaaccacaactagaatgcagtgaaaaaaatgctttatttgtgaaatttgtgatgctattgctttatttgtaaccattataagctgcaataaacaagttaacaacaacaattgcattcattttatgtttcaggttcagggggaggtgtgggaggttttttaaagcaagtaaaacctctacaaatgtggtaaaatcgataaggatccgtcgaccgatgcccttgagagccttcaacccagtcagctccttccggtgggcgcggggcatgactatcgtcgccgcacttatgactgtcttctttatcatgcaactcgtaggacaggtgccggcagcgctcttccgcttcctcgctcactgactcgctgcgctcggtcgttcggctgcggcgagcggtatcagctcactcaaaggcggtaatacggttatccacagaatcaggggataacgcaggaaagaacatgtgagcaaaaggccagcaaaaggccaggaaccgtaaaaaggccgcgttgctggcgtttttccataggctccgcccccctgacgagcatcacaaaaatcgacgctcaagtcagaggtggcgaaacccgacaggactataaagataccaggcgtttccccctggaagctccctcgtgcgctctcctgttccgaccctgccgcttaccggatacctgtccgcctttctcccttcgggaagcgtggcgctttctcaatgctcacgctgtaggtatctcagttcggtgtaggtcgttcgctccaagctgggctgtgtgcacgaaccccccgttcagcccgaccgctgcgccttatccggtaactatcgtcttgagtccaacccggtaagacacgacttatcgccactggcagcagccactggtaacaggattagcagagcgaggtatgtaggcggtgctacagagttcttgaagtggtggcctaactacggctacactagaaggacagtatttggtatctgcgctctgctgaagccagttaccttcggaaaaagagttggtagctcttgatccggcaaacaaaccaccgctggtagcggtggtttttttgtttgcaagcagcagattacgcgcagaaaaaaaggatctcaagaagatcctttgatcttttctacggggtctgacgctcagtggaacgaaaactcacgttaagggattttggtcatgagattatcaaaaaggatcttcacctagatccttttaaattaaaaatgaagttttaaatcaatctaaagtatatatgagtaaacttggtctgacagttaccaatgcttaatcagtgaggcacctatctcagcgatctgtctatttcgttcatccatagttgcctgactccccgtcgtgtagataactacgatacgggagggcttaccatctggccccagtgctgcaatgataccgcgggacccacgctcaccggctccagatttatcagcaataaaccagccagccggaagggccgagcgcagaagtggtcctgcaactttatccgcctccatccagtctattaattgttgccgggaagctagagtaagtagttcgccagttaatagtttgcgcaacgttgttgccattgctacaggcatcgtggtgtcacgctcgtcgtttggtatggcttcattcagctccggttcccaacgatcaaggcgagttacatgatcccccatgttgtgcaaaaaagcggttagctccttcggtcctccgatcgttgtcagaagtaagttggccgcagtgttatcactcatggttatggcagcactgcataattctcttactgtcatgccatccgtaagatgcttttctgtgactggtgagtactcaaccaagtcattctgagaatagtgtatgcggcgaccgagttgctcttgcccggcgtcaatacgggataataccgcgccacatagcagaactttaaaagtgctcatcattggaaaacgttcttcggggcgaaaactctcaaggatcttaccgctgttgagatccagttcgatgtaacccactcgtgcacccaactgatcttcagcatcttttactttcaccagcgtttctgggtgagcaaaaacaggaaggcaaaatgccgcaaaaaagggaataagggcgacacggaaatgttgaatactcatactcttcctttttcaatattattgaagcatttatcagggttattgtctcatgagcggatacatatttgaatgtatttagaaaaataaacaaataggggttccgcgcacatttccccgaaaagtgccacctgcaggaaacagctatgaccatgattacgccaagctctagctagaggtcgacggtatcgagccccagctggttctttccgcctcagaagccatagagcccaccgcatccccagcatgcctgctattgtcttcccaatcctcccccttgctgtcctgccccaccccaccccccagaatagaatgacacctactcagacaatgcgatgcaatttcctcattttattaggaaaggacagtgggagtggcaccttccagggtcaaggaaggcacgggggaggggcaaacaacagatggctggcaactagaaggcacagtcgaggctgatcagcgggtttaaactcaatggtgatggtgatgatgaccggttagactttcctcttcttcttgggagaaccaccagacttaatgctctcggcgatgatcttgtcgatgttggggatggcgatattccgggcggcgttgtagtcggcgttggcctcgtagccgcaggcccggcacttaaagatggcctggccgattctgttgccggagtcgatgttgccgcactcggagcatctctggctggtgtactgggggtcgatcttgatcactttgatgccggcctcctcggccttgtagatgatcttctgctgcaggtcgtagtaggtccagttctgcaggaatctgctgccgatgtctctgatgtttgtcagatcctccatctggattgtgccgcagccctccttgatggccatgtccacgatgtatctgctgtaccggtgattggtggtgtctctgaaattggcgatcttatccctcagctgctcaatgggcttgattctcttgtctctgccgtggccgcccctggcgccgccggcgtacttgccctgtctcagcatggagatgcgccggctctccacctgcctcctgaagttctcaatctcgccgccctccagcttgtacctggcgggggtgtgctggaaggccatgtacacggccacggccacgcccaggtcaatgcccatgatcttgttcaggtccagcactctggtctgtggctcgaagtcgtagctgatgttcaggtaccacttgttcttccggtcgtcgtggataatctggctggcgctcacctggtactcgccggacaggattctgtccatgatggtcttgccggcgcccctcacgatgatgatcacggagatctttctcttcacgttcatctcctgcttggcggggttgctcagcagagacaggctggcgatgtagtcgccgtgattcatcctgttcacggagatgttctccttgatcaggtccagggggatgtccctcttgtagctggggatagacatgtcgccgcgcaggatctccttctggtaggccttgaacctgtctgtggctctcttgatggtctggctcagatttccagagttcagtctgtaggcctttgtcttgatggtgtggtaggcgtagccgtgcacgttggtgtagcccaggatgtccttgctcttggggtactcgccgtggttatccttgtagtcgctgctgaagcccatccactcccaggccagctgtgtggccttattcagggcgaatctggtttcctgctgcagctgtctcaggatggtgccgaactccttccagtccaggtccagaggcttcacgatctcgtatctgtacaccttgatcatgactttcctcttcttcttgggcatggtggcggctctccctatagtgagtcgtattagcggccgcggatctctagcggatctgacggttcactaaaccagctctgcttatatagacctcccaccgtacacgcctaccgcccatttgcgtcaatggggcggagttgttacgacattttggaaagtcccgttgattttggtgccaaaacaaactcccattgacgtcaatggggtggagacttggaaatccccgtgagtcaaaccgctatccacgcccattgatgtactgccaaaaccgcatcaccatggtaatagcgatgactaatacgtagatgtactgccaagtaggaaagtcccataaggtcatgtactgggcataatgccaggcgggccatttaccgtcattgacgtcaatagggggcgtacttggcatatgatacacttgatgtactgccaagtgggcagtttaccgtaaatactccacccattgacgtcaatggaaagtccctattggcgttactatgggaacatacgtcattattgacgtcaatgggcgggggtcgttgggcggtcagccaggcgggccatttaccgtaagttatgtaacgcggaactccatatatgggctatgaactaatgaccccgtaattgattactattaataactagtcaataatcaatgtcaacgcgtatatctggcccgtacatcgcgaagcagcgcaaaacgcctaaccctaagcagattcttcatgcaattgtcggtcaagaatcgatagtactaacatacgctctccatcaaaacaaaacgaaacaaaacaaactagcaaaataggctgtccccagtgcaagtgcaggtgccagaacatttctctatcgata

SEQ ID NO: 109 - DNA, 6836 bp, Artificial Sequence
  pAsCas12fHs-3
ggtaccgattagtgaacggatctcgacggtatcgatcacgagactagcctcgagcggccgcccccttcaccgagggcctatttcccatgattccttcatatttgcatatacgatacaaggctgttagagagataattggaattaatttgactgtaaacacaaagatattagtacaaaatacgtgacgtagaaagtaataatttcttgggtagtttgcagttttaaaattatgttttaaaatggactatcatatgcttaccgtaacttgaaagtatttcgatttcttggctttatatatcttgtggaaaggacgaaacaccgattcgtcggttcagcgacgataagccgagaagtgccaataaaactgttaagtggtttggtaacgctcggtaaggtagccaaaaggctgaaactccgtgcacaaagaccgcacggacgcttcacatatagctcataaacaagggtttgcgagctagcttgtggagtgtgaacgctggggagaggagctggtgtttttttgaattctcgacctcgagacaaatggcagtattcatccacaattttaaaagaaaaggggggattggggggtacagtgcaggggaaagaatagtagacataatagcaacagacatacaaactaaagaattacaaaaacaaattacaaaaattcaaaattttcgggtttattacagggacagcagagatccactttggccgcggctcgagggggttggggttgcgccttttccaaggcagccctgggtttgcgcagggacgcggctgctctgggcgtggttccgggaaacgcagcggcgccgaccctgggactcgcacattcttcacgtccgttcgcagcgtcacccggatcttcgccgctacccttgtgggccccccggcgacgcttcctgctccgcccctaagtcgggaaggttccttgcggttcgcggcgtgccggacgtgacaaacggaagccgcacgtctcactagtaccctcgcagacggacagcgccagggagcaatggcagcgcgccgaccgcgatgggctgtggccaatagcggctgctcagcagggcgcgccgagagcagcggccgggaaggggcggtgcgggaggcggggtgtggggcggtagtgtgggccctgttcctgcccgcgcggtgttccgcattctgcaagcctccggagcgcacgtcggcagtcggctccctcgttgaccgaatcaccgacctctctccccagggggatccaccggagcttaccatgaccgagtacaagcccacggtgcgcctcgccacccgcgacgacgtccccagggccgtacgcaccctcgccgccgcgttcgccgactaccccgccacgcgccacaccgtcgatccggaccgccacatcgagcgggtcaccgagctgcaagaactcttcctcacgcgcgtcgggctcgacatcggcaaggtgtgggtcgcggacgacggcgccgcggtggcggtctggaccacgccggagagcgtcgaagcgggggcggtgttcgccgagatcggcccgcgcatggccgagttgagcggttcccggctggccgcgcagcaacagatggaaggcctcctggcgccgcaccggcccaaggagcccgcgtggttcctggccaccgtcggcgtctcgcccgaccaccagggcaagggtctgggcagcgccgtcgtgctccccggagtggaggcggccgagcgcgccggggtgcccgccttcctggaaacctccgcgccccgcaacctccccttctacgagcggctcggcttcaccgtcaccgccgacgtcgaggtgcccgaaggaccgcgcacctggtgcatgacccgcaagcccggtgcctgacgcccgccccacgacccgcagcgcccgaccgaaaggagcgcacgaccccatgcatcggtacctttaagaccaatgacttacaaggcagctgtagatcttagccactttctagagtcggggcggccggccgcttcgagcagacatgataagatacattgatgagtttggacaaaccacaactagaatgcagtgaaaaaaatgctttatttgtgaaatttgtgatgctattgctttatttgtaaccattataagctgcaataaacaagttaacaacaacaattgcattcattttatgtttcaggttcagggggaggtgtgggaggttttttaaagcaagtaaaacctctacaaatgtggtaaaatcgataaggatccgtcgaccgatgcccttgagagccttcaacccagtcagctccttccggtgggcgcggggcatgactatcgtcgccgcacttatgactgtcttctttatcatgcaactcgtaggacaggtgccggcagcgctcttccgcttcctcgctcactgactcgctgcgctcggtcgttcggctgcggcgagcggtatcagctcactcaaaggcggtaatacggttatccacagaatcaggggataacgcaggaaagaacatgtgagcaaaaggccagcaaaaggccaggaaccgtaaaaaggccgcgttgctggcgtttttccataggctccgcccccctgacgagcatcacaaaaatcgacgctcaagtcagaggtggcgaaacccgacaggactataaagataccaggcgtttccccctggaagctccctcgtgcgctctcctgttccgaccctgccgcttaccggatacctgtccgcctttctcccttcgggaagcgtggcgctttctcaatgctcacgctgtaggtatctcagttcggtgtaggtcgttcgctccaagctgggctgtgtgcacgaaccccccgttcagcccgaccgctgcgccttatccggtaactatcgtcttgagtccaacccggtaagacacgacttatcgccactggcagcagccactggtaacaggattagcagagcgaggtatgtaggcggtgctacagagttcttgaagtggtggcctaactacggctacactagaaggacagtatttggtatctgcgctctgctgaagccagttaccttcggaaaaagagttggtagctcttgatccggcaaacaaaccaccgctggtagcggtggtttttttgtttgcaagcagcagattacgcgcagaaaaaaaggatctcaagaagatcctttgatcttttctacggggtctgacgctcagtggaacgaaaactcacgttaagggattttggtcatgagattatcaaaaaggatcttcacctagatccttttaaattaaaaatgaagttttaaatcaatctaaagtatatatgagtaaacttggtctgacagttaccaatgcttaatcagtgaggcacctatctcagcgatctgtctatttcgttcatccatagttgcctgactccccgtcgtgtagataactacgatacgggagggcttaccatctggccccagtgctgcaatgataccgcgggacccacgctcaccggctccagatttatcagcaataaaccagccagccggaagggccgagcgcagaagtggtcctgcaactttatccgcctccatccagtctattaattgttgccgggaagctagagtaagtagttcgccagttaatagtttgcgcaacgttgttgccattgctacaggcatcgtggtgtcacgctcgtcgtttggtatggcttcattcagctccggttcccaacgatcaaggcgagttacatgatcccccatgttgtgcaaaaaagcggttagctccttcggtcctccgatcgttgtcagaagtaagttggccgcagtgttatcactcatggttatggcagcactgcataattctcttactgtcatgccatccgtaagatgcttttctgtgactggtgagtactcaaccaagtcattctgagaatagtgtatgcggcgaccgagttgctcttgcccggcgtcaatacgggataataccgcgccacatagcagaactttaaaagtgctcatcattggaaaacgttcttcggggcgaaaactctcaaggatcttaccgctgttgagatccagttcgatgtaacccactcgtgcacccaactgatcttcagcatcttttactttcaccagcgtttctgggtgagcaaaaacaggaaggcaaaatgccgcaaaaaagggaataagggcgacacggaaatgttgaatactcatactcttcctttttcaatattattgaagcatttatcagggttattgtctcatgagcggatacatatttgaatgtatttagaaaaataaacaaataggggttccgcgcacatttccccgaaaagtgccacctgcaggaaacagctatgaccatgattacgccaagctctagctagaggtcgacggtatcgagccccagctggttctttccgcctcagaagccatagagcccaccgcatccccagcatgcctgctattgtcttcccaatcctcccccttgctgtcctgccccaccccaccccccagaatagaatgacacctactcagacaatgcgatgcaatttcctcattttattaggaaaggacagtgggagtggcaccttccagggtcaaggaaggcacgggggaggggcaaacaacagatggctggcaactagaaggcacagtcgaggctgatcagcgggtttaaactcaatggtgatggtgatgatgaccggttagactttcctcttcttcttgggagaaccaccagacttaatgctctcggcgatgatcttgtcgatgttggggatggcgatattccgggcggcgttgtagtcggcgttggcctcgtagccgcaggcccggcacttaaagatggcctggccgattctgttgccggagtcgatgttgccgcactcggagcatctctggctggtgtactgggggtcgatcttgatcactttgatgccggcctcctcggccttgtagatgatcttctgctgcaggtcgtagtaggtccagttctgcaggaatctgctgccgatgtctctgatgtttgtcagatcctccatctggattgtgccgcagccctccttgatggccatgtccacgatgtatctgctgtaccggtgattggtggtgtctctgaaattggcgatcttatccctcagctgctcaatgggcttgattctcttgtctctgccgtggccgcccctggcgccgccggcgtacttgccctgtctcagcatggagatgcgccggctctccacctgcctcctgaagttctcaatctcgccgccctccagcttgtacctggcgggggtgtgctggaaggccatgtacacggccacggccacgcccaggtcaatgcccatgatcttgttcaggtccagcactctggtctgtggctcgaagtcgtagctgatgttcaggtaccacttgttcttccggtcgtcgtggataatctggctggcgctcacctggtactcgccggacaggattctgtccatgatggtcttgccggcgcccctcacgatgatgatcacggagatctttctcttcacgttcatctcctgcttggcggggttgctcagcagagacaggctggcgatgtagtcgccgtgattcatcctgttcacggagatgttctccttgatcaggtccagggggatgtccctcttgtagctggggatagacatgtcgccgcgcaggatctccttctggtaggccttgaacctgtctgtggctctcttgatggtctggctcagatttccagagttcagtctgtaggcctttgtcttgatggtgtggtaggcgtagccgtgcacgttggtgtagcccaggatgtccttgctcttggggtactcgccgtggttatccttgtagtcgctgctgaagcccatccactcccaggccagctgtgtggccttattcagggcgaatctggtttcctgctgcagctgtctcaggatggtgccgaactccttccagtccaggtccagaggcttcacgatctcgtatctgtacaccttgatcatgactttcctcttcttcttgggcatggtggcggctctccctatagtgagtcgtattagcggccgcggatctctagcggatctgacggttcactaaaccagctctgcttatatagacctcccaccgtacacgcctaccgcccatttgcgtcaatggggcggagttgttacgacattttggaaagtcccgttgattttggtgccaaaacaaactcccattgacgtcaatggggtggagacttggaaatccccgtgagtcaaaccgctatccacgcccattgatgtactgccaaaaccgcatcaccatggtaatagcgatgactaatacgtagatgtactgccaagtaggaaagtcccataaggtcatgtactgggcataatgccaggcgggccatttaccgtcattgacgtcaatagggggcgtacttggcatatgatacacttgatgtactgccaagtgggcagtttaccgtaaatactccacccattgacgtcaatggaaagtccctattggcgttactatgggaacatacgtcattattgacgtcaatgggcgggggtcgttgggcggtcagccaggcgggccatttaccgtaagttatgtaacgcggaactccatatatgggctatgaactaatgaccccgtaattgattactattaataactagtcaataatcaatgtcaacgcgtatatctggcccgtacatcgcgaagcagcgcaaaacgcctaaccctaagcagattcttcatgcaattgtcggtcaagaatcgatagtactaacatacgctctccatcaaaacaaaacgaaacaaaacaaactagcaaaataggctgtccccagtgcaagtgcaggtgccagaacatttctctatcgata

SEQ ID NO: 110 - DNA, 6836 bp, Artificial Sequence
  pAsCas12fHs-4
ggtaccgattagtgaacggatctcgacggtatcgatcacgagactagcctcgagcggccgcccccttcaccgagggcctatttcccatgattccttcatatttgcatatacgatacaaggctgttagagagataattggaattaatttgactgtaaacacaaagatattagtacaaaatacgtgacgtagaaagtaataatttcttgggtagtttgcagttttaaaattatgttttaaaatggactatcatatgcttaccgtaacttgaaagtatttcgatttcttggctttatatatcttgtggaaaggacgaaacaccgattcgtcggttcagcgacgataagccgagaagtgccaataaaactgttaagtggtttggtaacgctcggtaaggtagccaaaaggctgaaactccgtgcacaaagaccgcacggacgcttcacatatagctcataaacaagggtttgcgagctagcttgtggagtgtgaacaggcatcactgccccctgattttttttgaattctcgacctcgagacaaatggcagtattcatccacaattttaaaagaaaaggggggattggggggtacagtgcaggggaaagaatagtagacataatagcaacagacatacaaactaaagaattacaaaaacaaattacaaaaattcaaaattttcgggtttattacagggacagcagagatccactttggccgcggctcgagggggttggggttgcgccttttccaaggcagccctgggtttgcgcagggacgcggctgctctgggcgtggttccgggaaacgcagcggcgccgaccctgggactcgcacattcttcacgtccgttcgcagcgtcacccggatcttcgccgctacccttgtgggccccccggcgacgcttcctgctccgcccctaagtcgggaaggttccttgcggttcgcggcgtgccggacgtgacaaacggaagccgcacgtctcactagtaccctcgcagacggacagcgccagggagcaatggcagcgcgccgaccgcgatgggctgtggccaatagcggctgctcagcagggcgcgccgagagcagcggccgggaaggggcggtgcgggaggcggggtgtggggcggtagtgtgggccctgttcctgcccgcgcggtgttccgcattctgcaagcctccggagcgcacgtcggcagtcggctccctcgttgaccgaatcaccgacctctctccccagggggatccaccggagcttaccatgaccgagtacaagcccacggtgcgcctcgccacccgcgacgacgtccccagggccgtacgcaccctcgccgccgcgttcgccgactaccccgccacgcgccacaccgtcgatccggaccgccacatcgagcgggtcaccgagctgcaagaactcttcctcacgcgcgtcgggctcgacatcggcaaggtgtgggtcgcggacgacggcgccgcggtggcggtctggaccacgccggagagcgtcgaagcgggggcggtgttcgccgagatcggcccgcgcatggccgagttgagcggttcccggctggccgcgcagcaacagatggaaggcctcctggcgccgcaccggcccaaggagcccgcgtggttcctggccaccgtcggcgtctcgcccgaccaccagggcaagggtctgggcagcgccgtcgtgctccccggagtggaggcggccgagcgcgccggggtgcccgccttcctggaaacctccgcgccccgcaacctccccttctacgagcggctcggcttcaccgtcaccgccgacgtcgaggtgcccgaaggaccgcgcacctggtgcatgacccgcaagcccggtgcctgacgcccgccccacgacccgcagcgcccgaccgaaaggagcgcacgaccccatgcatcggtacctttaagaccaatgacttacaaggcagctgtagatcttagccactttctagagtcggggcggccggccgcttcgagcagacatgataagatacattgatgagtttggacaaaccacaactagaatgcagtgaaaaaaatgctttatttgtgaaatttgtgatgctattgctttatttgtaaccattataagctgcaataaacaagttaacaacaacaattgcattcattttatgtttcaggttcagggggaggtgtgggaggttttttaaagcaagtaaaacctctacaaatgtggtaaaatcgataaggatccgtcgaccgatgcccttgagagccttcaacccagtcagctccttccggtgggcgcggggcatgactatcgtcgccgcacttatgactgtcttctttatcatgcaactcgtaggacaggtgccggcagcgctcttccgcttcctcgctcactgactcgctgcgctcggtcgttcggctgcggcgagcggtatcagctcactcaaaggcggtaatacggttatccacagaatcaggggataacgcaggaaagaacatgtgagcaaaaggccagcaaaaggccaggaaccgtaaaaaggccgcgttgctggcgtttttccataggctccgcccccctgacgagcatcacaaaaatcgacgctcaagtcagaggtggcgaaacccgacaggactataaagataccaggcgtttccccctggaagctccctcgtgcgctctcctgttccgaccctgccgcttaccggatacctgtccgcctttctcccttcgggaagcgtggcgctttctcaatgctcacgctgtaggtatctcagttcggtgtaggtcgttcgctccaagctgggctgtgtgcacgaaccccccgttcagcccgaccgctgcgccttatccggtaactatcgtcttgagtccaacccggtaagacacgacttatcgccactggcagcagccactggtaacaggattagcagagcgaggtatgtaggcggtgctacagagttcttgaagtggtggcctaactacggctacactagaaggacagtatttggtatctgcgctctgctgaagccagttaccttcggaaaaagagttggtagctcttgatccggcaaacaaaccaccgctggtagcggtggtttttttgtttgcaagcagcagattacgcgcagaaaaaaaggatctcaagaagatcctttgatcttttctacggggtctgacgctcagtggaacgaaaactcacgttaagggattttggtcatgagattatcaaaaaggatcttcacctagatccttttaaattaaaaatgaagttttaaatcaatctaaagtatatatgagtaaacttggtctgacagttaccaatgcttaatcagtgaggcacctatctcagcgatctgtctatttcgttcatccatagttgcctgactccccgtcgtgtagataactacgatacgggagggcttaccatctggccccagtgctgcaatgataccgcgggacccacgctcaccggctccagatttatcagcaataaaccagccagccggaagggccgagcgcagaagtggtcctgcaactttatccgcctccatccagtctattaattgttgccgggaagctagagtaagtagttcgccagttaatagtttgcgcaacgttgttgccattgctacaggcatcgtggtgtcacgctcgtcgtttggtatggcttcattcagctccggttcccaacgatcaaggcgagttacatgatcccccatgttgtgcaaaaaagcggttagctccttcggtcctccgatcgttgtcagaagtaagttggccgcagtgttatcactcatggttatggcagcactgcataattctcttactgtcatgccatccgtaagatgcttttctgtgactggtgagtactcaaccaagtcattctgagaatagtgtatgcggcgaccgagttgctcttgcccggcgtcaatacgggataataccgcgccacatagcagaactttaaaagtgctcatcattggaaaacgttcttcggggcgaaaactctcaaggatcttaccgctgttgagatccagttcgatgtaacccactcgtgcacccaactgatcttcagcatcttttactttcaccagcgtttctgggtgagcaaaaacaggaaggcaaaatgccgcaaaaaagggaataagggcgacacggaaatgttgaatactcatactcttcctttttcaatattattgaagcatttatcagggttattgtctcatgagcggatacatatttgaatgtatttagaaaaataaacaaataggggttccgcgcacatttccccgaaaagtgccacctgcaggaaacagctatgaccatgattacgccaagctctagctagaggtcgacggtatcgagccccagctggttctttccgcctcagaagccatagagcccaccgcatccccagcatgcctgctattgtcttcccaatcctcccccttgctgtcctgccccaccccaccccccagaatagaatgacacctactcagacaatgcgatgcaatttcctcattttattaggaaaggacagtgggagtggcaccttccagggtcaaggaaggcacgggggaggggcaaacaacagatggctggcaactagaaggcacagtcgaggctgatcagcgggtttaaactcaatggtgatggtgatgatgaccggttagactttcctcttcttcttgggagaaccaccagacttaatgctctcggcgatgatcttgtcgatgttggggatggcgatattccgggcggcgttgtagtcggcgttggcctcgtagccgcaggcccggcacttaaagatggcctggccgattctgttgccggagtcgatgttgccgcactcggagcatctctggctggtgtactgggggtcgatcttgatcactttgatgccggcctcctcggccttgtagatgatcttctgctgcaggtcgtagtaggtccagttctgcaggaatctgctgccgatgtctctgatgtttgtcagatcctccatctggattgtgccgcagccctccttgatggccatgtccacgatgtatctgctgtaccggtgattggtggtgtctctgaaattggcgatcttatccctcagctgctcaatgggcttgattctcttgtctctgccgtggccgcccctggcgccgccggcgtacttgccctgtctcagcatggagatgcgccggctctccacctgcctcctgaagttctcaatctcgccgccctccagcttgtacctggcgggggtgtgctggaaggccatgtacacggccacggccacgcccaggtcaatgcccatgatcttgttcaggtccagcactctggtctgtggctcgaagtcgtagctgatgttcaggtaccacttgttcttccggtcgtcgtggataatctggctggcgctcacctggtactcgccggacaggattctgtccatgatggtcttgccggcgcccctcacgatgatgatcacggagatctttctcttcacgttcatctcctgcttggcggggttgctcagcagagacaggctggcgatgtagtcgccgtgattcatcctgttcacggagatgttctccttgatcaggtccagggggatgtccctcttgtagctggggatagacatgtcgccgcgcaggatctccttctggtaggccttgaacctgtctgtggctctcttgatggtctggctcagatttccagagttcagtctgtaggcctttgtcttgatggtgtggtaggcgtagccgtgcacgttggtgtagcccaggatgtccttgctcttggggtactcgccgtggttatccttgtagtcgctgctgaagcccatccactcccaggccagctgtgtggccttattcagggcgaatctggtttcctgctgcagctgtctcaggatggtgccgaactccttccagtccaggtccagaggcttcacgatctcgtatctgtacaccttgatcatgactttcctcttcttcttgggcatggtggcggctctccctatagtgagtcgtattagcggccgcggatctctagcggatctgacggttcactaaaccagctctgcttatatagacctcccaccgtacacgcctaccgcccatttgcgtcaatggggcggagttgttacgacattttggaaagtcccgttgattttggtgccaaaacaaactcccattgacgtcaatggggtggagacttggaaatccccgtgagtcaaaccgctatccacgcccattgatgtactgccaaaaccgcatcaccatggtaatagcgatgactaatacgtagatgtactgccaagtaggaaagtcccataaggtcatgtactgggcataatgccaggcgggccatttaccgtcattgacgtcaatagggggcgtacttggcatatgatacacttgatgtactgccaagtgggcagtttaccgtaaatactccacccattgacgtcaatggaaagtccctattggcgttactatgggaacatacgtcattattgacgtcaatgggcgggggtcgttgggcggtcagccaggcgggccatttaccgtaagttatgtaacgcggaactccatatatgggctatgaactaatgaccccgtaattgattactattaataactagtcaataatcaatgtcaacgcgtatatctggcccgtacatcgcgaagcagcgcaaaacgcctaaccctaagcagattcttcatgcaattgtcggtcaagaatcgatagtactaacatacgctctccatcaaaacaaaacgaaacaaaacaaactagcaaaataggctgtccccagtgcaagtgcaggtgccagaacatttctctatcgata

SEQ ID NO: 111 - DNA, 6836 bp, Artificial Sequence
  pAsCas12fHs-5
ggtaccgattagtgaacggatctcgacggtatcgatcacgagactagcctcgagcggccgcccccttcaccgagggcctatttcccatgattccttcatatttgcatatacgatacaaggctgttagagagataattggaattaatttgactgtaaacacaaagatattagtacaaaatacgtgacgtagaaagtaataatttcttgggtagtttgcagttttaaaattatgttttaaaatggactatcatatgcttaccgtaacttgaaagtatttcgatttcttggctttatatatcttgtggaaaggacgaaacaccgattcgtcggttcagcgacgataagccgagaagtgccaataaaactgttaagtggtttggtaacgctcggtaaggtagccaaaaggctgaaactccgtgcacaaagaccgcacggacgcttcacatatagctcataaacaagggtttgcgagctagcttgtggagtgtgaacagtatacgcttccacagaaatttttttgaattctcgacctcgagacaaatggcagtattcatccacaattttaaaagaaaaggggggattggggggtacagtgcaggggaaagaatagtagacataatagcaacagacatacaaactaaagaattacaaaaacaaattacaaaaattcaaaattttcgggtttattacagggacagcagagatccactttggccgcggctcgagggggttggggttgcgccttttccaaggcagccctgggtttgcgcagggacgcggctgctctgggcgtggttccgggaaacgcagcggcgccgaccctgggactcgcacattcttcacgtccgttcgcagcgtcacccggatcttcgccgctacccttgtgggccccccggcgacgcttcctgctccgcccctaagtcgggaaggttccttgcggttcgcggcgtgccggacgtgacaaacggaagccgcacgtctcactagtaccctcgcagacggacagcgccagggagcaatggcagcgcgccgaccgcgatgggctgtggccaatagcggctgctcagcagggcgcgccgagagcagcggccgggaaggggcggtgcgggaggcggggtgtggggcggtagtgtgggccctgttcctgcccgcgcggtgttccgcattctgcaagcctccggagcgcacgtcggcagtcggctccctcgttgaccgaatcaccgacctctctccccagggggatccaccggagcttaccatgaccgagtacaagcccacggtgcgcctcgccacccgcgacgacgtccccagggccgtacgcaccctcgccgccgcgttcgccgactaccccgccacgcgccacaccgtcgatccggaccgccacatcgagcgggtcaccgagctgcaagaactcttcctcacgcgcgtcgggctcgacatcggcaaggtgtgggtcgcggacgacggcgccgcggtggcggtctggaccacgccggagagcgtcgaagcgggggcggtgttcgccgagatcggcccgcgcatggccgagttgagcggttcccggctggccgcgcagcaacagatggaaggcctcctggcgccgcaccggcccaaggagcccgcgtggttcctggccaccgtcggcgtctcgcccgaccaccagggcaagggtctgggcagcgccgtcgtgctccccggagtggaggcggccgagcgcgccggggtgcccgccttcctggaaacctccgcgccccgcaacctccccttctacgagcggctcggcttcaccgtcaccgccgacgtcgaggtgcccgaaggaccgcgcacctggtgcatgacccgcaagcccggtgcctgacgcccgccccacgacccgcagcgcccgaccgaaaggagcgcacgaccccatgcatcggtacctttaagaccaatgacttacaaggcagctgtagatcttagccactttctagagtcggggcggccggccgcttcgagcagacatgataagatacattgatgagtttggacaaaccacaactagaatgcagtgaaaaaaatgctttatttgtgaaatttgtgatgctattgctttatttgtaaccattataagctgcaataaacaagttaacaacaacaattgcattcattttatgtttcaggttcagggggaggtgtgggaggttttttaaagcaagtaaaacctctacaaatgtggtaaaatcgataaggatccgtcgaccgatgcccttgagagccttcaacccagtcagctccttccggtgggcgcggggcatgactatcgtcgccgcacttatgactgtcttctttatcatgcaactcgtaggacaggtgccggcagcgctcttccgcttcctcgctcactgactcgctgcgctcggtcgttcggctgcggcgagcggtatcagctcactcaaaggcggtaatacggttatccacagaatcaggggataacgcaggaaagaacatgtgagcaaaaggccagcaaaaggccaggaaccgtaaaaaggccgcgttgctggcgtttttccataggctccgcccccctgacgagcatcacaaaaatcgacgctcaagtcagaggtggcgaaacccgacaggactataaagataccaggcgtttccccctggaagctccctcgtgcgctctcctgttccgaccctgccgcttaccggatacctgtccgcctttctcccttcgggaagcgtggcgctttctcaatgctcacgctgtaggtatctcagttcggtgtaggtcgttcgctccaagctgggctgtgtgcacgaaccccccgttcagcccgaccgctgcgccttatccggtaactatcgtcttgagtccaacccggtaagacacgacttatcgccactggcagcagccactggtaacaggattagcagagcgaggtatgtaggcggtgctacagagttcttgaagtggtggcctaactacggctacactagaaggacagtatttggtatctgcgctctgctgaagccagttaccttcggaaaaagagttggtagctcttgatccggcaaacaaaccaccgctggtagcggtggtttttttgtttgcaagcagcagattacgcgcagaaaaaaaggatctcaagaagatcctttgatcttttctacggggtctgacgctcagtggaacgaaaactcacgttaagggattttggtcatgagattatcaaaaaggatcttcacctagatccttttaaattaaaaatgaagttttaaatcaatctaaagtatatatgagtaaacttggtctgacagttaccaatgcttaatcagtgaggcacctatctcagcgatctgtctatttcgttcatccatagttgcctgactccccgtcgtgtagataactacgatacgggagggcttaccatctggccccagtgctgcaatgataccgcgggacccacgctcaccggctccagatttatcagcaataaaccagccagccggaagggccgagcgcagaagtggtcctgcaactttatccgcctccatccagtctattaattgttgccgggaagctagagtaagtagttcgccagttaatagtttgcgcaacgttgttgccattgctacaggcatcgtggtgtcacgctcgtcgtttggtatggcttcattcagctccggttcccaacgatcaaggcgagttacatgatcccccatgttgtgcaaaaaagcggttagctccttcggtcctccgatcgttgtcagaagtaagttggccgcagtgttatcactcatggttatggcagcactgcataattctcttactgtcatgccatccgtaagatgcttttctgtgactggtgagtactcaaccaagtcattctgagaatagtgtatgcggcgaccgagttgctcttgcccggcgtcaatacgggataataccgcgccacatagcagaactttaaaagtgctcatcattggaaaacgttcttcggggcgaaaactctcaaggatcttaccgctgttgagatccagttcgatgtaacccactcgtgcacccaactgatcttcagcatcttttactttcaccagcgtttctgggtgagcaaaaacaggaaggcaaaatgccgcaaaaaagggaataagggcgacacggaaatgttgaatactcatactcttcctttttcaatattattgaagcatttatcagggttattgtctcatgagcggatacatatttgaatgtatttagaaaaataaacaaataggggttccgcgcacatttccccgaaaagtgccacctgcaggaaacagctatgaccatgattacgccaagctctagctagaggtcgacggtatcgagccccagctggttctttccgcctcagaagccatagagcccaccgcatccccagcatgcctgctattgtcttcccaatcctcccccttgctgtcctgccccaccccaccccccagaatagaatgacacctactcagacaatgcgatgcaatttcctcattttattaggaaaggacagtgggagtggcaccttccagggtcaaggaaggcacgggggaggggcaaacaacagatggctggcaactagaaggcacagtcgaggctgatcagcgggtttaaactcaatggtgatggtgatgatgaccggttagactttcctcttcttcttgggagaaccaccagacttaatgctctcggcgatgatcttgtcgatgttggggatggcgatattccgggcggcgttgtagtcggcgttggcctcgtagccgcaggcccggcacttaaagatggcctggccgattctgttgccggagtcgatgttgccgcactcggagcatctctggctggtgtactgggggtcgatcttgatcactttgatgccggcctcctcggccttgtagatgatcttctgctgcaggtcgtagtaggtccagttctgcaggaatctgctgccgatgtctctgatgtttgtcagatcctccatctggattgtgccgcagccctccttgatggccatgtccacgatgtatctgctgtaccggtgattggtggtgtctctgaaattggcgatcttatccctcagctgctcaatgggcttgattctcttgtctctgccgtggccgcccctggcgccgccggcgtacttgccctgtctcagcatggagatgcgccggctctccacctgcctcctgaagttctcaatctcgccgccctccagcttgtacctggcgggggtgtgctggaaggccatgtacacggccacggccacgcccaggtcaatgcccatgatcttgttcaggtccagcactctggtctgtggctcgaagtcgtagctgatgttcaggtaccacttgttcttccggtcgtcgtggataatctggctggcgctcacctggtactcgccggacaggattctgtccatgatggtcttgccggcgcccctcacgatgatgatcacggagatctttctcttcacgttcatctcctgcttggcggggttgctcagcagagacaggctggcgatgtagtcgccgtgattcatcctgttcacggagatgttctccttgatcaggtccagggggatgtccctcttgtagctggggatagacatgtcgccgcgcaggatctccttctggtaggccttgaacctgtctgtggctctcttgatggtctggctcagatttccagagttcagtctgtaggcctttgtcttgatggtgtggtaggcgtagccgtgcacgttggtgtagcccaggatgtccttgctcttggggtactcgccgtggttatccttgtagtcgctgctgaagcccatccactcccaggccagctgtgtggccttattcagggcgaatctggtttcctgctgcagctgtctcaggatggtgccgaactccttccagtccaggtccagaggcttcacgatctcgtatctgtacaccttgatcatgactttcctcttcttcttgggcatggtggcggctctccctatagtgagtcgtattagcggccgcggatctctagcggatctgacggttcactaaaccagctctgcttatatagacctcccaccgtacacgcctaccgcccatttgcgtcaatggggcggagttgttacgacattttggaaagtcccgttgattttggtgccaaaacaaactcccattgacgtcaatggggtggagacttggaaatccccgtgagtcaaaccgctatccacgcccattgatgtactgccaaaaccgcatcaccatggtaatagcgatgactaatacgtagatgtactgccaagtaggaaagtcccataaggtcatgtactgggcataatgccaggcgggccatttaccgtcattgacgtcaatagggggcgtacttggcatatgatacacttgatgtactgccaagtgggcagtttaccgtaaatactccacccattgacgtcaatggaaagtccctattggcgttactatgggaacatacgtcattattgacgtcaatgggcgggggtcgttgggcggtcagccaggcgggccatttaccgtaagttatgtaacgcggaactccatatatgggctatgaactaatgaccccgtaattgattactattaataactagtcaataatcaatgtcaacgcgtatatctggcccgtacatcgcgaagcagcgcaaaacgcctaaccctaagcagattcttcatgcaattgtcggtcaagaatcgatagtactaacatacgctctccatcaaaacaaaacgaaacaaaacaaactagcaaaataggctgtccccagtgcaagtgcaggtgccagaacatttctctatcgata

SEQ ID NO: 112 - DNA, 6836 bp, Artificial Sequence
  pAsCas12fHs-6
ggtaccgattagtgaacggatctcgacggtatcgatcacgagactagcctcgagcggccgcccccttcaccgagggcctatttcccatgattccttcatatttgcatatacgatacaaggctgttagagagataattggaattaatttgactgtaaacacaaagatattagtacaaaatacgtgacgtagaaagtaataatttcttgggtagtttgcagttttaaaattatgttttaaaatggactatcatatgcttaccgtaacttgaaagtatttcgatttcttggctttatatatcttgtggaaaggacgaaacaccgattcgtcggttcagcgacgataagccgagaagtgccaataaaactgttaagtggtttggtaacgctcggtaaggtagccaaaaggctgaaactccgtgcacaaagaccgcacggacgcttcacatatagctcataaacaagggtttgcgagctagcttgtggagtgtgaactggccacatggagtgacctgtttttttgaattctcgacctcgagacaaatggcagtattcatccacaattttaaaagaaaaggggggattggggggtacagtgcaggggaaagaatagtagacataatagcaacagacatacaaactaaagaattacaaaaacaaattacaaaaattcaaaattttcgggtttattacagggacagcagagatccactttggccgcggctcgagggggttggggttgcgccttttccaaggcagccctgggtttgcgcagggacgcggctgctctgggcgtggttccgggaaacgcagcggcgccgaccctgggactcgcacattcttcacgtccgttcgcagcgtcacccggatcttcgccgctacccttgtgggccccccggcgacgcttcctgctccgcccctaagtcgggaaggttccttgcggttcgcggcgtgccggacgtgacaaacggaagccgcacgtctcactagtaccctcgcagacggacagcgccagggagcaatggcagcgcgccgaccgcgatgggctgtggccaatagcggctgctcagcagggcgcgccgagagcagcggccgggaaggggcggtgcgggaggcggggtgtggggcggtagtgtgggccctgttcctgcccgcgcggtgttccgcattctgcaagcctccggagcgcacgtcggcagtcggctccctcgttgaccgaatcaccgacctctctccccagggggatccaccggagcttaccatgaccgagtacaagcccacggtgcgcctcgccacccgcgacgacgtccccagggccgtacgcaccctcgccgccgcgttcgccgactaccccgccacgcgccacaccgtcgatccggaccgccacatcgagcgggtcaccgagctgcaagaactcttcctcacgcgcgtcgggctcgacatcggcaaggtgtgggtcgcggacgacggcgccgcggtggcggtctggaccacgccggagagcgtcgaagcgggggcggtgttcgccgagatcggcccgcgcatggccgagttgagcggttcccggctggccgcgcagcaacagatggaaggcctcctggcgccgcaccggcccaaggagcccgcgtggttcctggccaccgtcggcgtctcgcccgaccaccagggcaagggtctgggcagcgccgtcgtgctccccggagtggaggcggccgagcgcgccggggtgcccgccttcctggaaacctccgcgccccgcaacctccccttctacgagcggctcggcttcaccgtcaccgccgacgtcgaggtgcccgaaggaccgcgcacctggtgcatgacccgcaagcccggtgcctgacgcccgccccacgacccgcagcgcccgaccgaaaggagcgcacgaccccatgcatcggtacctttaagaccaatgacttacaaggcagctgtagatcttagccactttctagagtcggggcggccggccgcttcgagcagacatgataagatacattgatgagtttggacaaaccacaactagaatgcagtgaaaaaaatgctttatttgtgaaatttgtgatgctattgctttatttgtaaccattataagctgcaataaacaagttaacaacaacaattgcattcattttatgtttcaggttcagggggaggtgtgggaggttttttaaagcaagtaaaacctctacaaatgtggtaaaatcgataaggatccgtcgaccgatgcccttgagagccttcaacccagtcagctccttccggtgggcgcggggcatgactatcgtcgccgcacttatgactgtcttctttatcatgcaactcgtaggacaggtgccggcagcgctcttccgcttcctcgctcactgactcgctgcgctcggtcgttcggctgcggcgagcggtatcagctcactcaaaggcggtaatacggttatccacagaatcaggggataacgcaggaaagaacatgtgagcaaaaggccagcaaaaggccaggaaccgtaaaaaggccgcgttgctggcgtttttccataggctccgcccccctgacgagcatcacaaaaatcgacgctcaagtcagaggtggcgaaacccgacaggactataaagataccaggcgtttccccctggaagctccctcgtgcgctctcctgttccgaccctgccgcttaccggatacctgtccgcctttctcccttcgggaagcgtggcgctttctcaatgctcacgctgtaggtatctcagttcggtgtaggtcgttcgctccaagctgggctgtgtgcacgaaccccccgttcagcccgaccgctgcgccttatccggtaactatcgtcttgagtccaacccggtaagacacgacttatcgccactggcagcagccactggtaacaggattagcagagcgaggtatgtaggcggtgctacagagttcttgaagtggtggcctaactacggctacactagaaggacagtatttggtatctgcgctctgctgaagccagttaccttcggaaaaagagttggtagctcttgatccggcaaacaaaccaccgctggtagcggtggtttttttgtttgcaagcagcagattacgcgcagaaaaaaaggatctcaagaagatcctttgatcttttctacggggtctgacgctcagtggaacgaaaactcacgttaagggattttggtcatgagattatcaaaaaggatcttcacctagatccttttaaattaaaaatgaagttttaaatcaatctaaagtatatatgagtaaacttggtctgacagttaccaatgcttaatcagtgaggcacctatctcagcgatctgtctatttcgttcatccatagttgcctgactccccgtcgtgtagataactacgatacgggagggcttaccatctggccccagtgctgcaatgataccgcgggacccacgctcaccggctccagatttatcagcaataaaccagccagccggaagggccgagcgcagaagtggtcctgcaactttatccgcctccatccagtctattaattgttgccgggaagctagagtaagtagttcgccagttaatagtttgcgcaacgttgttgccattgctacaggcatcgtggtgtcacgctcgtcgtttggtatggcttcattcagctccggttcccaacgatcaaggcgagttacatgatcccccatgttgtgcaaaaaagcggttagctccttcggtcctccgatcgttgtcagaagtaagttggccgcagtgttatcactcatggttatggcagcactgcataattctcttactgtcatgccatccgtaagatgcttttctgtgactggtgagtactcaaccaagtcattctgagaatagtgtatgcggcgaccgagttgctcttgcccggcgtcaatacgggataataccgcgccacatagcagaactttaaaagtgctcatcattggaaaacgttcttcggggcgaaaactctcaaggatcttaccgctgttgagatccagttcgatgtaacccactcgtgcacccaactgatcttcagcatcttttactttcaccagcgtttctgggtgagcaaaaacaggaaggcaaaatgccgcaaaaaagggaataagggcgacacggaaatgttgaatactcatactcttcctttttcaatattattgaagcatttatcagggttattgtctcatgagcggatacatatttgaatgtatttagaaaaataaacaaataggggttccgcgcacatttccccgaaaagtgccacctgcaggaaacagctatgaccatgattacgccaagctctagctagaggtcgacggtatcgagccccagctggttctttccgcctcagaagccatagagcccaccgcatccccagcatgcctgctattgtcttcccaatcctcccccttgctgtcctgccccaccccaccccccagaatagaatgacacctactcagacaatgcgatgcaatttcctcattttattaggaaaggacagtgggagtggcaccttccagggtcaaggaaggcacgggggaggggcaaacaacagatggctggcaactagaaggcacagtcgaggctgatcagcgggtttaaactcaatggtgatggtgatgatgaccggttagactttcctcttcttcttgggagaaccaccagacttaatgctctcggcgatgatcttgtcgatgttggggatggcgatattccgggcggcgttgtagtcggcgttggcctcgtagccgcaggcccggcacttaaagatggcctggccgattctgttgccggagtcgatgttgccgcactcggagcatctctggctggtgtactgggggtcgatcttgatcactttgatgccggcctcctcggccttgtagatgatcttctgctgcaggtcgtagtaggtccagttctgcaggaatctgctgccgatgtctctgatgtttgtcagatcctccatctggattgtgccgcagccctccttgatggccatgtccacgatgtatctgctgtaccggtgattggtggtgtctctgaaattggcgatcttatccctcagctgctcaatgggcttgattctcttgtctctgccgtggccgcccctggcgccgccggcgtacttgccctgtctcagcatggagatgcgccggctctccacctgcctcctgaagttctcaatctcgccgccctccagcttgtacctggcgggggtgtgctggaaggccatgtacacggccacggccacgcccaggtcaatgcccatgatcttgttcaggtccagcactctggtctgtggctcgaagtcgtagctgatgttcaggtaccacttgttcttccggtcgtcgtggataatctggctggcgctcacctggtactcgccggacaggattctgtccatgatggtcttgccggcgcccctcacgatgatgatcacggagatctttctcttcacgttcatctcctgcttggcggggttgctcagcagagacaggctggcgatgtagtcgccgtgattcatcctgttcacggagatgttctccttgatcaggtccagggggatgtccctcttgtagctggggatagacatgtcgccgcgcaggatctccttctggtaggccttgaacctgtctgtggctctcttgatggtctggctcagatttccagagttcagtctgtaggcctttgtcttgatggtgtggtaggcgtagccgtgcacgttggtgtagcccaggatgtccttgctcttggggtactcgccgtggttatccttgtagtcgctgctgaagcccatccactcccaggccagctgtgtggccttattcagggcgaatctggtttcctgctgcagctgtctcaggatggtgccgaactccttccagtccaggtccagaggcttcacgatctcgtatctgtacaccttgatcatgactttcctcttcttcttgggcatggtggcggctctccctatagtgagtcgtattagcggccgcggatctctagcggatctgacggttcactaaaccagctctgcttatatagacctcccaccgtacacgcctaccgcccatttgcgtcaatggggcggagttgttacgacattttggaaagtcccgttgattttggtgccaaaacaaactcccattgacgtcaatggggtggagacttggaaatccccgtgagtcaaaccgctatccacgcccattgatgtactgccaaaaccgcatcaccatggtaatagcgatgactaatacgtagatgtactgccaagtaggaaagtcccataaggtcatgtactgggcataatgccaggcgggccatttaccgtcattgacgtcaatagggggcgtacttggcatatgatacacttgatgtactgccaagtgggcagtttaccgtaaatactccacccattgacgtcaatggaaagtccctattggcgttactatgggaacatacgtcattattgacgtcaatgggcgggggtcgttgggcggtcagccaggcgggccatttaccgtaagttatgtaacgcggaactccatatatgggctatgaactaatgaccccgtaattgattactattaataactagtcaataatcaatgtcaacgcgtatatctggcccgtacatcgcgaagcagcgcaaaacgcctaaccctaagcagattcttcatgcaattgtcggtcaagaatcgatagtactaacatacgctctccatcaaaacaaaacgaaacaaaacaaactagcaaaataggctgtccccagtgcaagtgcaggtgccagaacatttctctatcgata

SEQ ID NO: 113 - DNA, 6836 bp, Artificial Sequence
  pAsCas12fHs-7
ggtaccgattagtgaacggatctcgacggtatcgatcacgagactagcctcgagcggccgcccccttcaccgagggcctatttcccatgattccttcatatttgcatatacgatacaaggctgttagagagataattggaattaatttgactgtaaacacaaagatattagtacaaaatacgtgacgtagaaagtaataatttcttgggtagtttgcagttttaaaattatgttttaaaatggactatcatatgcttaccgtaacttgaaagtatttcgatttcttggctttatatatcttgtggaaaggacgaaacaccgattcgtcggttcagcgacgataagccgagaagtgccaataaaactgttaagtggtttggtaacgctcggtaaggtagccaaaaggctgaaactccgtgcacaaagaccgcacggacgcttcacatatagctcataaacaagggtttgcgagctagcttgtggagtgtgaacctgtgagctctagtccccactttttttgaattctcgacctcgagacaaatggcagtattcatccacaattttaaaagaaaaggggggattggggggtacagtgcaggggaaagaatagtagacataatagcaacagacatacaaactaaagaattacaaaaacaaattacaaaaattcaaaattttcgggtttattacagggacagcagagatccactttggccgcggctcgagggggttggggttgcgccttttccaaggcagccctgggtttgcgcagggacgcggctgctctgggcgtggttccgggaaacgcagcggcgccgaccctgggactcgcacattcttcacgtccgttcgcagcgtcacccggatcttcgccgctacccttgtgggccccccggcgacgcttcctgctccgcccctaagtcgggaaggttccttgcggttcgcggcgtgccggacgtgacaaacggaagccgcacgtctcactagtaccctcgcagacggacagcgccagggagcaatggcagcgcgccgaccgcgatgggctgtggccaatagcggctgctcagcagggcgcgccgagagcagcggccgggaaggggcggtgcgggaggcggggtgtggggcggtagtgtgggccctgttcctgcccgcgcggtgttccgcattctgcaagcctccggagcgcacgtcggcagtcggctccctcgttgaccgaatcaccgacctctctccccagggggatccaccggagcttaccatgaccgagtacaagcccacggtgcgcctcgccacccgcgacgacgtccccagggccgtacgcaccctcgccgccgcgttcgccgactaccccgccacgcgccacaccgtcgatccggaccgccacatcgagcgggtcaccgagctgcaagaactcttcctcacgcgcgtcgggctcgacatcggcaaggtgtgggtcgcggacgacggcgccgcggtggcggtctggaccacgccggagagcgtcgaagcgggggcggtgttcgccgagatcggcccgcgcatggccgagttgagcggttcccggctggccgcgcagcaacagatggaaggcctcctggcgccgcaccggcccaaggagcccgcgtggttcctggccaccgtcggcgtctcgcccgaccaccagggcaagggtctgggcagcgccgtcgtgctccccggagtggaggcggccgagcgcgccggggtgcccgccttcctggaaacctccgcgccccgcaacctccccttctacgagcggctcggcttcaccgtcaccgccgacgtcgaggtgcccgaaggaccgcgcacctggtgcatgacccgcaagcccggtgcctgacgcccgccccacgacccgcagcgcccgaccgaaaggagcgcacgaccccatgcatcggtacctttaagaccaatgacttacaaggcagctgtagatcttagccactttctagagtcggggcggccggccgcttcgagcagacatgataagatacattgatgagtttggacaaaccacaactagaatgcagtgaaaaaaatgctttatttgtgaaatttgtgatgctattgctttatttgtaaccattataagctgcaataaacaagttaacaacaacaattgcattcattttatgtttcaggttcagggggaggtgtgggaggttttttaaagcaagtaaaacctctacaaatgtggtaaaatcgataaggatccgtcgaccgatgcccttgagagccttcaacccagtcagctccttccggtgggcgcggggcatgactatcgtcgccgcacttatgactgtcttctttatcatgcaactcgtaggacaggtgccggcagcgctcttccgcttcctcgctcactgactcgctgcgctcggtcgttcggctgcggcgagcggtatcagctcactcaaaggcggtaatacggttatccacagaatcaggggataacgcaggaaagaacatgtgagcaaaaggccagcaaaaggccaggaaccgtaaaaaggccgcgttgctggcgtttttccataggctccgcccccctgacgagcatcacaaaaatcgacgctcaagtcagaggtggcgaaacccgacaggactataaagataccaggcgtttccccctggaagctccctcgtgcgctctcctgttccgaccctgccgcttaccggatacctgtccgcctttctcccttcgggaagcgtggcgctttctcaatgctcacgctgtaggtatctcagttcggtgtaggtcgttcgctccaagctgggctgtgtgcacgaaccccccgttcagcccgaccgctgcgccttatccggtaactatcgtcttgagtccaacccggtaagacacgacttatcgccactggcagcagccactggtaacaggattagcagagcgaggtatgtaggcggtgctacagagttcttgaagtggtggcctaactacggctacactagaaggacagtatttggtatctgcgctctgctgaagccagttaccttcggaaaaagagttggtagctcttgatccggcaaacaaaccaccgctggtagcggtggtttttttgtttgcaagcagcagattacgcgcagaaaaaaaggatctcaagaagatcctttgatcttttctacggggtctgacgctcagtggaacgaaaactcacgttaagggattttggtcatgagattatcaaaaaggatcttcacctagatccttttaaattaaaaatgaagttttaaatcaatctaaagtatatatgagtaaacttggtctgacagttaccaatgcttaatcagtgaggcacctatctcagcgatctgtctatttcgttcatccatagttgcctgactccccgtcgtgtagataactacgatacgggagggcttaccatctggccccagtgctgcaatgataccgcgggacccacgctcaccggctccagatttatcagcaataaaccagccagccggaagggccgagcgcagaagtggtcctgcaactttatccgcctccatccagtctattaattgttgccgggaagctagagtaagtagttcgccagttaatagtttgcgcaacgttgttgccattgctacaggcatcgtggtgtcacgctcgtcgtttggtatggcttcattcagctccggttcccaacgatcaaggcgagttacatgatcccccatgttgtgcaaaaaagcggttagctccttcggtcctccgatcgttgtcagaagtaagttggccgcagtgttatcactcatggttatggcagcactgcataattctcttactgtcatgccatccgtaagatgcttttctgtgactggtgagtactcaaccaagtcattctgagaatagtgtatgcggcgaccgagttgctcttgcccggcgtcaatacgggataataccgcgccacatagcagaactttaaaagtgctcatcattggaaaacgttcttcggggcgaaaactctcaaggatcttaccgctgttgagatccagttcgatgtaacccactcgtgcacccaactgatcttcagcatcttttactttcaccagcgtttctgggtgagcaaaaacaggaaggcaaaatgccgcaaaaaagggaataagggcgacacggaaatgttgaatactcatactcttcctttttcaatattattgaagcatttatcagggttattgtctcatgagcggatacatatttgaatgtatttagaaaaataaacaaataggggttccgcgcacatttccccgaaaagtgccacctgcaggaaacagctatgaccatgattacgccaagctctagctagaggtcgacggtatcgagccccagctggttctttccgcctcagaagccatagagcccaccgcatccccagcatgcctgctattgtcttcccaatcctcccccttgctgtcctgccccaccccaccccccagaatagaatgacacctactcagacaatgcgatgcaatttcctcattttattaggaaaggacagtgggagtggcaccttccagggtcaaggaaggcacgggggaggggcaaacaacagatggctggcaactagaaggcacagtcgaggctgatcagcgggtttaaactcaatggtgatggtgatgatgaccggttagactttcctcttcttcttgggagaaccaccagacttaatgctctcggcgatgatcttgtcgatgttggggatggcgatattccgggcggcgttgtagtcggcgttggcctcgtagccgcaggcccggcacttaaagatggcctggccgattctgttgccggagtcgatgttgccgcactcggagcatctctggctggtgtactgggggtcgatcttgatcactttgatgccggcctcctcggccttgtagatgatcttctgctgcaggtcgtagtaggtccagttctgcaggaatctgctgccgatgtctctgatgtttgtcagatcctccatctggattgtgccgcagccctccttgatggccatgtccacgatgtatctgctgtaccggtgattggtggtgtctctgaaattggcgatcttatccctcagctgctcaatgggcttgattctcttgtctctgccgtggccgcccctggcgccgccggcgtacttgccctgtctcagcatggagatgcgccggctctccacctgcctcctgaagttctcaatctcgccgccctccagcttgtacctggcgggggtgtgctggaaggccatgtacacggccacggccacgcccaggtcaatgcccatgatcttgttcaggtccagcactctggtctgtggctcgaagtcgtagctgatgttcaggtaccacttgttcttccggtcgtcgtggataatctggctggcgctcacctggtactcgccggacaggattctgtccatgatggtcttgccggcgcccctcacgatgatgatcacggagatctttctcttcacgttcatctcctgcttggcggggttgctcagcagagacaggctggcgatgtagtcgccgtgattcatcctgttcacggagatgttctccttgatcaggtccagggggatgtccctcttgtagctggggatagacatgtcgccgcgcaggatctccttctggtaggccttgaacctgtctgtggctctcttgatggtctggctcagatttccagagttcagtctgtaggcctttgtcttgatggtgtggtaggcgtagccgtgcacgttggtgtagcccaggatgtccttgctcttggggtactcgccgtggttatccttgtagtcgctgctgaagcccatccactcccaggccagctgtgtggccttattcagggcgaatctggtttcctgctgcagctgtctcaggatggtgccgaactccttccagtccaggtccagaggcttcacgatctcgtatctgtacaccttgatcatgactttcctcttcttcttgggcatggtggcggctctccctatagtgagtcgtattagcggccgcggatctctagcggatctgacggttcactaaaccagctctgcttatatagacctcccaccgtacacgcctaccgcccatttgcgtcaatggggcggagttgttacgacattttggaaagtcccgttgattttggtgccaaaacaaactcccattgacgtcaatggggtggagacttggaaatccccgtgagtcaaaccgctatccacgcccattgatgtactgccaaaaccgcatcaccatggtaatagcgatgactaatacgtagatgtactgccaagtaggaaagtcccataaggtcatgtactgggcataatgccaggcgggccatttaccgtcattgacgtcaatagggggcgtacttggcatatgatacacttgatgtactgccaagtgggcagtttaccgtaaatactccacccattgacgtcaatggaaagtccctattggcgttactatgggaacatacgtcattattgacgtcaatgggcgggggtcgttgggcggtcagccaggcgggccatttaccgtaagttatgtaacgcggaactccatatatgggctatgaactaatgaccccgtaattgattactattaataactagtcaataatcaatgtcaacgcgtatatctggcccgtacatcgcgaagcagcgcaaaacgcctaaccctaagcagattcttcatgcaattgtcggtcaagaatcgatagtactaacatacgctctccatcaaaacaaaacgaaacaaaacaaactagcaaaataggctgtccccagtgcaagtgcaggtgccagaacatttctctatcgata

SEQ ID NO: 114 - DNA, 214 bp, Artificial Sequence
  sgRNAv1-1
aagctaatacgactcactataggattcgtcggttcagcgacgataagccgagaagtgccaataaaactgttaagtggtttggtaacgctcggtaaggtagccaaaaggctgaaactccgtgcacaaagaccgcacggacgcttcacatatagctcataaacaagggtttgcgagctagcttgtggagtgtgaacctctcaagacccacaatcca

SEQ ID NO: 115 - DNA, 214 bp, Artificial Sequence
  sgRNAv1-2
aagctaatacgactcactataggattcgtcggttcagcgacgataagccgagaagtgccaataaaactgttaagtggtttggtaacgctcggtaaggtagccaaaaggctgaaactccgtgcacaaagaccgcacggacgcttcacatatagctcataaacaagggtttgcgagctagcttgtggagtgtgaacaagaagggatgtggtgcatt

SEQ ID NO: 116 - DNA, 214 bp, Artificial Sequence
  sgRNAv1-3
aagctaatacgactcactataggattcgtcggttcagcgacgataagccgagaagtgccaataaaactgttaagtggtttggtaacgctcggtaaggtagccaaaaggctgaaactccgtgcacaaagaccgcacggacgcttcacatatagctcataaacaagggtttgcgagctagcttgtggagtgtgaacgctggggagaggagctggtg

SEQ ID NO: 117 - DNA, 214 bp, Artificial Sequence
  sgRNAv1-4
aagctaatacgactcactataggattcgtcggttcagcgacgataagccgagaagtgccaataaaactgttaagtggtttggtaacgctcggtaaggtagccaaaaggctgaaactccgtgcacaaagaccgcacggacgcttcacatatagctcataaacaagggtttgcgagctagcttgtggagtgtgaacaggcatcactgccccctgat

SEQ ID NO: 118 - DNA, 214 bp, Artificial Sequence
  sgRNAv1-5
aagctaatacgactcactataggattcgtcggttcagcgacgataagccgagaagtgccaataaaactgttaagtggtttggtaacgctcggtaaggtagccaaaaggctgaaactccgtgcacaaagaccgcacggacgcttcacatatagctcataaacaagggtttgcgagctagcttgtggagtgtgaacagtatacgcttccacagaaa

SEQ ID NO: 119 - DNA, 214 bp, Artificial Sequence
  sgRNAv1-7
aagctaatacgactcactataggattcgtcggttcagcgacgataagccgagaagtgccaataaaactgttaagtggtttggtaacgctcggtaaggtagccaaaaggctgaaactccgtgcacaaagaccgcacggacgcttcacatatagctcataaacaagggtttgcgagctagcttgtggagtgtgaacctgtgagctctagtccccac

SEQ ID NO: 120 - DNA, 1491 bp, Artificial Sequence
  SpCas12f_human optimized
atgggcgagagcgtgaaggccatcaagctgaagatcctggatatgtttctggaccctgagtgtaccaagcaggatgataactggagaaaggacctgagcaccatgagcagattttgcgccgaggccggcaatatgtgcctgagggatctgtataattactttagcatgcctaaggaggataggattagcagcaaggacctgtacaacgccatgtaccacaagaccaagctgctgcaccctgagctgcccggcaaggtggccaaccagatcgtgaaccacgccaaggatgtgtggaagagaaacgccaagctgatctacagaaaccagatcagcatgcctacatacaagattaccacagcccctatcaggctgcagaacaacatctacaagctgatcaagaacaaaaataagtacatcatcgacgtgcagctgtattccaaggagtactccaaggactctggcaagggcacccacaggtacttcctggtggccgtgagagacagcagcacaaggatgatcttcgacaggatcatgtctaaggatcacatcgattccagcaagtcctacacccagggccagctgcagatcaagaaggaccaccagggcaagtggtactgcatcatcccatacaccttcccaacccacgagacagtgctggaccccgacaaggtcatgggcgtggacctgggcgtggccaaggccgtgtactgggccttcaacagcagctacaagcgcggctgcatcgacggcggcgagatcgagcacttccggaagatgatcagagccaggagagtgagcatccagaaccagatcaagcactccggcgacgcaaggaagggccacggcagaaagcgggccctgaagccaatcgaaaccctgtctgagaaggagaagaacttccgggacaccatcaaccacagatacgccaacaggatcgtggaggccgccattaagcagggctgcggcacaatccagatcgagaatctggagggcatcgccgacaccaccggcagcaagttcctgaagaattggccttactacgatctgcagaccaagatcgtgaataaggccaaggagcacggcatcaccgtggtggccatcaaccctcagtacacatcccagagatgttccatgtgcggctacatcgaaaagacaaaccgcagcagccaggccgtgttcgagtgcaagcagtgcggctacggcagcaggaccatctgcatcaactgtagacacgtgcaggtgagcggcgacgtgtgtgaggagtgcggcggcatcgtgaagaaggaaaacgtgaacgccgattacaatgccgccaagaacatcagcaccccctacatcgaccagattatcatggagaagtgcctggagctgggcatcccctacagaagcatcacctgtaaggagtgcggccacatccaggccagcggcaatacctgcgaggtgtgcggcagcaccaacatcctgaagcctaagaagatcagaaaggccaag

SEQ ID NO: 121 - DNA, 7078 bp, Artificial Sequence
  pSpCas12fHs
ggtaccgattagtgaacggatctcgacggtatcgatcacgagactagcctcgagcggccgcccccttcaccgagggcctatttcccatgattccttcatatttgcatatacgatacaaggctgttagagagataattggaattaatttgactgtaaacacaaagatattagtacaaaatacgtgacgtagaaagtaataatttcttgggtagtttgcagttttaaaattatgttttaaaatggactatcatatgcttaccgtaacttgaaagtatttcgatttcttggctttatatatcttgtggaaaggacgaaacaccgaagcctgacataatttactctgtttcgcgcgccagggcagttaggtgccctaaaagagcgaagtggccgaaaggaaaggctaacgcttctctaacgctacggcgaccttggcgaaatgccatcaataccacgcggcccgaaagggttcgcgcgaaactgagtataagcgcgtggattgaaaccgagacccgagagagggtcggtctcctttttttgaattctcgacctcgagacaaatggcagtattcatccacaattttaaaagaaaaggggggattggggggtacagtgcaggggaaagaatagtagacataatagcaacagacatacaaactaaagaattacaaaaacaaattacaaaaattcaaaattttcgggtttattacagggacagcagagatccactttggccgcggctcgagggggttggggttgcgccttttccaaggcagccctgggtttgcgcagggacgcggctgctctgggcgtggttccgggaaacgcagcggcgccgaccctgggactcgcacattcttcacgtccgttcgcagcgtcacccggatcttcgccgctacccttgtgggccccccggcgacgcttcctgctccgcccctaagtcgggaaggttccttgcggttcgcggcgtgccggacgtgacaaacggaagccgcacgtctcactagtaccctcgcagacggacagcgccagggagcaatggcagcgcgccgaccgcgatgggctgtggccaatagcggctgctcagcagggcgcgccgagagcagcggccgggaaggggcggtgcgggaggcggggtgtggggcggtagtgtgggccctgttcctgcccgcgcggtgttccgcattctgcaagcctccggagcgcacgtcggcagtcggctccctcgttgaccgaatcaccgacctctctccccagggggatccaccggagcttaccatgaccgagtacaagcccacggtgcgcctcgccacccgcgacgacgtccccagggccgtacgcaccctcgccgccgcgttcgccgactaccccgccacgcgccacaccgtcgatccggaccgccacatcgagcgggtcaccgagctgcaagaactcttcctcacgcgcgtcgggctcgacatcggcaaggtgtgggtcgcggacgacggcgccgcggtggcggtctggaccacgccggagagcgtcgaagcgggggcggtgttcgccgagatcggcccgcgcatggccgagttgagcggttcccggctggccgcgcagcaacagatggaaggcctcctggcgccgcaccggcccaaggagcccgcgtggttcctggccaccgtcggcgtctcgcccgaccaccagggcaagggtctgggcagcgccgtcgtgctccccggagtggaggcggccgagcgcgccggggtgcccgccttcctggaaacctccgcgccccgcaacctccccttctacgagcggctcggcttcaccgtcaccgccgacgtcgaggtgcccgaaggaccgcgcacctggtgcatgacccgcaagcccggtgcctgacgcccgccccacgacccgcagcgcccgaccgaaaggagcgcacgaccccatgcatcggtacctttaagaccaatgacttacaaggcagctgtagatcttagccactttctagagtcggggcggccggccgcttcgagcagacatgataagatacattgatgagtttggacaaaccacaactagaatgcagtgaaaaaaatgctttatttgtgaaatttgtgatgctattgctttatttgtaaccattataagctgcaataaacaagttaacaacaacaattgcattcattttatgtttcaggttcagggggaggtgtgggaggttttttaaagcaagtaaaacctctacaaatgtggtaaaatcgataaggatccgtcgaccgatgcccttgagagccttcaacccagtcagctccttccggtgggcgcggggcatgactatcgtcgccgcacttatgactgtcttctttatcatgcaactcgtaggacaggtgccggcagcgctcttccgcttcctcgctcactgactcgctgcgctcggtcgttcggctgcggcgagcggtatcagctcactcaaaggcggtaatacggttatccacagaatcaggggataacgcaggaaagaacatgtgagcaaaaggccagcaaaaggccaggaaccgtaaaaaggccgcgttgctggcgtttttccataggctccgcccccctgacgagcatcacaaaaatcgacgctcaagtcagaggtggcgaaacccgacaggactataaagataccaggcgtttccccctggaagctccctcgtgcgctctcctgttccgaccctgccgcttaccggatacctgtccgcctttctcccttcgggaagcgtggcgctttctcaatgctcacgctgtaggtatctcagttcggtgtaggtcgttcgctccaagctgggctgtgtgcacgaaccccccgttcagcccgaccgctgcgccttatccggtaactatcgtcttgagtccaacccggtaagacacgacttatcgccactggcagcagccactggtaacaggattagcagagcgaggtatgtaggcggtgctacagagttcttgaagtggtggcctaactacggctacactagaaggacagtatttggtatctgcgctctgctgaagccagttaccttcggaaaaagagttggtagctcttgatccggcaaacaaaccaccgctggtagcggtggtttttttgtttgcaagcagcagattacgcgcagaaaaaaaggatctcaagaagatcctttgatcttttctacggggtctgacgctcagtggaacgaaaactcacgttaagggattttggtcatgagattatcaaaaaggatcttcacctagatccttttaaattaaaaatgaagttttaaatcaatctaaagtatatatgagtaaacttggtctgacagttaccaatgcttaatcagtgaggcacctatctcagcgatctgtctatttcgttcatccatagttgcctgactccccgtcgtgtagataactacgatacgggagggcttaccatctggccccagtgctgcaatgataccgcgggacccacgctcaccggctccagatttatcagcaataaaccagccagccggaagggccgagcgcagaagtggtcctgcaactttatccgcctccatccagtctattaattgttgccgggaagctagagtaagtagttcgccagttaatagtttgcgcaacgttgttgccattgctacaggcatcgtggtgtcacgctcgtcgtttggtatggcttcattcagctccggttcccaacgatcaaggcgagttacatgatcccccatgttgtgcaaaaaagcggttagctccttcggtcctccgatcgttgtcagaagtaagttggccgcagtgttatcactcatggttatggcagcactgcataattctcttactgtcatgccatccgtaagatgcttttctgtgactggtgagtactcaaccaagtcattctgagaatagtgtatgcggcgaccgagttgctcttgcccggcgtcaatacgggataataccgcgccacatagcagaactttaaaagtgctcatcattggaaaacgttcttcggggcgaaaactctcaaggatcttaccgctgttgagatccagttcgatgtaacccactcgtgcacccaactgatcttcagcatcttttactttcaccagcgtttctgggtgagcaaaaacaggaaggcaaaatgccgcaaaaaagggaataagggcgacacggaaatgttgaatactcatactcttcctttttcaatattattgaagcatttatcagggttattgtctcatgagcggatacatatttgaatgtatttagaaaaataaacaaataggggttccgcgcacatttccccgaaaagtgccacctgcaggaaacagctatgaccatgattacgccaagctctagctagaggtcgacggtatcgagccccagctggttctttccgcctcagaagccatagagcccaccgcatccccagcatgcctgctattgtcttcccaatcctcccccttgctgtcctgccccaccccaccccccagaatagaatgacacctactcagacaatgcgatgcaatttcctcattttattaggaaaggacagtgggagtggcaccttccagggtcaaggaaggcacgggggaggggcaaacaacagatggctggcaactagaaggcacagtcgaggctgatcagcgggtttaaactcaatggtgatggtgatgatgaccggttagactttcctcttcttcttgggagaaccaccagacttggcctttctgatcttcttaggcttcaggatgttggtgctgccgcacacctcgcaggtattgccgctggcctggatgtggccgcactccttacaggtgatgcttctgtaggggatgcccagctccaggcacttctccatgataatctggtcgatgtagggggtgctgatgttcttggcggcattgtaatcggcgttcacgttttccttcttcacgatgccgccgcactcctcacacacgtcgccgctcacctgcacgtgtctacagttgatgcagatggtcctgctgccgtagccgcactgcttgcactcgaacacggcctggctgctgcggtttgtcttttcgatgtagccgcacatggaacatctctgggatgtgtactgagggttgatggccaccacggtgatgccgtgctccttggccttattcacgatcttggtctgcagatcgtagtaaggccaattcttcaggaacttgctgccggtggtgtcggcgatgccctccagattctcgatctggattgtgccgcagccctgcttaatggcggcctccacgatcctgttggcgtatctgtggttgatggtgtcccggaagttcttctccttctcagacagggtttcgattggcttcagggcccgctttctgccgtggcccttccttgcgtcgccggagtgcttgatctggttctggatgctcactctcctggctctgatcatcttccggaagtgctcgatctcgccgccgtcgatgcagccgcgcttgtagctgctgttgaaggcccagtacacggccttggccacgcccaggtccacgcccatgaccttgtcggggtccagcactgtctcgtgggttgggaaggtgtatgggatgatgcagtaccacttgccctggtggtccttcttgatctgcagctggccctgggtgtaggacttgctggaatcgatgtgatccttagacatgatcctgtcgaagatcatccttgtgctgctgtctctcacggccaccaggaagtacctgtgggtgcccttgccagagtccttggagtactccttggaatacagctgcacgtcgatgatgtacttatttttgttcttgatcagcttgtagatgttgttctgcagcctgataggggctgtggtaatcttgtatgtaggcatgctgatctggtttctgtagatcagcttggcgtttctcttccacacatccttggcgtggttcacgatctggttggccaccttgccgggcagctcagggtgcagcagcttggtcttgtggtacatggcgttgtacaggtccttgctgctaatcctatcctccttaggcatgctaaagtaattatacagatccctcaggcacatattgccggcctcggcgcaaaatctgctcatggtgctcaggtcctttctccagttatcatcctgcttggtacactcagggtccagaaacatatccaggatcttcagcttgatggccttcacgctctcgcccatgactttcctcttcttcttgggcatggtggcggctctccctatagtgagtcgtattagcggccgcggatctctagcggatctgacggttcactaaaccagctctgcttatatagacctcccaccgtacacgcctaccgcccatttgcgtcaatggggcggagttgttacgacattttggaaagtcccgttgattttggtgccaaaacaaactcccattgacgtcaatggggtggagacttggaaatccccgtgagtcaaaccgctatccacgcccattgatgtactgccaaaaccgcatcaccatggtaatagcgatgactaatacgtagatgtactgccaagtaggaaagtcccataaggtcatgtactgggcataatgccaggcgggccatttaccgtcattgacgtcaatagggggcgtacttggcatatgatacacttgatgtactgccaagtgggcagtttaccgtaaatactccacccattgacgtcaatggaaagtccctattggcgttactatgggaacatacgtcattattgacgtcaatgggcgggggtcgttgggcggtcagccaggcgggccatttaccgtaagttatgtaacgcggaactccatatatgggctatgaactaatgaccccgtaattgattactattaataactagtcaataatcaatgtcaacgcgtatatctggcccgtacatcgcgaagcagcgcaaaacgcctaaccctaagcagattcttcatgcaattgtcggtcaagaatcgatagtactaacatacgctctccatcaaaacaaaacgaaacaaaacaaactagcaaaataggctgtccccagtgcaagtgcaggtgccagaacatttctctatcgata

SEQ ID NO: 122 - DNA, 7072 bp, Artificial Sequence
  pSpCas12fHs-S1
ggtaccgattagtgaacggatctcgacggtatcgatcacgagactagcctcgagcggccgcccccttcaccgagggcctatttcccatgattccttcatatttgcatatacgatacaaggctgttagagagataattggaattaatttgactgtaaacacaaagatattagtacaaaatacgtgacgtagaaagtaataatttcttgggtagtttgcagttttaaaattatgttttaaaatggactatcatatgcttaccgtaacttgaaagtatttcgatttcttggctttatatatcttgtggaaaggacgaaacaccgaagcctgacataatttactctgtttcgcgcgccagggcagttaggtgccctaaaagagcgaagtggccgaaaggaaaggctaacgcttctctaacgctacggcgaccttggcgaaatgccatcaataccacgcggcccgaaagggttcgcgcgaaactgagtataagcgcgtggattgaaacacacagaggacccctagtaatttttttgaattctcgacctcgagacaaatggcagtattcatccacaattttaaaagaaaaggggggattggggggtacagtgcaggggaaagaatagtagacataatagcaacagacatacaaactaaagaattacaaaaacaaattacaaaaattcaaaattttcgggtttattacagggacagcagagatccactttggccgcggctcgagggggttggggttgcgccttttccaaggcagccctgggtttgcgcagggacgcggctgctctgggcgtggttccgggaaacgcagcggcgccgaccctgggactcgcacattcttcacgtccgttcgcagcgtcacccggatcttcgccgctacccttgtgggccccccggcgacgcttcctgctccgcccctaagtcgggaaggttccttgcggttcgcggcgtgccggacgtgacaaacggaagccgcacgtctcactagtaccctcgcagacggacagcgccagggagcaatggcagcgcgccgaccgcgatgggctgtggccaatagcggctgctcagcagggcgcgccgagagcagcggccgggaaggggcggtgcgggaggcggggtgtggggcggtagtgtgggccctgttcctgcccgcgcggtgttccgcattctgcaagcctccggagcgcacgtcggcagtcggctccctcgttgaccgaatcaccgacctctctccccagggggatccaccggagcttaccatgaccgagtacaagcccacggtgcgcctcgccacccgcgacgacgtccccagggccgtacgcaccctcgccgccgcgttcgccgactaccccgccacgcgccacaccgtcgatccggaccgccacatcgagcgggtcaccgagctgcaagaactcttcctcacgcgcgtcgggctcgacatcggcaaggtgtgggtcgcggacgacggcgccgcggtggcggtctggaccacgccggagagcgtcgaagcgggggcggtgttcgccgagatcggcccgcgcatggccgagttgagcggttcccggctggccgcgcagcaacagatggaaggcctcctggcgccgcaccggcccaaggagcccgcgtggttcctggccaccgtcggcgtctcgcccgaccaccagggcaagggtctgggcagcgccgtcgtgctccccggagtggaggcggccgagcgcgccggggtgcccgccttcctggaaacctccgcgccccgcaacctccccttctacgagcggctcggcttcaccgtcaccgccgacgtcgaggtgcccgaaggaccgcgcacctggtgcatgacccgcaagcccggtgcctgacgcccgccccacgacccgcagcgcccgaccgaaaggagcgcacgaccccatgcatcggtacctttaagaccaatgacttacaaggcagctgtagatcttagccactttctagagtcggggcggccggccgcttcgagcagacatgataagatacattgatgagtttggacaaaccacaactagaatgcagtgaaaaaaatgctttatttgtgaaatttgtgatgctattgctttatttgtaaccattataagctgcaataaacaagttaacaacaacaattgcattcattttatgtttcaggttcagggggaggtgtgggaggttttttaaagcaagtaaaacctctacaaatgtggtaaaatcgataaggatccgtcgaccgatgcccttgagagccttcaacccagtcagctccttccggtgggcgcggggcatgactatcgtcgccgcacttatgactgtcttctttatcatgcaactcgtaggacaggtgccggcagcgctcttccgcttcctcgctcactgactcgctgcgctcggtcgttcggctgcggcgagcggtatcagctcactcaaaggcggtaatacggttatccacagaatcaggggataacgcaggaaagaacatgtgagcaaaaggccagcaaaaggccaggaaccgtaaaaaggccgcgttgctggcgtttttccataggctccgcccccctgacgagcatcacaaaaatcgacgctcaagtcagaggtggcgaaacccgacaggactataaagataccaggcgtttccccctggaagctccctcgtgcgctctcctgttccgaccctgccgcttaccggatacctgtccgcctttctcccttcgggaagcgtggcgctttctcaatgctcacgctgtaggtatctcagttcggtgtaggtcgttcgctccaagctgggctgtgtgcacgaaccccccgttcagcccgaccgctgcgccttatccggtaactatcgtcttgagtccaacccggtaagacacgacttatcgccactggcagcagccactggtaacaggattagcagagcgaggtatgtaggcggtgctacagagttcttgaagtggtggcctaactacggctacactagaaggacagtatttggtatctgcgctctgctgaagccagttaccttcggaaaaagagttggtagctcttgatccggcaaacaaaccaccgctggtagcggtggtttttttgtttgcaagcagcagattacgcgcagaaaaaaaggatctcaagaagatcctttgatcttttctacggggtctgacgctcagtggaacgaaaactcacgttaagggattttggtcatgagattatcaaaaaggatcttcacctagatccttttaaattaaaaatgaagttttaaatcaatctaaagtatatatgagtaaacttggtctgacagttaccaatgcttaatcagtgaggcacctatctcagcgatctgtctatttcgttcatccatagttgcctgactccccgtcgtgtagataactacgatacgggagggcttaccatctggccccagtgctgcaatgataccgcgggacccacgctcaccggctccagatttatcagcaataaaccagccagccggaagggccgagcgcagaagtggtcctgcaactttatccgcctccatccagtctattaattgttgccgggaagctagagtaagtagttcgccagttaatagtttgcgcaacgttgttgccattgctacaggcatcgtggtgtcacgctcgtcgtttggtatggcttcattcagctccggttcccaacgatcaaggcgagttacatgatcccccatgttgtgcaaaaaagcggttagctccttcggtcctccgatcgttgtcagaagtaagttggccgcagtgttatcactcatggttatggcagcactgcataattctcttactgtcatgccatccgtaagatgcttttctgtgactggtgagtactcaaccaagtcattctgagaatagtgtatgcggcgaccgagttgctcttgcccggcgtcaatacgggataataccgcgccacatagcagaactttaaaagtgctcatcattggaaaacgttcttcggggcgaaaactctcaaggatcttaccgctgttgagatccagttcgatgtaacccactcgtgcacccaactgatcttcagcatcttttactttcaccagcgtttctgggtgagcaaaaacaggaaggcaaaatgccgcaaaaaagggaataagggcgacacggaaatgttgaatactcatactcttcctttttcaatattattgaagcatttatcagggttattgtctcatgagcggatacatatttgaatgtatttagaaaaataaacaaataggggttccgcgcacatttccccgaaaagtgccacctgcaggaaacagctatgaccatgattacgccaagctctagctagaggtcgacggtatcgagccccagctggttctttccgcctcagaagccatagagcccaccgcatccccagcatgcctgctattgtcttcccaatcctcccccttgctgtcctgccccaccccaccccccagaatagaatgacacctactcagacaatgcgatgcaatttcctcattttattaggaaaggacagtgggagtggcaccttccagggtcaaggaaggcacgggggaggggcaaacaacagatggctggcaactagaaggcacagtcgaggctgatcagcgggtttaaactcaatggtgatggtgatgatgaccggttagactttcctcttcttcttgggagaaccaccagacttggcctttctgatcttcttaggcttcaggatgttggtgctgccgcacacctcgcaggtattgccgctggcctggatgtggccgcactccttacaggtgatgcttctgtaggggatgcccagctccaggcacttctccatgataatctggtcgatgtagggggtgctgatgttcttggcggcattgtaatcggcgttcacgttttccttcttcacgatgccgccgcactcctcacacacgtcgccgctcacctgcacgtgtctacagttgatgcagatggtcctgctgccgtagccgcactgcttgcactcgaacacggcctggctgctgcggtttgtcttttcgatgtagccgcacatggaacatctctgggatgtgtactgagggttgatggccaccacggtgatgccgtgctccttggccttattcacgatcttggtctgcagatcgtagtaaggccaattcttcaggaacttgctgccggtggtgtcggcgatgccctccagattctcgatctggattgtgccgcagccctgcttaatggcggcctccacgatcctgttggcgtatctgtggttgatggtgtcccggaagttcttctccttctcagacagggtttcgattggcttcagggcccgctttctgccgtggcccttccttgcgtcgccggagtgcttgatctggttctggatgctcactctcctggctctgatcatcttccggaagtgctcgatctcgccgccgtcgatgcagccgcgcttgtagctgctgttgaaggcccagtacacggccttggccacgcccaggtccacgcccatgaccttgtcggggtccagcactgtctcgtgggttgggaaggtgtatgggatgatgcagtaccacttgccctggtggtccttcttgatctgcagctggccctgggtgtaggacttgctggaatcgatgtgatccttagacatgatcctgtcgaagatcatccttgtgctgctgtctctcacggccaccaggaagtacctgtgggtgcccttgccagagtccttggagtactccttggaatacagctgcacgtcgatgatgtacttatttttgttcttgatcagcttgtagatgttgttctgcagcctgataggggctgtggtaatcttgtatgtaggcatgctgatctggtttctgtagatcagcttggcgtttctcttccacacatccttggcgtggttcacgatctggttggccaccttgccgggcagctcagggtgcagcagcttggtcttgtggtacatggcgttgtacaggtccttgctgctaatcctatcctccttaggcatgctaaagtaattatacagatccctcaggcacatattgccggcctcggcgcaaaatctgctcatggtgctcaggtcctttctccagttatcatcctgcttggtacactcagggtccagaaacatatccaggatcttcagcttgatggccttcacgctctcgcccatgactttcctcttcttcttgggcatggtggcggctctccctatagtgagtcgtattagcggccgcggatctctagcggatctgacggttcactaaaccagctctgcttatatagacctcccaccgtacacgcctaccgcccatttgcgtcaatggggcggagttgttacgacattttggaaagtcccgttgattttggtgccaaaacaaactcccattgacgtcaatggggtggagacttggaaatccccgtgagtcaaaccgctatccacgcccattgatgtactgccaaaaccgcatcaccatggtaatagcgatgactaatacgtagatgtactgccaagtaggaaagtcccataaggtcatgtactgggcataatgccaggcgggccatttaccgtcattgacgtcaatagggggcgtacttggcatatgatacacttgatgtactgccaagtgggcagtttaccgtaaatactccacccattgacgtcaatggaaagtccctattggcgttactatgggaacatacgtcattattgacgtcaatgggcgggggtcgttgggcggtcagccaggcgggccatttaccgtaagttatgtaacgcggaactccatatatgggctatgaactaatgaccccgtaattgattactattaataactagtcaataatcaatgtcaacgcgtatatctggcccgtacatcgcgaagcagcgcaaaacgcctaaccctaagcagattcttcatgcaattgtcggtcaagaatcgatagtactaacatacgctctccatcaaaacaaaacgaaacaaaacaaactagcaaaataggctgtccccagtgcaagtgcaggtgccagaacatttctctatcgata

SEQ ID NO: 123 - DNA, 7072 bp, Artificial Sequence
  pSpCas12fHs-S17
ggtaccgattagtgaacggatctcgacggtatcgatcacgagactagcctcgagcggccgcccccttcaccgagggcctatttcccatgattccttcatatttgcatatacgatacaaggctgttagagagataattggaattaatttgactgtaaacacaaagatattagtacaaaatacgtgacgtagaaagtaataatttcttgggtagtttgcagttttaaaattatgttttaaaatggactatcatatgcttaccgtaacttgaaagtatttcgatttcttggctttatatatcttgtggaaaggacgaaacaccgaagcctgacataatttactctgtttcgcgcgccagggcagttaggtgccctaaaagagcgaagtggccgaaaggaaaggctaacgcttctctaacgctacggcgaccttggcgaaatgccatcaataccacgcggcccgaaagggttcgcgcgaaactgagtataagcgcgtggattgaaacaatgcctggcacagcatggttttttttgaattctcgacctcgagacaaatggcagtattcatccacaattttaaaagaaaaggggggattggggggtacagtgcaggggaaagaatagtagacataatagcaacagacatacaaactaaagaattacaaaaacaaattacaaaaattcaaaattttcgggtttattacagggacagcagagatccactttggccgcggctcgagggggttggggttgcgccttttccaaggcagccctgggtttgcgcagggacgcggctgctctgggcgtggttccgggaaacgcagcggcgccgaccctgggactcgcacattcttcacgtccgttcgcagcgtcacccggatcttcgccgctacccttgtgggccccccggcgacgcttcctgctccgcccctaagtcgggaaggttccttgcggttcgcggcgtgccggacgtgacaaacggaagccgcacgtctcactagtaccctcgcagacggacagcgccagggagcaatggcagcgcgccgaccgcgatgggctgtggccaatagcggctgctcagcagggcgcgccgagagcagcggccgggaaggggcggtgcgggaggcggggtgtggggcggtagtgtgggccctgttcctgcccgcgcggtgttccgcattctgcaagcctccggagcgcacgtcggcagtcggctccctcgttgaccgaatcaccgacctctctccccagggggatccaccggagcttaccatgaccgagtacaagcccacggtgcgcctcgccacccgcgacgacgtccccagggccgtacgcaccctcgccgccgcgttcgccgactaccccgccacgcgccacaccgtcgatccggaccgccacatcgagcgggtcaccgagctgcaagaactcttcctcacgcgcgtcgggctcgacatcggcaaggtgtgggtcgcggacgacggcgccgcggtggcggtctggaccacgccggagagcgtcgaagcgggggcggtgttcgccgagatcggcccgcgcatggccgagttgagcggttcccggctggccgcgcagcaacagatggaaggcctcctggcgccgcaccggcccaaggagcccgcgtggttcctggccaccgtcggcgtctcgcccgaccaccagggcaagggtctgggcagcgccgtcgtgctccccggagtggaggcggccgagcgcgccggggtgcccgccttcctggaaacctccgcgccccgcaacctccccttctacgagcggctcggcttcaccgtcaccgccgacgtcgaggtgcccgaaggaccgcgcacctggtgcatgacccgcaagcccggtgcctgacgcccgccccacgacccgcagcgcccgaccgaaaggagcgcacgaccccatgcatcggtacctttaagaccaatgacttacaaggcagctgtagatcttagccactttctagagtcggggcggccggccgcttcgagcagacatgataagatacattgatgagtttggacaaaccacaactagaatgcagtgaaaaaaatgctttatttgtgaaatttgtgatgctattgctttatttgtaaccattataagctgcaataaacaagttaacaacaacaattgcattcattttatgtttcaggttcagggggaggtgtgggaggttttttaaagcaagtaaaacctctacaaatgtggtaaaatcgataaggatccgtcgaccgatgcccttgagagccttcaacccagtcagctccttccggtgggcgcggggcatgactatcgtcgccgcacttatgactgtcttctttatcatgcaactcgtaggacaggtgccggcagcgctcttccgcttcctcgctcactgactcgctgcgctcggtcgttcggctgcggcgagcggtatcagctcactcaaaggcggtaatacggttatccacagaatcaggggataacgcaggaaagaacatgtgagcaaaaggccagcaaaaggccaggaaccgtaaaaaggccgcgttgctggcgtttttccataggctccgcccccctgacgagcatcacaaaaatcgacgctcaagtcagaggtggcgaaacccgacaggactataaagataccaggcgtttccccctggaagctccctcgtgcgctctcctgttccgaccctgccgcttaccggatacctgtccgcctttctcccttcgggaagcgtggcgctttctcaatgctcacgctgtaggtatctcagttcggtgtaggtcgttcgctccaagctgggctgtgtgcacgaaccccccgttcagcccgaccgctgcgccttatccggtaactatcgtcttgagtccaacccggtaagacacgacttatcgccactggcagcagccactggtaacaggattagcagagcgaggtatgtaggcggtgctacagagttcttgaagtggtggcctaactacggctacactagaaggacagtatttggtatctgcgctctgctgaagccagttaccttcggaaaaagagttggtagctcttgatccggcaaacaaaccaccgctggtagcggtggtttttttgtttgcaagcagcagattacgcgcagaaaaaaaggatctcaagaagatcctttgatcttttctacggggtctgacgctcagtggaacgaaaactcacgttaagggattttggtcatgagattatcaaaaaggatcttcacctagatccttttaaattaaaaatgaagttttaaatcaatctaaagtatatatgagtaaacttggtctgacagttaccaatgcttaatcagtgaggcacctatctcagcgatctgtctatttcgttcatccatagttgcctgactccccgtcgtgtagataactacgatacgggagggcttaccatctggccccagtgctgcaatgataccgcgggacccacgctcaccggctccagatttatcagcaataaaccagccagccggaagggccgagcgcagaagtggtcctgcaactttatccgcctccatccagtctattaattgttgccgggaagctagagtaagtagttcgccagttaatagtttgcgcaacgttgttgccattgctacaggcatcgtggtgtcacgctcgtcgtttggtatggcttcattcagctccggttcccaacgatcaaggcgagttacatgatcccccatgttgtgcaaaaaagcggttagctccttcggtcctccgatcgttgtcagaagtaagttggccgcagtgttatcactcatggttatggcagcactgcataattctcttactgtcatgccatccgtaagatgcttttctgtgactggtgagtactcaaccaagtcattctgagaatagtgtatgcggcgaccgagttgctcttgcccggcgtcaatacgggataataccgcgccacatagcagaactttaaaagtgctcatcattggaaaacgttcttcggggcgaaaactctcaaggatcttaccgctgttgagatccagttcgatgtaacccactcgtgcacccaactgatcttcagcatcttttactttcaccagcgtttctgggtgagcaaaaacaggaaggcaaaatgccgcaaaaaagggaataagggcgacacggaaatgttgaatactcatactcttcctttttcaatattattgaagcatttatcagggttattgtctcatgagcggatacatatttgaatgtatttagaaaaataaacaaataggggttccgcgcacatttccccgaaaagtgccacctgcaggaaacagctatgaccatgattacgccaagctctagctagaggtcgacggtatcgagccccagctggttctttccgcctcagaagccatagagcccaccgcatccccagcatgcctgctattgtcttcccaatcctcccccttgctgtcctgccccaccccaccccccagaatagaatgacacctactcagacaatgcgatgcaatttcctcattttattaggaaaggacagtgggagtggcaccttccagggtcaaggaaggcacgggggaggggcaaacaacagatggctggcaactagaaggcacagtcgaggctgatcagcgggtttaaactcaatggtgatggtgatgatgaccggttagactttcctcttcttcttgggagaaccaccagacttggcctttctgatcttcttaggcttcaggatgttggtgctgccgcacacctcgcaggtattgccgctggcctggatgtggccgcactccttacaggtgatgcttctgtaggggatgcccagctccaggcacttctccatgataatctggtcgatgtagggggtgctgatgttcttggcggcattgtaatcggcgttcacgttttccttcttcacgatgccgccgcactcctcacacacgtcgccgctcacctgcacgtgtctacagttgatgcagatggtcctgctgccgtagccgcactgcttgcactcgaacacggcctggctgctgcggtttgtcttttcgatgtagccgcacatggaacatctctgggatgtgtactgagggttgatggccaccacggtgatgccgtgctccttggccttattcacgatcttggtctgcagatcgtagtaaggccaattcttcaggaacttgctgccggtggtgtcggcgatgccctccagattctcgatctggattgtgccgcagccctgcttaatggcggcctccacgatcctgttggcgtatctgtggttgatggtgtcccggaagttcttctccttctcagacagggtttcgattggcttcagggcccgctttctgccgtggcccttccttgcgtcgccggagtgcttgatctggttctggatgctcactctcctggctctgatcatcttccggaagtgctcgatctcgccgccgtcgatgcagccgcgcttgtagctgctgttgaaggcccagtacacggccttggccacgcccaggtccacgcccatgaccttgtcggggtccagcactgtctcgtgggttgggaaggtgtatgggatgatgcagtaccacttgccctggtggtccttcttgatctgcagctggccctgggtgtaggacttgctggaatcgatgtgatccttagacatgatcctgtcgaagatcatccttgtgctgctgtctctcacggccaccaggaagtacctgtgggtgcccttgccagagtccttggagtactccttggaatacagctgcacgtcgatgatgtacttatttttgttcttgatcagcttgtagatgttgttctgcagcctgataggggctgtggtaatcttgtatgtaggcatgctgatctggtttctgtagatcagcttggcgtttctcttccacacatccttggcgtggttcacgatctggttggccaccttgccgggcagctcagggtgcagcagcttggtcttgtggtacatggcgttgtacaggtccttgctgctaatcctatcctccttaggcatgctaaagtaattatacagatccctcaggcacatattgccggcctcggcgcaaaatctgctcatggtgctcaggtcctttctccagttatcatcctgcttggtacactcagggtccagaaacatatccaggatcttcagcttgatggccttcacgctctcgcccatgactttcctcttcttcttgggcatggtggcggctctccctatagtgagtcgtattagcggccgcggatctctagcggatctgacggttcactaaaccagctctgcttatatagacctcccaccgtacacgcctaccgcccatttgcgtcaatggggcggagttgttacgacattttggaaagtcccgttgattttggtgccaaaacaaactcccattgacgtcaatggggtggagacttggaaatccccgtgagtcaaaccgctatccacgcccattgatgtactgccaaaaccgcatcaccatggtaatagcgatgactaatacgtagatgtactgccaagtaggaaagtcccataaggtcatgtactgggcataatgccaggcgggccatttaccgtcattgacgtcaatagggggcgtacttggcatatgatacacttgatgtactgccaagtgggcagtttaccgtaaatactccacccattgacgtcaatggaaagtccctattggcgttactatgggaacatacgtcattattgacgtcaatgggcgggggtcgttgggcggtcagccaggcgggccatttaccgtaagttatgtaacgcggaactccatatatgggctatgaactaatgaccccgtaattgattactattaataactagtcaataatcaatgtcaacgcgtatatctggcccgtacatcgcgaagcagcgcaaaacgcctaaccctaagcagattcttcatgcaattgtcggtcaagaatcgatagtactaacatacgctctccatcaaaacaaaacgaaacaaaacaaactagcaaaataggctgtccccagtgcaagtgcaggtgccagaacatttctctatcgata

SEQ ID NO: 124 - DNA, 7072 bp, Artificial Sequence
  pspcas12fhs-s34
ggtaccgattagtgaacggatctcgacggtatcgatcacgagactagcctcgagcggccgcccccttcaccgagggcctatttcccatgattccttcatatttgcatatacgatacaaggctgttagagagataattggaattaatttgactgtaaacacaaagatattagtacaaaatacgtgacgtagaaagtaataatttcttgggtagtttgcagttttaaaattatgttttaaaatggactatcatatgcttaccgtaacttgaaagtatttcgatttcttggctttatatatcttgtggaaaggacgaaacaccgaagcctgacataatttactctgtttcgcgcgccagggcagttaggtgccctaaaagagcgaagtggccgaaaggaaaggctaacgcttctctaacgctacggcgaccttggcgaaatgccatcaataccacgcggcccgaaagggttcgcgcgaaactgagtataagcgcgtggattgaaacctcttggggaaatgattctttttttttgaattctcgacctcgagacaaatggcagtattcatccacaattttaaaagaaaaggggggattggggggtacagtgcaggggaaagaatagtagacataatagcaacagacatacaaactaaagaattacaaaaacaaattacaaaaattcaaaattttcgggtttattacagggacagcagagatccactttggccgcggctcgagggggttggggttgcgccttttccaaggcagccctgggtttgcgcagggacgcggctgctctgggcgtggttccgggaaacgcagcggcgccgaccctgggactcgcacattcttcacgtccgttcgcagcgtcacccggatcttcgccgctacccttgtgggccccccggcgacgcttcctgctccgcccctaagtcgggaaggttccttgcggttcgcggcgtgccggacgtgacaaacggaagccgcacgtctcactagtaccctcgcagacggacagcgccagggagcaatggcagcgcgccgaccgcgatgggctgtggccaatagcggctgctcagcagggcgcgccgagagcagcggccgggaaggggcggtgcgggaggcggggtgtggggcggtagtgtgggccctgttcctgcccgcgcggtgttccgcattctgcaagcctccggagcgcacgtcggcagtcggctccctcgttgaccgaatcaccgacctctctccccagggggatccaccggagcttaccatgaccgagtacaagcccacggtgcgcctcgccacccgcgacgacgtccccagggccgtacgcaccctcgccgccgcgttcgccgactaccccgccacgcgccacaccgtcgatccggaccgccacatcgagcgggtcaccgagctgcaagaactcttcctcacgcgcgtcgggctcgacatcggcaaggtgtgggtcgcggacgacggcgccgcggtggcggtctggaccacgccggagagcgtcgaagcgggggcggtgttcgccgagatcggcccgcgcatggccgagttgagcggttcccggctggccgcgcagcaacagatggaaggcctcctggcgccgcaccggcccaaggagcccgcgtggttcctggccaccgtcggcgtctcgcccgaccaccagggcaagggtctgggcagcgccgtcgtgctccccggagtggaggcggccgagcgcgccggggtgcccgccttcctggaaacctccgcgccccgcaacctccccttctacgagcggctcggcttcaccgtcaccgccgacgtcgaggtgcccgaaggaccgcgcacctggtgcatgacccgcaagcccggtgcctgacgcccgccccacgacccgcagcgcccgaccgaaaggagcgcacgaccccatgcatcggtacctttaagaccaatgacttacaaggcagctgtagatcttagccactttctagagtcggggcggccggccgcttcgagcagacatgataagatacattgatgagtttggacaaaccacaactagaatgcagtgaaaaaaatgctttatttgtgaaatttgtgatgctattgctttatttgtaaccattataagctgcaataaacaagttaacaacaacaattgcattcattttatgtttcaggttcagggggaggtgtgggaggttttttaaagcaagtaaaacctctacaaatgtggtaaaatcgataaggatccgtcgaccgatgcccttgagagccttcaacccagtcagctccttccggtgggcgcggggcatgactatcgtcgccgcacttatgactgtcttctttatcatgcaactcgtaggacaggtgccggcagcgctcttccgcttcctcgctcactgactcgctgcgctcggtcgttcggctgcggcgagcggtatcagctcactcaaaggcggtaatacggttatccacagaatcaggggataacgcaggaaagaacatgtgagcaaaaggccagcaaaaggccaggaaccgtaaaaaggccgcgttgctggcgtttttccataggctccgcccccctgacgagcatcacaaaaatcgacgctcaagtcagaggtggcgaaacccgacaggactataaagataccaggcgtttccccctggaagctccctcgtgcgctctcctgttccgaccctgccgcttaccggatacctgtccgcctttctcccttcgggaagcgtggcgctttctcaatgctcacgctgtaggtatctcagttcggtgtaggtcgttcgctccaagctgggctgtgtgcacgaaccccccgttcagcccgaccgctgcgccttatccggtaactatcgtcttgagtccaacccggtaagacacgacttatcgccactggcagcagccactggtaacaggattagcagagcgaggtatgtaggcggtgctacagagttcttgaagtggtggcctaactacggctacactagaaggacagtatttggtatctgcgctctgctgaagccagttaccttcggaaaaagagttggtagctcttgatccggcaaacaaaccaccgctggtagcggtggtttttttgtttgcaagcagcagattacgcgcagaaaaaaaggatctcaagaagatcctttgatcttttctacggggtctgacgctcagtggaacgaaaactcacgttaagggattttggtcatgagattatcaaaaaggatcttcacctagatccttttaaattaaaaatgaagttttaaatcaatctaaagtatatatgagtaaacttggtctgacagttaccaatgcttaatcagtgaggcacctatctcagcgatctgtctatttcgttcatccatagttgcctgactccccgtcgtgtagataactacgatacgggagggcttaccatctggccccagtgctgcaatgataccgcgggacccacgctcaccggctccagatttatcagcaataaaccagccagccggaagggccgagcgcagaagtggtcctgcaactttatccgcctccatccagtctattaattgttgccgggaagctagagtaagtagttcgccagttaatagtttgcgcaacgttgttgccattgctacaggcatcgtggtgtcacgctcgtcgtttggtatggcttcattcagctccggttcccaacgatcaaggcgagttacatgatcccccatgttgtgcaaaaaagcggttagctccttcggtcctccgatcgttgtcagaagtaagttggccgcagtgttatcactcatggttatggcagcactgcataattctcttactgtcatgccatccgtaagatgcttttctgtgactggtgagtactcaaccaagtcattctgagaatagtgtatgcggcgaccgagttgctcttgcccggcgtcaatacgggataataccgcgccacatagcagaactttaaaagtgctcatcattggaaaacgttcttcggggcgaaaactctcaaggatcttaccgctgttgagatccagttcgatgtaacccactcgtgcacccaactgatcttcagcatcttttactttcaccagcgtttctgggtgagcaaaaacaggaaggcaaaatgccgcaaaaaagggaataagggcgacacggaaatgttgaatactcatactcttcctttttcaatattattgaagcatttatcagggttattgtctcatgagcggatacatatttgaatgtatttagaaaaataaacaaataggggttccgcgcacatttccccgaaaagtgccacctgcaggaaacagctatgaccatgattacgccaagctctagctagaggtcgacggtatcgagccccagctggttctttccgcctcagaagccatagagcccaccgcatccccagcatgcctgctattgtcttcccaatcctcccccttgctgtcctgccccaccccaccccccagaatagaatgacacctactcagacaatgcgatgcaatttcctcattttattaggaaaggacagtgggagtggcaccttccagggtcaaggaaggcacgggggaggggcaaacaacagatggctggcaactagaaggcacagtcgaggctgatcagcgggtttaaactcaatggtgatggtgatgatgaccggttagactttcctcttcttcttgggagaaccaccagacttggcctttctgatcttcttaggcttcaggatgttggtgctgccgcacacctcgcaggtattgccgctggcctggatgtggccgcactccttacaggtgatgcttctgtaggggatgcccagctccaggcacttctccatgataatctggtcgatgtagggggtgctgatgttcttggcggcattgtaatcggcgttcacgttttccttcttcacgatgccgccgcactcctcacacacgtcgccgctcacctgcacgtgtctacagttgatgcagatggtcctgctgccgtagccgcactgcttgcactcgaacacggcctggctgctgcggtttgtcttttcgatgtagccgcacatggaacatctctgggatgtgtactgagggttgatggccaccacggtgatgccgtgctccttggccttattcacgatcttggtctgcagatcgtagtaaggccaattcttcaggaacttgctgccggtggtgtcggcgatgccctccagattctcgatctggattgtgccgcagccctgcttaatggcggcctccacgatcctgttggcgtatctgtggttgatggtgtcccggaagttcttctccttctcagacagggtttcgattggcttcagggcccgctttctgccgtggcccttccttgcgtcgccggagtgcttgatctggttctggatgctcactctcctggctctgatcatcttccggaagtgctcgatctcgccgccgtcgatgcagccgcgcttgtagctgctgttgaaggcccagtacacggccttggccacgcccaggtccacgcccatgaccttgtcggggtccagcactgtctcgtgggttgggaaggtgtatgggatgatgcagtaccacttgccctggtggtccttcttgatctgcagctggccctgggtgtaggacttgctggaatcgatgtgatccttagacatgatcctgtcgaagatcatccttgtgctgctgtctctcacggccaccaggaagtacctgtgggtgcccttgccagagtccttggagtactccttggaatacagctgcacgtcgatgatgtacttatttttgttcttgatcagcttgtagatgttgttctgcagcctgataggggctgtggtaatcttgtatgtaggcatgctgatctggtttctgtagatcagcttggcgtttctcttccacacatccttggcgtggttcacgatctggttggccaccttgccgggcagctcagggtgcagcagcttggtcttgtggtacatggcgttgtacaggtccttgctgctaatcctatcctccttaggcatgctaaagtaattatacagatccctcaggcacatattgccggcctcggcgcaaaatctgctcatggtgctcaggtcctttctccagttatcatcctgcttggtacactcagggtccagaaacatatccaggatcttcagcttgatggccttcacgctctcgcccatgactttcctcttcttcttgggcatggtggcggctctccctatagtgagtcgtattagcggccgcggatctctagcggatctgacggttcactaaaccagctctgcttatatagacctcccaccgtacacgcctaccgcccatttgcgtcaatggggcggagttgttacgacattttggaaagtcccgttgattttggtgccaaaacaaactcccattgacgtcaatggggtggagacttggaaatccccgtgagtcaaaccgctatccacgcccattgatgtactgccaaaaccgcatcaccatggtaatagcgatgactaatacgtagatgtactgccaagtaggaaagtcccataaggtcatgtactgggcataatgccaggcgggccatttaccgtcattgacgtcaatagggggcgtacttggcatatgatacacttgatgtactgccaagtgggcagtttaccgtaaatactccacccattgacgtcaatggaaagtccctattggcgttactatgggaacatacgtcattattgacgtcaatgggcgggggtcgttgggcggtcagccaggcgggccatttaccgtaagttatgtaacgcggaactccatatatgggctatgaactaatgaccccgtaattgattactattaataactagtcaataatcaatgtcaacgcgtatatctggcccgtacatcgcgaagcagcgcaaaacgcctaaccctaagcagattcttcatgcaattgtcggtcaagaatcgatagtactaacatacgctctccatcaaaacaaaacgaaacaaaacaaactagcaaaataggctgtccccagtgcaagtgcaggtgccagaacatttctctatcgata

SEQ ID NO: 125 - DNA, 7072 bp, Artificial Sequence
  pSpCas12fHs-S37
ggtaccgattagtgaacggatctcgacggtatcgatcacgagactagcctcgagcggccgcccccttcaccgagggcctatttcccatgattccttcatatttgcatatacgatacaaggctgttagagagataattggaattaatttgactgtaaacacaaagatattagtacaaaatacgtgacgtagaaagtaataatttcttgggtagtttgcagttttaaaattatgttttaaaatggactatcatatgcttaccgtaacttgaaagtatttcgatttcttggctttatatatcttgtggaaaggacgaaacaccgaagcctgacataatttactctgtttcgcgcgccagggcagttaggtgccctaaaagagcgaagtggccgaaaggaaaggctaacgcttctctaacgctacggcgaccttggcgaaatgccatcaataccacgcggcccgaaagggttcgcgcgaaactgagtataagcgcgtggattgaaactcttgaaggggacaggctactttttttgaattctcgacctcgagacaaatggcagtattcatccacaattttaaaagaaaaggggggattggggggtacagtgcaggggaaagaatagtagacataatagcaacagacatacaaactaaagaattacaaaaacaaattacaaaaattcaaaattttcgggtttattacagggacagcagagatccactttggccgcggctcgagggggttggggttgcgccttttccaaggcagccctgggtttgcgcagggacgcggctgctctgggcgtggttccgggaaacgcagcggcgccgaccctgggactcgcacattcttcacgtccgttcgcagcgtcacccggatcttcgccgctacccttgtgggccccccggcgacgcttcctgctccgcccctaagtcgggaaggttccttgcggttcgcggcgtgccggacgtgacaaacggaagccgcacgtctcactagtaccctcgcagacggacagcgccagggagcaatggcagcgcgccgaccgcgatgggctgtggccaatagcggctgctcagcagggcgcgccgagagcagcggccgggaaggggcggtgcgggaggcggggtgtggggcggtagtgtgggccctgttcctgcccgcgcggtgttccgcattctgcaagcctccggagcgcacgtcggcagtcggctccctcgttgaccgaatcaccgacctctctccccagggggatccaccggagcttaccatgaccgagtacaagcccacggtgcgcctcgccacccgcgacgacgtccccagggccgtacgcaccctcgccgccgcgttcgccgactaccccgccacgcgccacaccgtcgatccggaccgccacatcgagcgggtcaccgagctgcaagaactcttcctcacgcgcgtcgggctcgacatcggcaaggtgtgggtcgcggacgacggcgccgcggtggcggtctggaccacgccggagagcgtcgaagcgggggcggtgttcgccgagatcggcccgcgcatggccgagttgagcggttcccggctggccgcgcagcaacagatggaaggcctcctggcgccgcaccggcccaaggagcccgcgtggttcctggccaccgtcggcgtctcgcccgaccaccagggcaagggtctgggcagcgccgtcgtgctccccggagtggaggcggccgagcgcgccggggtgcccgccttcctggaaacctccgcgccccgcaacctccccttctacgagcggctcggcttcaccgtcaccgccgacgtcgaggtgcccgaaggaccgcgcacctggtgcatgacccgcaagcccggtgcctgacgcccgccccacgacccgcagcgcccgaccgaaaggagcgcacgaccccatgcatcggtacctttaagaccaatgacttacaaggcagctgtagatcttagccactttctagagtcggggcggccggccgcttcgagcagacatgataagatacattgatgagtttggacaaaccacaactagaatgcagtgaaaaaaatgctttatttgtgaaatttgtgatgctattgctttatttgtaaccattataagctgcaataaacaagttaacaacaacaattgcattcattttatgtttcaggttcagggggaggtgtgggaggttttttaaagcaagtaaaacctctacaaatgtggtaaaatcgataaggatccgtcgaccgatgcccttgagagccttcaacccagtcagctccttccggtgggcgcggggcatgactatcgtcgccgcacttatgactgtcttctttatcatgcaactcgtaggacaggtgccggcagcgctcttccgcttcctcgctcactgactcgctgcgctcggtcgttcggctgcggcgagcggtatcagctcactcaaaggcggtaatacggttatccacagaatcaggggataacgcaggaaagaacatgtgagcaaaaggccagcaaaaggccaggaaccgtaaaaaggccgcgttgctggcgtttttccataggctccgcccccctgacgagcatcacaaaaatcgacgctcaagtcagaggtggcgaaacccgacaggactataaagataccaggcgtttccccctggaagctccctcgtgcgctctcctgttccgaccctgccgcttaccggatacctgtccgcctttctcccttcgggaagcgtggcgctttctcaatgctcacgctgtaggtatctcagttcggtgtaggtcgttcgctccaagctgggctgtgtgcacgaaccccccgttcagcccgaccgctgcgccttatccggtaactatcgtcttgagtccaacccggtaagacacgacttatcgccactggcagcagccactggtaacaggattagcagagcgaggtatgtaggcggtgctacagagttcttgaagtggtggcctaactacggctacactagaaggacagtatttggtatctgcgctctgctgaagccagttaccttcggaaaaagagttggtagctcttgatccggcaaacaaaccaccgctggtagcggtggtttttttgtttgcaagcagcagattacgcgcagaaaaaaaggatctcaagaagatcctttgatcttttctacggggtctgacgctcagtggaacgaaaactcacgttaagggattttggtcatgagattatcaaaaaggatcttcacctagatccttttaaattaaaaatgaagttttaaatcaatctaaagtatatatgagtaaacttggtctgacagttaccaatgcttaatcagtgaggcacctatctcagcgatctgtctatttcgttcatccatagttgcctgactccccgtcgtgtagataactacgatacgggagggcttaccatctggccccagtgctgcaatgataccgcgggacccacgctcaccggctccagatttatcagcaataaaccagccagccggaagggccgagcgcagaagtggtcctgcaactttatccgcctccatccagtctattaattgttgccgggaagctagagtaagtagttcgccagttaatagtttgcgcaacgttgttgccattgctacaggcatcgtggtgtcacgctcgtcgtttggtatggcttcattcagctccggttcccaacgatcaaggcgagttacatgatcccccatgttgtgcaaaaaagcggttagctccttcggtcctccgatcgttgtcagaagtaagttggccgcagtgttatcactcatggttatggcagcactgcataattctcttactgtcatgccatccgtaagatgcttttctgtgactggtgagtactcaaccaagtcattctgagaatagtgtatgcggcgaccgagttgctcttgcccggcgtcaatacgggataataccgcgccacatagcagaactttaaaagtgctcatcattggaaaacgttcttcggggcgaaaactctcaaggatcttaccgctgttgagatccagttcgatgtaacccactcgtgcacccaactgatcttcagcatcttttactttcaccagcgtttctgggtgagcaaaaacaggaaggcaaaatgccgcaaaaaagggaataagggcgacacggaaatgttgaatactcatactcttcctttttcaatattattgaagcatttatcagggttattgtctcatgagcggatacatatttgaatgtatttagaaaaataaacaaataggggttccgcgcacatttccccgaaaagtgccacctgcaggaaacagctatgaccatgattacgccaagctctagctagaggtcgacggtatcgagccccagctggttctttccgcctcagaagccatagagcccaccgcatccccagcatgcctgctattgtcttcccaatcctcccccttgctgtcctgccccaccccaccccccagaatagaatgacacctactcagacaatgcgatgcaatttcctcattttattaggaaaggacagtgggagtggcaccttccagggtcaaggaaggcacgggggaggggcaaacaacagatggctggcaactagaaggcacagtcgaggctgatcagcgggtttaaactcaatggtgatggtgatgatgaccggttagactttcctcttcttcttgggagaaccaccagacttggcctttctgatcttcttaggcttcaggatgttggtgctgccgcacacctcgcaggtattgccgctggcctggatgtggccgcactccttacaggtgatgcttctgtaggggatgcccagctccaggcacttctccatgataatctggtcgatgtagggggtgctgatgttcttggcggcattgtaatcggcgttcacgttttccttcttcacgatgccgccgcactcctcacacacgtcgccgctcacctgcacgtgtctacagttgatgcagatggtcctgctgccgtagccgcactgcttgcactcgaacacggcctggctgctgcggtttgtcttttcgatgtagccgcacatggaacatctctgggatgtgtactgagggttgatggccaccacggtgatgccgtgctccttggccttattcacgatcttggtctgcagatcgtagtaaggccaattcttcaggaacttgctgccggtggtgtcggcgatgccctccagattctcgatctggattgtgccgcagccctgcttaatggcggcctccacgatcctgttggcgtatctgtggttgatggtgtcccggaagttcttctccttctcagacagggtttcgattggcttcagggcccgctttctgccgtggcccttccttgcgtcgccggagtgcttgatctggttctggatgctcactctcctggctctgatcatcttccggaagtgctcgatctcgccgccgtcgatgcagccgcgcttgtagctgctgttgaaggcccagtacacggccttggccacgcccaggtccacgcccatgaccttgtcggggtccagcactgtctcgtgggttgggaaggtgtatgggatgatgcagtaccacttgccctggtggtccttcttgatctgcagctggccctgggtgtaggacttgctggaatcgatgtgatccttagacatgatcctgtcgaagatcatccttgtgctgctgtctctcacggccaccaggaagtacctgtgggtgcccttgccagagtccttggagtactccttggaatacagctgcacgtcgatgatgtacttatttttgttcttgatcagcttgtagatgttgttctgcagcctgataggggctgtggtaatcttgtatgtaggcatgctgatctggtttctgtagatcagcttggcgtttctcttccacacatccttggcgtggttcacgatctggttggccaccttgccgggcagctcagggtgcagcagcttggtcttgtggtacatggcgttgtacaggtccttgctgctaatcctatcctccttaggcatgctaaagtaattatacagatccctcaggcacatattgccggcctcggcgcaaaatctgctcatggtgctcaggtcctttctccagttatcatcctgcttggtacactcagggtccagaaacatatccaggatcttcagcttgatggccttcacgctctcgcccatgactttcctcttcttcttgggcatggtggcggctctccctatagtgagtcgtattagcggccgcggatctctagcggatctgacggttcactaaaccagctctgcttatatagacctcccaccgtacacgcctaccgcccatttgcgtcaatggggcggagttgttacgacattttggaaagtcccgttgattttggtgccaaaacaaactcccattgacgtcaatggggtggagacttggaaatccccgtgagtcaaaccgctatccacgcccattgatgtactgccaaaaccgcatcaccatggtaatagcgatgactaatacgtagatgtactgccaagtaggaaagtcccataaggtcatgtactgggcataatgccaggcgggccatttaccgtcattgacgtcaatagggggcgtacttggcatatgatacacttgatgtactgccaagtgggcagtttaccgtaaatactccacccattgacgtcaatggaaagtccctattggcgttactatgggaacatacgtcattattgacgtcaatgggcgggggtcgttgggcggtcagccaggcgggccatttaccgtaagttatgtaacgcggaactccatatatgggctatgaactaatgaccccgtaattgattactattaataactagtcaataatcaatgtcaacgcgtatatctggcccgtacatcgcgaagcagcgcaaaacgcctaaccctaagcagattcttcatgcaattgtcggtcaagaatcgatagtactaacatacgctctccatcaaaacaaaacgaaacaaaacaaactagcaaaataggctgtccccagtgcaagtgcaggtgccagaacatttctctatcgata

SEQ ID NO: 126 - protein, 433 aa, Artificial Sequence
  EsCas12f_AA
MVCNKVVKIALICDQIDKDGKDVNYNDIYKLLWDLQKQTREAKNKVIRLCWEWSGYSSEYFKTHEEYPKDKEIFGISLRGYLYDRIKGDYNLYSGNLSQSAEIAYKEYKNSLKDVLRGDKSIINYRENQPLDIKNKAIQLLYENDNFFVRVALINKDKQKELNFKDCSVRFKLLVKDDSTRTILERCFDEVYTITASKIMYNKKKKQWYINLGYKFTKEIDKTLDKDRILGVDLGVINPLVASVYGSYDRLIIGGGEIDKFRKRVEANKVQMLKQGKYCGDGRIGHGVNTRNKPAYNIEDKISRFRDTVNHKYSKAVVDYAVKNNCGTIQMEDLKGITQNKNERYLKNWTYFDLQTKIEYKAKALGIEVKYKNPKYTSQRCSKCGHIAEENRPEQKTFKCVKCGFKVNADYNASQNLAIKDIDKIIEQYYNKG

SEQ ID NO: 127 - DNA, 1299 bp, Artificial Sequence
  EsCas12f_NA
atggtttgcaacaaagtggtgaaaatcgcgctgatctgcgaccagatcgataaagacggtaaagatgtgaactacaacgacatctacaaactgctgtgggacctgcagaaacagacccgtgaagcgaaaaacaaagtgatccgcctgtgctgggaatggtccggctacagcagcgaatacttcaaaacccacgaagaatacccgaaagataaagaaatcttcggcatcagcctgcgtggctacctgtacgaccgcattaaaggcgactacaacctgtactctggtaacctgtctcagtctgccgaaatcgcgtacaaagaatacaaaaacagcctgaaagatgttctgcgcggcgataaatctatcatcaactaccgcgaaaaccagccgctggatattaaaaacaaagcgatccagctgctgtacgaaaacgataacttcttcgtacgtgttgcgctgatcaacaaagataaacagaaagaactgaacttcaaagactgcagcgttcgcttcaaactgctggtgaaagatgatagcacccgtaccatcctggaacgttgcttcgacgaagtttataccatcaccgcgagcaaaatcatgtacaacaaaaagaaaaaacagtggtacatcaacctgggctacaaattcaccaaagaaatcgataaaaccctggacaaggaccgtatcctgggtgttgacctgggcgttatcaacccgctggttgcgtccgtgtacggcagctatgatcgcctgatcatcggcggtggtgaaatcgataaatttcgtaaacgcgtggaagcgaacaaagttcagatgctgaaacagggtaaatactgcggcgacggccgcatcggccacggcgttaacacccgtaacaaaccggcgtataacatcgaagataaaatctcccgcttccgtgataccgtgaaccacaaatactctaaagcggttgtggattacgcggtgaaaaacaactgcggtaccatccagatggaggacctgaaaggcatcacccagaacaaaaacgaacgttacctgaaaaactggacctatttcgacctgcagaccaaaatcgaatacaaagcgaaagcgctgggcatcgaagttaaatacaaaaacccgaaatacacctcccagcgttgcagcaaatgcggccacattgcggaagaaaaccgcccggaacagaaaaccttcaaatgcgtgaaatgcggcttcaaagttaacgcggattacaacgcgagccagaacctggcgatcaaagacattgacaaaatcatcgaacagtactacaacaaaggc

SEQ ID NO: 128 - DNA, 6956 bp, Artificial Sequence
  pET28a-SUMO-EsCas12f
tggcgaatgggacgcgccctgtagcggcgcattaagcgcggcgggtgtggtggttacgcgcagcgtgaccgctacacttgccagcgccctagcgcccgctcctttcgctttcttcccttcctttctcgccacgttcgccggctttccccgtcaagctctaaatcgggggctccctttagggttccgatttagtgctttacggcacctcgaccccaaaaaacttgattagggtgatggttcacgtagtgggccatcgccctgatagacggtttttcgccctttgacgttggagtccacgttctttaatagtggactcttgttccaaactggaacaacactcaaccctatctcggtctattcttttgatttataagggattttgccgatttcggcctattggttaaaaaatgagctgatttaacaaaaatttaacgcgaattttaacaaaatattaacgtttacaatttcaggtggcacttttcggggaaatgtgcgcggaacccctatttgtttatttttctaaatacattcaaatatgtatccgctcatgaattaattcttagaaaaactcatcgagcatcaaatgaaactgcaatttattcatatcaggattatcaataccatatttttgaaaaagccgtttctgtaatgaaggagaaaactcaccgaggcagttccataggatggcaagatcctggtatcggtctgcgattccgactcgtccaacatcaatacaacctattaatttcccctcgtcaaaaataaggttatcaagtgagaaatcaccatgagtgacgactgaatccggtgagaatggcaaaagtttatgcatttctttccagacttgttcaacaggccagccattacgctcgtcatcaaaatcactcgcatcaaccaaaccgttattcattcgtgattgcgcctgagcgagacgaaatacgcgatcgctgttaaaaggacaattacaaacaggaatcgaatgcaaccggcgcaggaacactgccagcgcatcaacaatattttcacctgaatcaggatattcttctaatacctggaatgctgttttcccggggatcgcagtggtgagtaaccatgcatcatcaggagtacggataaaatgcttgatggtcggaagaggcataaattccgtcagccagtttagtctgaccatctcatctgtaacatcattggcaacgctacctttgccatgtttcagaaacaactctggcgcatcgggcttcccatacaatcgatagattgtcgcacctgattgcccgacattatcgcgagcccatttatacccatataaatcagcatccatgttggaatttaatcgcggcctagagcaagacgtttcccgttgaatatggctcataacaccccttgtattactgtttatgtaagcagacagttttattgttcatgaccaaaatcccttaacgtgagttttcgttccactgagcgtcagaccccgtagaaaagatcaaaggatcttcttgagatcctttttttctgcgcgtaatctgctgcttgcaaacaaaaaaaccaccgctaccagcggtggtttgtttgccggatcaagagctaccaactctttttccgaaggtaactggcttcagcagagcgcagataccaaatactgtccttctagtgtagccgtagttaggccaccacttcaagaactctgtagcaccgcctacatacctcgctctgctaatcctgttaccagtggctgctgccagtggcgataagtcgtgtcttaccgggttggactcaagacgatagttaccggataaggcgcagcggtcgggctgaacggggggttcgtgcacacagcccagcttggagcgaacgacctacaccgaactgagatacctacagcgtgagctatgagaaagcgccacgcttcccgaagggagaaaggcggacaggtatccggtaagcggcagggtcggaacaggagagcgcacgagggagcttccagggggaaacgcctggtatctttatagtcctgtcgggtttcgccacctctgacttgagcgtcgatttttgtgatgctcgtcaggggggcggagcctatggaaaaacgccagcaacgcggcctttttacggttcctggccttttgctggccttttgctcacatgttctttcctgcgttatcccctgattctgtggataaccgtattaccgcctttgagtgagctgataccgctcgccgcagccgaacgaccgagcgcagcgagtcagtgagcgaggaagcggaagagcgcctgatgcggtattttctccttacgcatctgtgcggtatttcacaccgcatatatggtgcactctcagtacaatctgctctgatgccgcatagttaagccagtatacactccgctatcgctacgtgactgggtcatggctgcgccccgacacccgccaacacccgctgacgcgccctgacgggcttgtctgctcccggcatccgcttacagacaagctgtgaccgtctccgggagctgcatgtgtcagaggttttcaccgtcatcaccgaaacgcgcgaggcagctgcggtaaagctcatcagcgtggtcgtgaagcgattcacagatgtctgcctgttcatccgcgtccagctcgttgagtttctccagaagcgttaatgtctggcttctgataaagcgggccatgttaagggcggttttttcctgtttggtcactgatgcctccgtgtaagggggatttctgttcatgggggtaatgataccgatgaaacgagagaggatgctcacgatacgggttactgatgatgaacatgcccggttactggaacgttgtgagggtaaacaactggcggtatggatgcggcgggaccagagaaaaatcactcagggtcaatgccagcgcttcgttaatacagatgtaggtgttccacagggtagccagcagcatcctgcgatgcagatccggaacataatggtgcagggcgctgacttccgcgtttccagactttacgaaacacggaaaccgaagaccattcatgttgttgctcaggtcgcagacgttttgcagcagcagtcgcttcacgttcgctcgcgtatcggtgattcattctgctaaccagtaaggcaaccccgccagcctagccgggtcctcaacgacaggagcacgatcatgcgcacccgtggggccgccatgccggcgataatggcctgcttctcgccgaaacgtttggtggcgggaccagtgacgaaggcttgagcgagggcgtgcaagattccgaataccgcaagcgacaggccgatcatcgtcgcgctccagcgaaagcggtcctcgccgaaaatgacccagagcgctgccggcacctgtcctacgagttgcatgataaagaagacagtcataagtgcggcgacgatagtcatgccccgcgcccaccggaaggagctgactgggttgaaggctctcaagggcatcggtcgagatcccggtgcctaatgagtgagctaacttacattaattgcgttgcgctcactgcccgctttccagtcgggaaacctgtcgtgccagctgcattaatgaatcggccaacgcgcggggagaggcggtttgcgtattgggcgccagggtggtttttcttttcaccagtgagacgggcaacagctgattgcccttcaccgcctggccctgagagagttgcagcaagcggtccacgctggtttgccccagcaggcgaaaatcctgtttgatggtggttaacggcgggatataacatgagctgtcttcggtatcgtcgtatcccactaccgagatatccgcaccaacgcgcagcccggactcggtaatggcgcgcattgcgcccagcgccatctgatcgttggcaaccagcatcgcagtgggaacgatgccctcattcagcatttgcatggtttgttgaaaaccggacatggcactccagtcgccttcccgttccgctatcggctgaatttgattgcgagtgagatatttatgccagccagccagacgcagacgcgccgagacagaacttaatgggcccgctaacagcgcgatttgctggtgacccaatgcgaccagatgctccacgcccagtcgcgtaccgtcttcatgggagaaaataatactgttgatgggtgtctggtcagagacatcaagaaataacgccggaacattagtgcaggcagcttccacagcaatggcatcctggtcatccagcggatagttaatgatcagcccactgacgcgttgcgcgagaagattgtgcaccgccgctttacaggcttcgacgccgcttcgttctaccatcgacaccaccacgctggcacccagttgatcggcgcgagatttaatcgccgcgacaatttgcgacggcgcgtgcagggccagactggaggtggcaacgccaatcagcaacgactgtttgcccgccagttgttgtgccacgcggttgggaatgtaattcagctccgccatcgccgcttccactttttcccgcgttttcgcagaaacgtggctggcctggttcaccacgcgggaaacggtctgataagagacaccggcatactctgcgacatcgtataacgttactggtttcacattcaccaccctgaattgactctcttccgggcgctatcatgccataccgcgaaaggttttgcgccattcgatggtgtccgggatctcgacgctctcccttatgcgactcctgcattaggaagcagcccagtagtaggttgaggccgttgagcaccgccgccgcaaggaatggtgcatgcaaggagatggcgcccaacagtcccccggccacggggcctgccaccatacccacgccgaaacaagcgctcatgagcccgaagtggcgagcccgatcttccccatcggtgatgtcggcgatataggcgccagcaaccgcacctgtggcgccggtgatgccggccacgatgcgtccggcgtagaggatcgagatctcgatcccgcgaaattaatacgactcactataggggaattgtgagcggataacaattcccctctagaaataattttgtttaactttaagaaggagatataccatgggcagcagccatcatcatcatcatcacagcagcggcctggtgccgcgcggcagcatgtcggactcagaagtcaatcaagaagctaagccagaggtcaagccagaagtcaagcctgagactcacatcaatttaaaggtgtccgatggatcttcagagatcttcttcaagatcaaaaagaccactcctttaagaaggctgatggaagcgttcgctaaaagacagggtaaggaaatggactccttaagattcttgtacgacggtattagaattcaagctgatcagacccctgaagatttggacatggaggataacgatattattgaggctcacagagaacagattggtggtcatagtagtcttgaagtcctctttcagggacccatggtttgcaacaaagtggtgaaaatcgcgctgatctgcgaccagatcgataaagacggtaaagatgtgaactacaacgacatctacaaactgctgtgggacctgcagaaacagacccgtgaagcgaaaaacaaagtgatccgcctgtgctgggaatggtccggctacagcagcgaatacttcaaaacccacgaagaatacccgaaagataaagaaatcttcggcatcagcctgcgtggctacctgtacgaccgcattaaaggcgactacaacctgtactctggtaacctgtctcagtctgccgaaatcgcgtacaaagaatacaaaaacagcctgaaagatgttctgcgcggcgataaatctatcatcaactaccgcgaaaaccagccgctggatattaaaaacaaagcgatccagctgctgtacgaaaacgataacttcttcgtacgtgttgcgctgatcaacaaagataaacagaaagaactgaacttcaaagactgcagcgttcgcttcaaactgctggtgaaagatgatagcacccgtaccatcctggaacgttgcttcgacgaagtttataccatcaccgcgagcaaaatcatgtacaacaaaaagaaaaaacagtggtacatcaacctgggctacaaattcaccaaagaaatcgataaaaccctggacaaggaccgtatcctgggtgttgacctgggcgttatcaacccgctggttgcgtccgtgtacggcagctatgatcgcctgatcatcggcggtggtgaaatcgataaatttcgtaaacgcgtggaagcgaacaaagttcagatgctgaaacagggtaaatactgcggcgacggccgcatcggccacggcgttaacacccgtaacaaaccggcgtataacatcgaagataaaatctcccgcttccgtgataccgtgaaccacaaatactctaaagcggttgtggattacgcggtgaaaaacaactgcggtaccatccagatggaggacctgaaaggcatcacccagaacaaaaacgaacgttacctgaaaaactggacctatttcgacctgcagaccaaaatcgaatacaaagcgaaagcgctgggcatcgaagttaaatacaaaaacccgaaatacacctcccagcgttgcagcaaatgcggccacattgcggaagaaaaccgcccggaacagaaaaccttcaaatgcgtgaaatgcggcttcaaagttaacgcggattacaacgcgagccagaacctggcgatcaaagacattgacaaaatcatcgaacagtactacaacaaaggcgcttaagaattcgagctccgtcgacaagcttgcggccgcactcgagcaccaccaccaccaccactgagatccggctgctaacaaagcccgaaaggaagctgagttggctgctgccaccgctgagcaataactagcataaccccttggggcctctaaacgggtcttgaggggttttttgctgaaaggaggaactatatccggat

SEQ ID NO: 129 - RNA, 189 nt, Artificial Sequence
  EssgRNA
ugcgaauguauaauucacauucaauccgggcggcuuggcguccguaaaucgagaaaguacauuguaaaaacguaauuuuuucguauaguggauacacucgauaagguuaaugcauacgauauuaaucccguaugccgucuauauuuguguuuuugcaguugcaaucuacaugcacggguauagugcaag

SEQ ID NO: 130 - DNA, 234 bp, Artificial Sequence
  EssgRNA_pUC19
aagctaatacgactcactataggggtgcgaatgtataattcacattcaatccgggcggcttggcgtccgtaaatcgagaaagtacattgtaaaaacgtaattttttcgtatagtggatacactcgataaggttaatgcatacgatattaatcccgtatgccgtctatatttgtgtttttgcagttgcaatctacatgcacgggtatagtgcaagctggcgtttttccataggct